European Patent Specification EP 3 615 665 B1, published November 26, 2025. Title: NOVEL ANTI-CRISPR GENES AND PROTEINS AND METHODS OF USE. Applicant: DuPont Nutrition Biosciences ApS and Universite Laval (Canada) Fremaux, Christophe Horvath, Philippe Hynes, Alexander Moineau, Sylvain Romero, Dennis A Rousseau, Genevieve. The sequence listing filed with the application follows.

SEQUENCE LISTING (552 sequences)

SEQ ID NO: 1 - DNA, 327 bp, Bacteriophage O1205
atggcatacggaaaaagcagatacaactcatataggaaacgcagtttcaatagaagcgataagcaacgtagagaatacgcacaagaaatggatagattagaacaaacatttgaaaaacttgatggttggtatctatctagcatgaaagatagtgcgtataaagatttcggaaaatacgaaattcgcttatcaaatcattcagcagacaacaaatatcatgacctagaaaatggtcgtttaattgttaatgtcaaagcaagtaaattgaaattcgttgatatcaaatgttactataagggatttaagacaaagaaggatgtaatctaa

SEQ ID NO: 2 - protein, 108 aa, Bacteriophage O1205
MAYGKSRYNSYRKRSFNRSDKQRREYAQEMDRLEQTFEKLDGWYLSSMKDSAYKDFGKYEIRLSNHSADNKYHDLENGRLIVNVKASKLKFVDIKCYYKGFKTKKDVI

SEQ ID NO: 3 - DNA, 423 bp, Bacteriophage Sfi21
atggcatacggaaaaagtagatataactcatatagaaagcgcagttttaacagaagtaataagcaacgtagagaatacgcacaagaaatggatagattagagaaagctttcgaaaatcttgacggatggtatctatctagcatgaaagatagtgcgtacaaagatttcggaaaatacgaaattcgcttatcaaatcattcagcagacaacaaatatcatgacctagaaaatggtcgtttaattgttaatgtcaaagcaagtaaattgaacttcgttgatatcatcgagaacaaacttgataaaatcattgagaagattgatactcttgatttagataagtacagattcattaatgctactaaattggaacgtgatatcaaatgctactataaaggctataagacaaagaaggatgtaatctaa

SEQ ID NO: 4 - protein, 140 aa, Bacteriophage Sfi21
MAYGKSRYNSYRKRSFNRSNKQRREYAQEMDRLEKAFENLDGWYLSSMKDSAYKDFGKYEIRLSNHSADNKYHDLENGRLIVNVKASKLNFVDIIENKLDKIIEKIDTLDLDKYRFINATKLERDIKCYYKGYKTKKDVI

SEQ ID NO: 5 - DNA, 423 bp, Bacteriophage TP-778L
atggcatacggaaaaagcagatacaactcatatagaaaacgtagtttcaacataagtgacacaaagcgtagggaatatgcaaaagaaatggagaaattagaacaagcatttgaaaagctagatggttggtatctatctagcatgaaggatagtgcatacaaggattttggaaaatacgaaatccgcttatcaaatcattcagcagacaataaatatcatgacctagaaaatggtcgtttaattgttaatgttaaagcaagtaaattgaacttcgttgatatcatcgaaaacaaacttgataaaatcatcgagaagattgataagcttgatttagataagtacagatttattaacgctactagaatggagcatgacattaaatgctactataaaggatttaagacaaagaaagatgtaatctaa

SEQ ID NO: 6 - protein, 140 aa, Bacteriophage TP-778L
MAYGKSRYNSYRKRSFNISDTKRREYAKEMEKLEQAFEKLDGWYLSSMKDSAYKDFGKYEIRLSNHSADNKYHDLENGRLIVNVKASKLNFVDIIENKLDKIIEKIDKLDLDKYRFINATRMEHDIKCYYKGFKTKKDVI

SEQ ID NO: 7 - DNA, 423 bp, Streptococcus sp.
atggcatttggcaagaacagatacaatccatacaggaaacgtagttttaatcgtagtgataaacaatgtcgagagtatgctcaggcaatggacgaactagaacaagcctttgaggaacttgatggatggcacttatctagtatgatggatagtgcttataagaattttgaaaagtaccaggttcgcctatcaaatcattcagcagacaaccaatatcatgacttagaaaatggttacttgattgtcaatgttaaagcaagtaaattgaactttgtcgatattatcgaaaataaattggataagattttagagaaagtagacaagcttgatcttgataagtataggtttatcaatgcgaccaatctggaacatgatattaaatgttatctcaaaggctataagacgaaaaaagacgtgatttaa

SEQ ID NO: 8 - protein, 140 aa, Streptococcus sp.
MAFGKNRYNPYRKRSFNRSDKQCREYAQAMDELEQAFEELDGWHLSSMMDSAYKNFEKYQVRLSNHSADNQYHDLENGYLIVNVKASKLNFVDIIENKLDKILEKVDKLDLDKYRFINATNLEHDIKCYLKGYKTKKDVI

SEQ ID NO: 9 - DNA, 423 bp, Bacteriophage D4276
atggcatacggaaaaagtagatataactcatatagaaagcgcagttttaacagaagtaataagcaacgtagagaatacgcacaagaaatggatagattagagaaagctttcgaaaatcttgacggatggtatctatctagcatgaaagacagtgcttacaaggattttgggaaatacgaaattcgcttatcaaatcattcggcagacaacaaatatcacgacttagaaaacggtcgtttaattgttaatattaaagctagtaaattgaatttcgttgatatcatcgagaataagcttgataaaataatcgagaagattgataagcttgatttagataagtaccgattcatcaatgcgaccaacctagagcatgatatcaaatgctattacaaggggtttaaaacgaaaaaggaggtaatctaa

SEQ ID NO: 10 - protein, 140 aa, Bacteriophage D4276
MAYGKSRYNSYRKRSFNRSNKQRREYAQEMDRLEKAFENLDGWYLSSMKDSAYKDFGKYEIRLSNHSADNKYHDLENGRLIVNIKASKLNFVDIIENKLDKIIEKIDKLDLDKYRFINATNLEHDIKCYYKGFKTKKEVI

SEQ ID NO: 11 - DNA, 423 bp, Bacteriophage D1126
atggcatacggaaaaagcagatacaattcatataggaagcgaaacttctctataagcgacaatcagcgtagggaatatgctaaaaaaatgaaggagttagaacaagcgtttgaaaaccttgacggatggtatctatctagcatgaaagatagtgcgtacaaagatttcggaaaatacgaaattcgcttatcaaatcattcagcagacaatagatatcatgacctagaaaatggtcgcttaatcgttaatgttaaagctagtaaattgaacttcgttgatatcatcgagaataaacttggtaaaatcattgagaagattgatactcttgatttagataagtacagattcattaatgctactaaattggaacgtgatatcaaatgctactataaaggctataagacaaagaaggatgtaatctaa

SEQ ID NO: 12 - protein, 140 aa, Bacteriophage D1126
MAYGKSRYNSYRKRNFSISDNQRREYAKKMKELEQAFENLDGWYLSSMKDSAYKDFGKYEIRLSNHSADNRYHDLENGRLIVNVKASKLNFVDIIENKLGKIIEKIDTLDLDKYRFINATKLERDIKCYYKGYKTKKDVI

SEQ ID NO: 13 - DNA, 423 bp, Bacteriophage D4250
atggcatacggaaaaagtagatataactcatatagaaaacgcagtttcaacagaagcgataaacagcgtagagaatacgcacaagcaatggaagaattagagcaagcatttgaaaactttgatgattggtatctatcaagcatgaaagacagtgcttacaaggattttgggaaatacgaaattcgcttatcaaatcattcggcagacaacaaatatcacgacttagaaaacggtcgtttaattgttaatattaaagctagtaaattgaatttcgttgatatcatcgagaataagcttgataaaataatcgagaagattgataagcttgatttagataagtaccgattcatcaatgcgaccaacctagagcatgatatcaaatgctattacaaggggtttaaaacgaaaaaggaggtaatctaa

SEQ ID NO: 14 - protein, 140 aa, Bacteriophage D4250
MAYGKSRYNSYRKRSFNRSDKQRREYAQAMEELEQAFENFDDWYLSSMKDSAYKDFGKYEIRLSNHSADNKYHDLENGRLIVNIKASKLNFVDIIENKLDKIIEKIDKLDLDKYRFINATNLEHDIKCYYKGFKTKKEVI

SEQ ID NO: 15 - DNA, 423 bp, Bacteriophage D4252
atggcatacggaaaaagcagatacaactcatatagaaagcgcagttttaacagaagtgataagcaacgtagagaatacgctaaaaaaatgaaggagttagaacaagcgtttgaaaaccttgatggttggtatctatcgagcatgaatgacagtgcttataaaaattttggcaaatatgaagttcgattgtcaaatcattcggcagataataaatatcacgacatagaaaacggtcgtttaattgttaatgttaaagctagtaaattgaatttcgttgatatcatcgagaacaagcttgataaaataatcgagaagattgataagcttgatttagataagtaccgattcatcaacgctaccaatctagagcataatattaaatgctattacaagggatttaagacaaagaaggatgtaatataa

SEQ ID NO: 16 - protein, 140 aa, Bacteriophage D4252
MAYGKSRYNSYRKRSFNRSDKQRREYAKKMKELEQAFENLDGWYLSSMNDSAYKNFGKYEVRLSNHSADNKYHDIENGRLIVNVKASKLNFVDIIENKLDKIIEKIDKLDLDKYRFINATNLEHNIKCYYKGFKTKKDVI

SEQ ID NO: 17 - DNA, 423 bp, Bacteriophage D4598
atggcatacggaaaaagtagatataactcatatagaaaacgcagtttcaacagaagcgataaacagcgtggagaatacgcacaagcaatggaagaattagagcaagcatttgaaaactttgatgattggtatctatcaagcatgaaagacagtgcttacaaggattttgggaaatacgaaattcgcttatcaaatcattcggcagacaataaatatcatgacctagaaaatggtcgcttaatcgttaatgttaaagctagtaaattgaacttcgtcgatatcatcgagaataaaatcgataaaatcattgagaagattgataagcttgatttagataagtaccgattcatcaacgctaccaacctagagcatgatatcaaatgttattacaagggatttaagacaaaaaaggatgtaatctaa

SEQ ID NO: 18 - protein, 140 aa, Bacteriophage D4598
MAYGKSRYNSYRKRSFNRSDKQRGEYAQAMEELEQAFENFDDWYLSSMKDSAYKDFGKYEIRLSNHSADNKYHDLENGRLIVNVKASKLNFVDIIENKIDKIIEKIDKLDLDKYRFINATNLEHDIKCYYKGFKTKKDVI

SEQ ID NO: 19 - DNA, 423 bp, Streptococcus mutans
atggcatttggaaaaagaagatataactcgtatcgtaaacgcagttttaatagaagtgataagcaacgtcgagaatatgcacaagcaatggaagaacttgaacaaacatttgaaaatcttgaaggttggaatttatcaagcatgaaagatagtgcttataaagattatgataaatatgaagttcgactttcaaatcattcagctgataatcaatatcataacttacaagatggtaaattaatcatcaatatcaaagctagtaaaatgaattttgtttggattatagaaaataaacttgatgcaattcttgaaaaagtaaataagttagaccttagcaaatacagatttattaatgctacaagtttagatcatgatatcaaatgttattacaaaaattataaaacaaagaaagatgtaatttaa

SEQ ID NO: 20 - protein, 140 aa, Streptococcus mutans
MAFGKRRYNSYRKRSFNRSDKQRREYAQAMEELEQTFENLEGWNLSSMKDSAYKDYDKYEVRLSNHSADNQYHNLQDGKLIINIKASKMNFVWIIENKLDAILEKVNKLDLSKYRFINATSLDHDIKCYYKNYKTKKDVI

SEQ ID NO: 21 - DNA, 423 bp, Streptococcus mutans
atggcatttggaacaagaagatataattcatatcgtaaacgcagttttaatagaagtgataagcaacgtcgagaatatgcacaagcaatggaagaacttgaacaaacatttgaaaatcttgaagattggaatttgtcgagcatgaaagatagtgcttataaagattatgataaatatgaagttcgactttcaaatcattcagctgataatcaatatcataacttacaagatggtaaattaatcatcaatatcaaagctagtaaaatgaattttgtttggattatagaaaataaacttgatgcaattcttgaaaaagtaaataagttagaccttagcagatacagatttattaatgctacaaatttagaacatgatatcaaatgttattacaaaaattataaaacaaagaaagatgtaatttaa

SEQ ID NO: 22 - protein, 140 aa, Streptococcus mutans
MAFGTRRYNSYRKRSFNRSDKQRREYAQAMEELEQTFENLEDWNLSSMKDSAYKDYDKYEVRLSNHSADNQYHNLQDGKLIINIKASKMNFVWIIENKLDAILEKVNKLDLSRYRFINATNLEHDIKCYYKNYKTKKDVI

SEQ ID NO: 23 - DNA, 423 bp, Streptococcus mutans
atggcatttggaacaagaagatataattcatatcgtaaacgcagttttaatagaagtgataagcaacgtcgagaatatgcacaagcaatggaagaacttgaacaaacatttgaaaatcttgaagattggaatttgtcgagcatgaaagatagtgcttataaagattatgataaatatgaagttagactttcaaatcattcagctgataatcaatatcataacttacaagatggtaaattaatcatcaatatcaaagctagtaaaatgaattttgtttggattatagaaaataaacttgatgtaattcttgaaaaagtaaataagttagaccttagcaaatacagatttattaatgctacaagtttagatcatgatatcaaatgttattacaaaaattataaaacaaagaaagatgtaatctaa

SEQ ID NO: 24 - protein, 140 aa, Streptococcus mutans
MAFGTRRYNSYRKRSFNRSDKQRREYAQAMEELEQTFENLEDWNLSSMKDSAYKDYDKYEVRLSNHSADNQYHNLQDGKLIINIKASKMNFVWIIENKLDVILEKVNKLDLSKYRFINATSLDHDIKCYYKNYKTKKDVI

SEQ ID NO: 25 - DNA, 423 bp, Streptococcus mutans
atggcatttggaacaagaagatataattcatatcgtaaacgcaattttaatagaagtgataaacaacgtcgagaatatgcacaagcaatggaagaacttgaacaaacatttgaaaatcttgaagattggaatttgtcgagcatgaaagatagtgcttataaagattatgataaatttgaagttcgactttcaaatcattcagctgataatcaatatcataacttacaagatggtaaattaatcatcaatatcaaagctagtaaaatgaattttgtttggattatagaaaataaacttgatgcaattcttgaaaaggtaaataagttagaccttagcaaatacagatttattaatgctacaagtttagatcatgatatcaaatgttattacaaaaattataaaacaaaaaaagatgtaatttaa

SEQ ID NO: 26 - protein, 140 aa, Streptococcus mutans
MAFGTRRYNSYRKRNFNRSDKQRREYAQAMEELEQTFENLEDWNLSSMKDSAYKDYDKFEVRLSNHSADNQYHNLQDGKLIINIKASKMNFVWIIENKLDAILEKVNKLDLSKYRFINATSLDHDIKCYYKNYKTKKDVI

SEQ ID NO: 27 - DNA, 552 bp, Bacteriophage D1811
atgaaaataaatgacgacatcaaagagttaattttagaatatatgagccgttacttcaaattcgagaacgacttttataaactgccaggcatcaagttcactgatgcaaattggcagaagttcaaaaatggaggcactgacattgagaagatgggggcggcacgagtaaacgccatgctcgactgcctattcgacgatttcgagcttgctatgattggcaaggctcaaactaattattacaatgataattcactaaagatgaacatgccattttacacttactatgacatgttcaaaaagcagcaacttctaaaatggcttaaaaataaccgtgatgatgtcatcggcggaactggtaggatgtacacagcaagtggtaattacattgctaacgcttatttagaggtggcattagaatcgagctcgcttggtagtggctcttacatgcttcaaatgaggtttaaagactattcaaaaggtcaagaacctattccgtcaggtcgtcagaatcgacttgaatggattgaaaacaatctcgaaaacattcgataa

SEQ ID NO: 28 - protein, 183 aa, Bacteriophage D1811
MKINDDIKELILEYMSRYFKFENDFYKLPGIKFTDANWQKFKNGGTDIEKMGAARVNAMLDCLFDDFELAMIGKAQTNYYNDNSLKMNMPFYTYYDMFKKQQLLKWLKNNRDDVIGGTGRMYTASGNYIANAYLEVALESSSLGSGSYMLQMRFKDYSKGQEPIPSGRQNRLEWIENNLENIR

SEQ ID NO: 29 - DNA, 552 bp, Bacteriophage D1024
atgaaaataaatgacgacatcaaagagttaattttagaatatatgagccgttacttcaaattcgagaacgacttttataaactgccaggcatcaagttcactgatgcaaattggcagaagttcaaaaatggaggcactgacattgagaagatgggggcggcacgagtaaatgccatgctttcctgcctattcgaggattttgagcttgcaatgattggcaaggctcaaactaattattacattgataactcacttaaattgaacatgccattttacgcttactatgacatgttcaaaaagcaacttcttataaattggcttaaaaataaccgtgatgatgtcatctgcggaactggtaggatgtacacagcaagtggtaattacattgctaacgcttatttagaggtggcattagaatctagccgtctgggtggtggtgagtacatgttgcaaatgcgttttaaaaattattcaagaagtcaagaacctattccgtctggtcgtcagaatcgacttgaatggattgaaaacaatcttgaaaacattcgataa

SEQ ID NO: 30 - protein, 183 aa, Bacteriophage D1024
MKINDDIKELILEYMSRYFKFENDFYKLPGIKFTDANWQKFKNGGTDIEKMGAARVNAMLSCLFEDFELAMIGKAQTNYYIDNSLKLNMPFYAYYDMFKKQLLINWLKNNRDDVICGTGRMYTASGNYIANAYLEVALESSRLGGGEYMLQMRFKNYSRSQEPIPSGRQNRLEWIENNLENIR

SEQ ID NO: 31 - DNA, 552 bp, Bacteriophage D4530
atgaaaatcaataatgacatcaaagagctaattttggaatatgtaagtcgctattttaaatttgaaaacgacttctacaaattgccaggcatcaaattcactgatgcaaattggcaaaaattcaagaatggagatacttccatcgagaagatgggggcagcacgagtaaatgccatgcttgactgcctgttcgaagattttgagcttgcaatgattggcaaggctcaaactaattattacaatgataattcactaaagatgaacatgccattttacacttactatgacatgttcaaaaagcagcaacttctaaaatggcttaaaaataaccgtgatgatgtcatctgcggaactggtaggatgtacacagcaagtggtaattacattgctaacgcttatttagaaattgcgttagaatctagccgtctgggtagtggctcttacatgcttcaaatgagattcaaagactattcaagaagtcaagaacctattccgtctggtcgccaaaatagactagaatggattgagagcaacttggaaaacattcgataa

SEQ ID NO: 32 - protein, 183 aa, Bacteriophage D4530
MKINNDIKELILEYVSRYFKFENDFYKLPGIKFTDANWQKFKNGDTSIEKMGAARVNAMLDCLFEDFELAMIGKAQTNYYNDNSLKMNMPFYTYYDMFKKQQLLKWLKNNRDDVICGTGRMYTASGNYIANAYLEIALESSRLGSGSYMLQMRFKDYSRSQEPIPSGRQNRLEWIESNLENIR

SEQ ID NO: 33 - DNA, 552 bp, Bacteriophage D2759
atgaaaatcaataatgacatcaaagagctaattttggaatatgtaagtcgctattttaaatttgaaaacgacttctacaaattgccaggcatcaaattcactgatgcaaattggcaaaaattcaagaatggagatacttccatcgagaagatgggggcagcacgagtaaatgccatgcttgactgcctattcgacgattttgagcttgctttgattggcaaggctcaaactaattattacattgataactcacttaaattgaacatgccattttacgcttactatgacatgttcaaaaagcagcaacttctaaaatggcttaaaaataaccgtgatgatgtcatctgcggaactggtaggatgtacacagcaagtggtaattacattgctaactcttatttagaggtagcgttagaatctagccgtctgggtagtggctcttacatgcttcaaatgagattcaaagactattcaagaagtcaagaacctattccatctggtcgccaaaatagactagaatggattgagagcaacttggaaaacattcgataa

SEQ ID NO: 34 - protein, 183 aa, Bacteriophage D2759
MKINNDIKELILEYVSRYFKFENDFYKLPGIKFTDANWQKFKNGDTSIEKMGAARVNAMLDCLFDDFELALIGKAQTNYYIDNSLKLNMPFYAYYDMFKKQQLLKWLKNNRDDVICGTGRMYTASGNYIANSYLEVALESSRLGSGSYMLQMRFKDYSRSQEPIPSGRQNRLEWIESNLENIR

SEQ ID NO: 35 - DNA, 552 bp, Bacteriophage D1297
atgaaaatcaataatgacatcaaagagctaattttggaatatgtaagtcgctattttaaatttgaaaacgacttctacaaattgcaaggcatcaaattcactgatgcaaattggcaaaaattcaagaatggagatacttccatcgagaagatgggggcagcacgagtaaatgccatgcttgactgcctattcgacgattttgagcttgctttgattggcaaggctcaacaagaatactattcggataattccttgaaattgaacatgccattttacgcttactatgacatgttcaaaaagcagcaacttctaaaatggcttaaaaataaccgtgatgatgtcatctgcggaactggtaggatgtacacagcaagtggtaattacattgctaactcttatttagaggtagcgttagaatctagccgtctgggtagtggctcttacatgcttcaaatgagattcaaagactattcaagaagtcaagaacctattccgtcaggtcgcaaaaaccgacttgagtggattgaaaacaatctggaaaatattcgataa

SEQ ID NO: 36 - protein, 183 aa, Bacteriophage D1297
MKINNDIKELILEYVSRYFKFENDFYKLQGIKFTDANWQKFKNGDTSIEKMGAARVNAMLDCLFDDFELALIGKAQQEYYSDNSLKLNMPFYAYYDMFKKQQLLKWLKNNRDDVICGTGRMYTASGNYIANSYLEVALESSRLGSGSYMLQMRFKDYSRSQEPIPSGRKNRLEWIENNLENIR

SEQ ID NO: 37 - DNA, 552 bp, Bacteriophage M5728
atgaaaatcaataatgacatcaaagagctaattttggaatatgtaagtcgctattttaaatttgaaaacgacttctacaaattgccaggcatcaaattcactgatgcaaattggcaaaaattcaagaatggagatacttccatcgagaagatgggggcagcacgagtaaatgccatgcttgactgcctattcgacgattttgagcttgcttttattggcaaggctcaacaagaatactattcggataattccttgaaattgaacatgccattttacgcttactatgacatgttcaaaaagcagcaacttctaaaatggcttaaaaataaccgtgatgatgtcatctgcggaactggtaggatgtacacagcaagtggtaattacattgctaactcttatttagaggtagcgttagaatctagccgtctgggtagtggctcttacatgcttcaaatgagattcaaagactattcaagaagtcaagaacctattccatctggtcgccaaaatagactagaatggattgaaaacaatcttgagaatattcgataa

SEQ ID NO: 38 - protein, 183 aa, Bacteriophage M5728
MKINNDIKELILEYVSRYFKFENDFYKLPGIKFTDANWQKFKNGDTSIEKMGAARVNAMLDCLFDDFELAFIGKAQQEYYSDNSLKLNMPFYAYYDMFKKQQLLKWLKNNRDDVICGTGRMYTASGNYIANSYLEVALESSRLGSGSYMLQMRFKDYSRSQEPIPSGRQNRLEWIENNLENIR

SEQ ID NO: 39 - DNA, 552 bp, Bacteriophage D4419
atgaaaatcaataatgacatcaaagagctaattttggaatatgtaagtcgctattttaaatttgaaaacgacttctacaaattgccaggcatcaaattcactgatgcaaattggcaaaaattcaagaatggagatacttccatcgagaagatgggggcagcacgagtaaatgccatgcttgactgcctattcgacgattttgagcttgctttgattggcaaggctcaacaagaatactattcggataattccttgaaattgaacatgccattttacgcttactatgacatgttcaaaaagcagcaacttctaaaatggcttaaaaataaccgtgatgatgtcatctgcggaactggtaggatgtacacagcaagtggtaattacattgctaactcttatttagaggtagcgttagaatctagccgtctgggtagtggctcttacatgcttcaaatgagattcaaagactattcaagaagtcaagaacctattccatctggtcgccaaaatagactagaatggattgagagcaacttggaaaacattcgataa

SEQ ID NO: 40 - protein, 183 aa, Bacteriophage D4419
MKINNDIKELILEYVSRYFKFENDFYKLPGIKFTDANWQKFKNGDTSIEKMGAARVNAMLDCLFDDFELALIGKAQQEYYSDNSLKLNMPFYAYYDMFKKQQLLKWLKNNRDDVICGTGRMYTASGNYIANSYLEVALESSRLGSGSYMLQMRFKDYSRSQEPIPSGRQNRLEWIESNLENIR

SEQ ID NO: 41 - DNA, 552 bp, Bacteriophage D5891
atgaaaatcaataatgacatcaaagagctaattttggaatatgtaagtcgctattttaaatttgaaaacgacttctacaaattgccaggcatcaaattcactgatgcaaattggcaaaaattcaagaatggagatacttccatcgagaagatgggggcagcacgagtaaatgccatgcttgactgcctattcgacgattttgagcttgcttttattggcaaggctcaacaagaatactattcggataattccttgaaattgaacatgccattttacgcttactatgacatgttcaaaaagcagcaacttctaaaatggcttaaaaataaccgtgatgatgtcatctgcggaactggtaggatgtacacagcaagtggtaattacattgctaactcttatttagaggtagcgttagaatctagccgtctgggtagtggctcttacatgcttcaaatgagattcaaagactattcaagaagtcaagaacctattccatctggtcgccaaaatagactagaatggattgagagcaacttggaaaacattcgataa

SEQ ID NO: 42 - protein, 183 aa, Bacteriophage D5891
MKINNDIKELILEYVSRYFKFENDFYKLPGIKFTDANWQKFKNGDTSIEKMGAARVNAMLDCLFDDFELAFIGKAQQEYYSDNSLKLNMPFYAYYDMFKKQQLLKWLKNNRDDVICGTGRMYTASGNYIANSYLEVALESSRLGSGSYMLQMRFKDYSRSQEPIPSGRQNRLEWIESNLENIR

SEQ ID NO: 43 - DNA, 552 bp, Bacteriophage ALQ13.2
atgaaaatcaataatgacatcaaagagctaattttggaatatgtaagtcgctattttaaatttgaaaacgacttctacaaattgccaggcatcaaattcactgatgcaaattggcaaaaattcaagaacggagatacttccatcgagaagatgggggcagcacgagtaaatgccatgcttgactgcctattcgacgattttgagcttgctttgattggcaaggctcaacaagaatactattcggataattccttgaaattgaacatgccattttacgcttactatgacatgttaaaaaagcagcaacttctaaaatggcttaaaaataaccgtgatgatgtcatctgcggaactggtaggatgtacacagcaagtggtaattacattgctaactcttatttagaggtagcgttagaatctagccgtctgggtagtggctcttacatgcttcaaatgagattcaaagactattcaagaagtcaagaacctattccatctggtcgccaaaatagactagaatggattgagagcaacttggaaaacattcgatga

SEQ ID NO: 44 - protein, 183 aa, Bacteriophage ALQ13.2
MKINNDIKELILEYVSRYFKFENDFYKLPGIKFTDANWQKFKNGDTSIEKMGAARVNAMLDCLFDDFELALIGKAQQEYYSDNSLKLNMPFYAYYDMLKKQQLLKWLKNNRDDVICGTGRMYTASGNYIANSYLEVALESSRLGSGSYMLQMRFKDYSRSQEPIPSGRQNRLEWIESNLENIR

SEQ ID NO: 45 - DNA, 552 bp, Bacteriophage D802
atgaaaatcaataatgacatcaaagagctaattttggaatatgtaagtcgctattttaaattcgagaacgacttttacagattgcctggcatcaaattcactgatgccaactggcaaaaattcaagaatggaggcactgccattgagaagatgggagcagcacgagttaatgccatgctttcctgcctattcgaggattttgagcttgcaatgattggcaaggctcaatatgaatactattcggataattccttgaaattgaacatgccattttacgcttactatgacatgttcaaaaagcagcaacttctaaaatggcttaaaaataaccgtgatgatgtcatcggcggaactggtagaatgtacacgtcaagcggtagttacattgctaacgcttatttagaaattgcgttagaatctagccgtctgggtagtggctcttacatgcttcaaatgagattcaaagactattcaagaagtcaagaacctattccgtctggtcgccaaaatagacttgaatggattgagagcaacttggaaaacattcgataa

SEQ ID NO: 46 - protein, 183 aa, Bacteriophage D802
MKINNDIKELILEYVSRYFKFENDFYRLPGIKFTDANWQKFKNGGTAIEKMGAARVNAMLSCLFEDFELAMIGKAQYEYYSDNSLKLNMPFYAYYDMFKKQQLLKWLKNNRDDVIGGTGRMYTSSGSYIANAYLEIALESSRLGSGSYMLQMRFKDYSRSQEPIPSGRQNRLEWIESNLENIR

SEQ ID NO: 47 - DNA, 552 bp, Bacteriophage 73
atgaaaatcaataatgacatcaaagagctaattttggaatatgtaagtcgctattttaaatttgaaaacgacttctacaaattacctggcatcaaattcactgatgccaactggcaaaaattcaagaatggagatacttccatcgagaagatgggggcagcacgagtaaatgccatgcttgactgcctattcgaggattttgagcttgcaatgattggcaaggctcaaactaattattacattgataactcacttaaattgaacatgccattttacgcttactatgacatgttcaaaaagcagcaacttctaaaatggcttaaaaataaccgtgatgatgtcatcggcggaactggtaggatgtacacagcaagtggtaattacattgctaacgcttatttagaggtggcattagaatcgagctcgcttggtagtggctcttacatgcttcaaatgaggtttaaagactattcaaaaggtcaagaacctattccgtcaggtcgtcagaatcgacttgaatggattgaaaacaatctcgaaaacattcgataa

SEQ ID NO: 48 - protein, 183 aa, Bacteriophage 73
MKINNDIKELILEYVSRYFKFENDFYKLPGIKFTDANWQKFKNGDTSIEKMGAARVNAMLDCLFEDFELAMIGKAQTNYYIDNSLKLNMPFYAYYDMFKKQQLLKWLKNNRDDVIGGTGRMYTASGNYIANAYLEVALESSSLGSGSYMLQMRFKDYSKGQEPIPSGRQNRLEWIENNLENIR

SEQ ID NO: 49 - DNA, 552 bp, Bacteriophage DT1
atgaaaatcaataatgacatcaaagagctaattttggaatatgtaagtcgctattttaaatttgaaaacgacttctacaaattacctggcatcaaattcactgatgccaactggcaaaaattcaagaatggagaaacttcaatcgaaaaaatgggagcagcacgagttaatgccatgctttcatgcctattcgaggattttgagcttgcaatgattggcaaggctcaaactaattattacattgataactcacttaaattgaacatgccattttacgcttactatgacatgttcaaaaagcaacttcttataaattggcttaaaaataaccgtgatgatgtcatcggcggaactggtaggatgtacacagcaagtggtaattacattgctaacgcttatttagaggtggcattagaatcaagctcgcttggtagtggctcttacatgatccaaatgaggtttaaagactattcaaaaggtcaagaacctattccgtcaggtcgcaaaaaccgacttgagtggattgaaaacaatctggaaaatattcgataa

SEQ ID NO: 50 - protein, 183 aa, Bacteriophage DT1
MKINNDIKELILEYVSRYFKFENDFYKLPGIKFTDANWQKFKNGETSIEKMGAARVNAMLSCLFEDFELAMIGKAQTNYYIDNSLKLNMPFYAYYDMFKKQLLINWLKNNRDDVIGGTGRMYTASGNYIANAYLEVALESSSLGSGSYMIQMRFKDYSKGQEPIPSGRKNRLEWIENNLENIR

SEQ ID NO: 51 - DNA, 552 bp, Bacteriophage D1427
atgaaaatcaataatgacatcaaagagctaattttggaatatgtaagtcgctattttaaatttgaaaacgacttctacaaattacctggcatcaaattcactgatgccaactggcaaaaattcaagaatggagaaacttcaatcgaaaaaatgggagcagcacgagttaatgccatgctttcatgcctattcgaggattttgagcttgcaatgattggcaaggctcaaactaattattacattgataactcacttaaattgaacatgccattttacgcttactatgacatgttcaaaaagcaacttcttataaattggcttaaaaataaccgtgatgatgtcatcggcggaactggtaggatgtacacagcaagtggtaattacattgctaacgcttatttagaggtggcattagaatcaagctcgcttggtagtggctcttacatgatccaaatgaggtttaaagactattcaaaaggtcaagaacctattccgtcaggtcgccaaaatagactagaatggattgagagcaacttggaaaacattcgataa

SEQ ID NO: 52 - protein, 183 aa, Bacteriophage D1427
MKINNDIKELILEYVSRYFKFENDFYKLPGIKFTDANWQKFKNGETSIEKMGAARVNAMLSCLFEDFELAMIGKAQTNYYIDNSLKLNMPFYAYYDMFKKQLLINWLKNNRDDVIGGTGRMYTASGNYIANAYLEVALESSSLGSGSYMIQMRFKDYSKGQEPIPSGRQNRLEWIESNLENIR

SEQ ID NO: 53 - DNA, 552 bp, Bacteriophage N1162
atgaaaatcaataatgacatcaaagagctaattttggaatatgtaagtcgctattttaaatttgaaaacgacttctacaaattacctggcatcaaattcactgatgccaactggcaaaaattcaagaatggagatacttccatcgagaagatgggggcagcacgagtaaatgccatgcttgactgcctattcgaggattttgagcttgcaatgattggcaaggctcaaactaattattacattgataactcacttaaattgaacatgccattttacgcttactatgacatgttcaaaaagcagcaacttctaaaatggcttaaaaataaccgtgatgatgtcatcggcggaactggtaggatgtacacatcaaccggtaattacattgctaacgcttatttagaaattgcgttagaatctagccgtctgggtagtggctcttacatgatccaaatgaggtttaaagactattcaaaaggtcaagaacctattccgtctggtcgtcagaatcgacttgaatggattgaaaacaatctggaaaatattcgataa

SEQ ID NO: 54 - protein, 183 aa, Bacteriophage N1162
MKINNDIKELILEYVSRYFKFENDFYKLPGIKFTDANWQKFKNGDTSIEKMGAARVNAMLDCLFEDFELAMIGKAQTNYYIDNSLKLNMPFYAYYDMFKKQQLLKWLKNNRDDVIGGTGRMYTSTGNYIANAYLEIALESSRLGSGSYMIQMRFKDYSKGQEPIPSGRQNRLEWIENNLENIR

SEQ ID NO: 55 - DNA, 552 bp, Bacteriophage D1018
atgaaaatcaataatgatatcaaagagctaattttggaatatgtaagtcgctattttaaatttgaaaacgacttctacaaattgccagacatcaagttcacagatgctaattggcaaaaatttaagaatggagaaacttcaatcgaaaaaatgggagcagcacgagtaaatgccatgcttgactgcctattcgaggattttgagcttgcaatgattggcaaggctcaaactaattattacattgataactcacttaaattgaacatgccattttacgcttactatgacatgttcaaaaagcagcaacttctaaaatggcttaaaaataaccgtgatgatgtcatcggcggaactggtaggatgtacacatcaaccggtaattacattgctaacgcttatttagaaattgcgttagaatctagccgtctgggtagtggctcttacatgatccaaatgaggtttaaagactattcaaaaggtcaagaacctattccgtctggtcgtcagaatcgacttgaatggattgaaaacaatctggaaaatattcgataa

SEQ ID NO: 56 - protein, 183 aa, Bacteriophage D1018
MKINNDIKELILEYVSRYFKFENDFYKLPDIKFTDANWQKFKNGETSIEKMGAARVNAMLDCLFEDFELAMIGKAQTNYYIDNSLKLNMPFYAYYDMFKKQQLLKWLKNNRDDVIGGTGRMYTSTGNYIANAYLEIALESSRLGSGSYMIQMRFKDYSKGQEPIPSGRQNRLEWIENNLENIR

SEQ ID NO: 57 - DNA, 552 bp, Bacteriophage D3577
atgaaaataaacaacgatatcaaagagctaattttggaatacgctaaacgttatttcaagtttgaaaacgacttctacaaactgccagacatcaaattcactgatgccaactggcaaaaatttaagaatggagaaacttccatcgaaaaaatgggagcagcacgagttaatgccatgctttcctgcctgttcgacgattttgagcttgctatgattggcaaggctcaaactaattattacaatgataactcacttaaattgaacatgccattttacgcttactatgacatgttcaaaaagcagcaacttctaaaatggcttaaaaataaccgtgatgatatcatctgcggaactggtagaatgtacacttcaagaggtagttacattgctaacgcttatttagaggtagcgttagaatcaagcttgcttggtagtggctcttacatgcttcaaatgaggttcaaagactattcaaaaagtcaagaacctattccatctggtcgtcagaatcgacttgaatggattgagagcaacttggaaaatattcgataa

SEQ ID NO: 58 - protein, 183 aa, Bacteriophage D3577
MKINNDIKELILEYAKRYFKFENDFYKLPDIKFTDANWQKFKNGETSIEKMGAARVNAMLSCLFDDFELAMIGKAQTNYYNDNSLKLNMPFYAYYDMFKKQQLLKWLKNNRDDIICGTGRMYTSRGSYIANAYLEVALESSLLGSGSYMLQMRFKDYSKSQEPIPSGRQNRLEWIESNLENIR

SEQ ID NO: 59 - DNA, 552 bp, Bacteriophage CHPC577
atgaaaataaacaacgatatcaaagagctaattttggaatatggaagtcgctattttaaatttgaaaacgacttctacaaactgcctggcatcaagttcactgatgctaattggcaaaaattcaaaaatggtgatactttaatcgaaaaaatgggggcagcacgagtaaatgccatgcttgactgcctgttcgacgattttgagcttgctatgattggcaaggctcaaactaattattacaatgataattccttgaaattgaacatgccattttacgcttactatgacatgttcaaaaagcaacagcttatacattggctcaaaaacaaccgtgatgacatcgtaggcggaactggtagactgtacacttcaagcggtagttacattgctaacgcttatttagaaattgcattagaatcgagctcgcttggtagtggctcttacatgcttcaaatgagattcaaaaactattcaaaaagtcaagaacctattccatctggtcgccagaatcgacttgaatggattgaaaacaatcttgagaatattcgataa

SEQ ID NO: 60 - protein, 183 aa, Bacteriophage CHPC577
MKINNDIKELILEYGSRYFKFENDFYKLPGIKFTDANWQKFKNGDTLIEKMGAARVNAMLDCLFDDFELAMIGKAQTNYYNDNSLKLNMPFYAYYDMFKKQQLIHWLKNNRDDIVGGTGRLYTSSGSYIANAYLEIALESSSLGSGSYMLQMRFKNYSKSQEPIPSGRQNRLEWIENNLENIR

SEQ ID NO: 61 - DNA, 552 bp, Bacteriophage D4237
atgaaaataaataacgacatcaaagaattaattttagaatatatgagccgttacttcaaattcgaaaacgacttctacaaattgccagacatcaagttcacagatgctaattggcaaaaatttaagaatggagaaacttcaatcgaaaaaatgggagcagcacgagttaatgccatgctcaactgcctattcgaagattttgagcttgctatgattggcaaggctcaaattaattattacaatgataactcacttaaaatgaacatgccattttacgcttactatgatatgttcaaaaaacaacagcttctaaaatggcttaaagatcaccatgatgacatcatcggaggagctggcagaatgtacacatcaaccggtagttacattgctaatgcttatttagaggtagcgttagaatcaagctcgcttggtgatggtgagtacatgttgcaaatgcgttttaaaaattattcacgaagtcaagaacctattccgtcaggtcgcaaaaaccgacttgagtggattgaaaacaatctggaaaatattcgataa

SEQ ID NO: 62 - protein, 183 aa, Bacteriophage D4237
MKINNDIKELILEYMSRYFKFENDFYKLPDIKFTDANWQKFKNGETSIEKMGAARVNAMLNCLFEDFELAMIGKAQINYYNDNSLKMNMPFYAYYDMFKKQQLLKWLKDHHDDIIGGAGRMYTSTGSYIANAYLEVALESSSLGDGEYMLQMRFKNYSRSQEPIPSGRKNRLEWIENNLENIR

SEQ ID NO: 63 - DNA, 552 bp, Bacteriophage 9874
atgaaaataaatgacgacatcaaagaattaattttagaatatatgagccgttacttcaaattcgagaacgacttctacaaattgcctgacatcaaattcactgatgccaactggcaaaaattcaaaaatggagatacttccatcgagaagatgggggcagcacgagtaaatgccatgcttgactgcctattcgaagatttcgaacttgccatgattggcaaggctcaacaagaatactatttggataattcactaaagatgaacatgccattttacgcttattatgatatgttcaagaaaaaacagctcgtcaaatggcttaaagatcaccatgatgacatcctaggcggaactggtaggatgtacacttcagacggtagttacattgctaactcttatttagaggtagcgttagaatctagccgtctgggtagtggctcttacatgcttcaaatgagattcaaagactattcaagaagtcaagaacccattccgtcaggtcgcaaaaaccgacttgagtggattgaaaacaatctggaaaatattcgataa

SEQ ID NO: 64 - protein, 183 aa, Bacteriophage 9874
MKINDDIKELILEYMSRYFKFENDFYKLPDIKFTDANWQKFKNGDTSIEKMGAARVNAMLDCLFEDFELAMIGKAQQEYYLDNSLKMNMPFYAYYDMFKKKQLVKWLKDHHDDILGGTGRMYTSDGSYIANSYLEVALESSRLGSGSYMLQMRFKDYSRSQEPIPSGRKNRLEWIENNLENIR

SEQ ID NO: 65 - DNA, 552 bp, Bacteriophage 5093
atggaaatcaacaacgatatcaaagagttaattttggaatacgtgaaaagatacttcaagttcgagaacgacttctacaaattgcctgacatcaaattcactgatgccaactggcagaagttcaaaaatggcgaaacagccattgagaagatgggggcagcacgagtaaacgcaatgctcgactgcctattcgaagattttgagcttgccatgattggcaaggctcaaactaattattatattgataactcgcttaaattaaacatgccattttatgcttactatgatatgtttaagaaacaacagctcgtcaaatggcttgaaactagtcgtgaagacatcatcggaggggctggcagaatgtacacttcagacggtagttacattgctaacgcttatttagaagtagcgttagaatcaagctcgcttggtgatagtgaatacatgttgcaaatgcgttttaaaaattattcaaaaagtcaagaacctattccgtctggtcgtcaaaatagactggaatggattgaaaacaatcttaaaaacattcgataa

SEQ ID NO: 66 - protein, 183 aa, Bacteriophage 5093
MEINNDIKELILEYVKRYFKFENDFYKLPDIKFTDANWQKFKNGETAIEKMGAARVNAMLDCLFEDFELAMIGKAQTNYYIDNSLKLNMPFYAYYDMFKKQQLVKWLETSREDIIGGAGRMYTSDGSYIANAYLEVALESSSLGDSEYMLQMRFKNYSKSQEPIPSGRQNRLEWIENNLKNIR

SEQ ID NO: 67 - DNA, 552 bp, Bacteriophage D4154
atgctaataaataacgacatcaaagagttgattttggaatacgtcaaacgctattttaaatatgaaaatgacttctacagattgccgggcatcaagtttaccgatgcaaattggcagaagtttaaaaatggcgacacttccatcgagaagatgggggcagcacgagtaaacgccatgctcgactgcctattcgaagattttgagcttgccatgattggtaaggctcaaaccaattattatatcaataattcattgaaaatgaatatgccgttttacgcttactatgatatgttcaagaaggaacagcttatgaaatggcttgaaaccagccgtgaagacatcataggcggaactggcaggatgtacacttcagacggtagttacattgctaacgcttatttggaaattgcattagaatcgagctcgcttggtagtggctcttacatgcttcaaatgcgttttaaagattattcaaaaggtcaagagcctatcccgtctggtcgtcaaaaccgacttgagtggattgaaaacaatcttgaaaacattcgataa

SEQ ID NO: 68 - protein, 183 aa, Bacteriophage D4154
MLINNDIKELILEYVKRYFKYENDFYRLPGIKFTDANWQKFKNGDTSIEKMGAARVNAMLDCLFEDFELAMIGKAQTNYYINNSLKMNMPFYAYYDMFKKEQLMKWLETSREDIIGGTGRMYTSDGSYIANAYLEIALESSSLGSGSYMLQMRFKDYSKGQEPIPSGRQNRLEWIENNLENIR

SEQ ID NO: 69 - DNA, 552 bp, Streptococcus thermophilus
atgctaataaataacgacatcaaagagttgattttggaatacgtcaaacgctattttaaatttgaaaatgacttctacagattgccgggcatcaagtttaccgatgcaaattggcagaagtttaaaaatggcgacactgccattgagaagatgggggcatcacgagtaaactctatgcttgactgcctgttcgaagattttgagcttgctatgattggcaaggctcaagatgaatactatttggataattcactaaagatgaacatgccattttacgcttattatgatatgttcaagaaaaaacagctcgtcaaatggcttaaagatcaccatgatgacatcctaggcggaactggtaggatgtatacttcaagcggcaattacattgctaacgcttatttagaggtagcgttagaatcaagctcgcttggtagtggctcttacatgattcaaatgcgttttaaaaattattcaaaaggtcaagagcctatcccgtctggtcgtcaaaaccgacttgagtggattgaaaaaaacttggagaacattcgataa

SEQ ID NO: 70 - protein, 183 aa, Streptococcus thermophilus
MLINNDIKELILEYVKRYFKFENDFYRLPGIKFTDANWQKFKNGDTAIEKMGASRVNSMLDCLFEDFELAMIGKAQDEYYLDNSLKMNMPFYAYYDMFKKKQLVKWLKDHHDDILGGTGRMYTSSGNYIANAYLEVALESSSLGSGSYMIQMRFKNYSKGQEPIPSGRQNRLEWIEKNLENIR

SEQ ID NO: 71 - DNA, 552 bp, Streptococcus thermophilus
atggaaatcaacaacgatattaaacaactgatcttggaatacgctaaacgttatttcaagtttgagaacgacttttataaactgccaggcatcaagttcactgatgcaaattggcagaagttcaaaaatggaggcactgccattgagaagatgggggcagcacgagtaaacgccatgctcgactgcctattcgaagatttcgagcttgcaatgattggcaaggctcaacaagaatactattcggataattccttgaaagtaaatatggcattctatgcttattacgatcaattcaaaaaacaacagcttatgaaatggcttaaagataatcacgatgacatcataggagggactggtagaatgtacacgtcaagcggtagttacattgctaacgcttatttagaaattgcgttagaatctagccgtctgggtggtggttcttacatgatccaaatgaggtttaaagactattcaaaaggtcaagaacctattccgtctggtcgtcagaatcgacttgaatggattgagagcaacttggaaaacattcgataa

SEQ ID NO: 72 - protein, 183 aa, Streptococcus thermophilus
MEINNDIKQLILEYAKRYFKFENDFYKLPGIKFTDANWQKFKNGGTAIEKMGAARVNAMLDCLFEDFELAMIGKAQQEYYSDNSLKVNMAFYAYYDQFKKQQLMKWLKDNHDDIIGGTGRMYTSSGSYIANAYLEIALESSRLGGGSYMIQMRFKDYSKGQEPIPSGRQNRLEWIESNLENIR

SEQ ID NO: 73 - DNA, 552 bp, Bacteriophage Sfi19
atggaaatcaacaacgacattaaacaactgatcttggaatacgtgggacgctattttaaatttgaaaatgacttctacaaattgcccggcatcaaattcactgatgccaattggcagaagttcaaaaatggcgatacttccatcgaaaagatgggagcagcacgagtaaacgcaatgcttgactgcctgttcgaagatttcgaacttgccatgattggcaaggctcaaactaattattatattgataattcccttaaattaaacatgccattttacgcttattatgatatgttcaagaaggaacagcttatgaaatggcttaaagatcaccatgatgacatcataggcggaactggtaggatgtacatttcaagcggtagctacattgctaacgcttatttggaaattgcactagaatcaagtacgcttggtggtggtgagtacatgttgcaaatgcgctttaaaaattattcacgaagccaagaacctattccatcaggtcgcaaaaatagacttgaatggattgaaaacaatcttgaaaacattcgataa

SEQ ID NO: 74 - protein, 183 aa, Bacteriophage Sfi19
MEINNDIKQLILEYVGRYFKFENDFYKLPGIKFTDANWQKFKNGDTSIEKMGAARVNAMLDCLFEDFELAMIGKAQTNYYIDNSLKLNMPFYAYYDMFKKEQLMKWLKDHHDDIIGGTGRMYISSGSYIANAYLEIALESSTLGGGEYMLQMRFKNYSRSQEPIPSGRKNRLEWIENNLENIR

SEQ ID NO: 75 - DNA, 552 bp, Bacteriophage Sfi11
atggaaatcaacaacgacattaaacaactgatcttggaatacgtgggacgctattttaaatttgaaaatgacttctacaaattgcccggcatcaaattcactgatgccaattggcagaagttcaaaaatggcgatacttccatcgaaaagatgggagcagcacgagtaaacgcaatgcttgactgcctgttcgaagatttcgaacttgccatgattggcaaggctcaaactaattattatattgataattcccttaaattaaacatgccattttacgcttattatgatatgttcaagaaggaacagcttatgaaatggcttaaagatcaccatgatgacatcataggcggaactggtaggatgtacacttcaagcggtagctacattgctaacgcttatttggaaattgcactagaatcaagtacgcttggtggtggtgagtacatgttgcaaatgcgctttaaaaattattcacgaagccaagaacctattccatcaggtcgcaaaaatagacttgaatggattgaaaacaatcttgaaaacattcgataa

SEQ ID NO: 76 - protein, 183 aa, Bacteriophage Sfi11
MEINNDIKQLILEYVGRYFKFENDFYKLPGIKFTDANWQKFKNGDTSIEKMGAARVNAMLDCLFEDFELAMIGKAQTNYYIDNSLKLNMPFYAYYDMFKKEQLMKWLKDHHDDIIGGTGRMYTSSGSYIANAYLEIALESSTLGGGEYMLQMRFKNYSRSQEPIPSGRKNRLEWIENNLENIR

SEQ ID NO: 77 - DNA, 552 bp, Streptococcus thermophilus
atggaaatcaacaaagacatcaaagagttgattttggaatacgtcaaacgctattttaaatttgaaaatgatttctacagattgccgggcatcaagtttaccgatgccaactggcaaaaattcaagaatggagatacttccatcgagaagatgggggcagcacgagtaaacgccatgcttgactgcctgttcgaagatttcgaacttgctatgattggcaaggctcaagatgaatactatttggataattcacttaagtttaatatggcattccatacttattacgatcaatttaaaaaacaacagcttatgaaatggcttgaaactagcctcgaagacatcataggcggaactggtaggatgtacacttcaagcggtagttacattgctaacgcttatttggaaattgcactagaatcaagctcgcttggtggtggtgagtacatgttgcaaatgcgttttaaaaattattcacgaagccaagaacctattccgtcaggtcgcaaaaaccgacttgagtggattgaaaacaatctggaaaatatccgataa

SEQ ID NO: 78 - protein, 183 aa, Streptococcus thermophilus
MEINKDIKELILEYVKRYFKFENDFYRLPGIKFTDANWQKFKNGDTSIEKMGAARVNAMLDCLFEDFELAMIGKAQDEYYLDNSLKFNMAFHTYYDQFKKQQLMKWLETSLEDIIGGTGRMYTSSGSYIANAYLEIALESSSLGGGEYMLQMRFKNYSRSQEPIPSGRKNRLEWIENNLENIR

SEQ ID NO: 79 - DNA, 552 bp, Bacteriophage D4769
atgaaaatcaataatgacatcaaagagctaattttggaatatgtaagtcgctattttaaatttgaaaacgacttctacaaattacctggcatcaaattcactgatgccaactggcaaaaattcaagaatggagatacttccatcgagaagatgggggcagcacgagtaaacgccatgcttgactgcctgttcgaagatttcgaacttgctatgattggcaaggctcaagatgaatactatttggataattcacttaagtttaatatggcattccatacttattacgatcaatttaaaaaacaacagcttatgaaatggcttgaaactagcctcgaagacatcataggcggaactggtaggatgtacacttcaagcggtagttacattgctaacgcttatttggaaattgcactagaatcaagctcgcttggtggtggtgagtacatgttgcaaatgcgttttaaaaattattcacgaagccaagaacctattccgtcaggtcgcaaaaaccgacttgagtggattgaaaacaatctggaaaatatccgataa

SEQ ID NO: 80 - protein, 183 aa, Bacteriophage D4769
MKINNDIKELILEYVSRYFKFENDFYKLPGIKFTDANWQKFKNGDTSIEKMGAARVNAMLDCLFEDFELAMIGKAQDEYYLDNSLKFNMAFHTYYDQFKKQQLMKWLETSLEDIIGGTGRMYTSSGSYIANAYLEIALESSSLGGGEYMLQMRFKNYSRSQEPIPSGRKNRLEWIENNLENIR

SEQ ID NO: 81 - DNA, 552 bp, Bacteriophage D5691
atgattataaatattgatatcaaggaattgattttagagtatatgagtagatacttcaaatttgaaaatgatttctacaaactccccggcatcaaattcactgatgccaattggcaaaaatttaagaatggtgacacttccatcgaaaagatgggagcggctcgagtaaatgccatgctcgactgtctattcgatgactttgaacttgctatgattggcaaggctcaaattaattattacatagacaattcccttaaattgaacatgccattctatgcttattatgacatgttcaaaaaacaacaactgatcaaatggattgaaaccagccgtgatgatgtcatcggaggaactggcaggatgtatacagcaagcggaagctacatagctaacgcttatctagaaatagcactagaatctagctctctgggtggtggctcttatatgcttcaaatgagattcaaaaactactcacgaagccaagagccaataccatctggtcggaaaaaccgacttgagtggattgagagcaacttggaaaacattagataa

SEQ ID NO: 82 - protein, 183 aa, Bacteriophage D5691
MIINIDIKELILEYMSRYFKFENDFYKLPGIKFTDANWQKFKNGDTSIEKMGAARVNAMLDCLFDDFELAMIGKAQINYYIDNSLKLNMPFYAYYDMFKKQQLIKWIETSRDDVIGGTGRMYTASGSYIANAYLEIALESSSLGGGSYMLQMRFKNYSRSQEPIPSGRKNRLEWIESNLENIR

SEQ ID NO: 83 - DNA, 552 bp, Streptococcus sp.
atggaaatcaacaatgacatcaaagagttaatcttggaatacgtgggacgctatttcaagtttgaaaatgatttttacaaattgccgggcatcaaatttaccgatgcaaattggcaaaaattcaaaaacggtgatacatccatcgagaaaatgggggcggcacgagtaaacgcaatgctcgactgcctattcgatgatttcgagcttgctatgattggcaaggctcaaactgattattacattgataactcacttaaattgaacatgccattttatgcttattatgacatgttcaaaaaacaacagcttctaaaatggattgagaatagtcgtgaagacatcatcggaggggctggcagaatgtacacagcgggcggtaattggatttctagcgcttatttagagatcgcattagaatctagttccatcggtggcggtggctatatgcttcaaatgcggttcaaaaactactcaagagaccctagaccgattccagcaggccaccaaaatcgtctcgaatggattgaaaacaacttggagaatatccgataa

SEQ ID NO: 84 - protein, 183 aa, Streptococcus sp.
MEINNDIKELILEYVGRYFKFENDFYKLPGIKFTDANWQKFKNGDTSIEKMGAARVNAMLDCLFDDFELAMIGKAQTDYYIDNSLKLNMPFYAYYDMFKKQQLLKWIENSREDIIGGAGRMYTAGGNWISSAYLEIALESSSIGGGGYMLQMRFKNYSRDPRPIPAGHQNRLEWIENNLENIR

SEQ ID NO: 85 - DNA, 552 bp, Streptococcus sp.
atggaaatcaacaatgacatcaaggacctaattttagaatacgtaggacgatattttcgatttgaaaacgacttctacaaacttcccagaatcaagtttaccgattccaattggcaaaaattcaagaacggtgacacttccatcgaaaaaatgggagctggcagagtgaacgcaatgctcgattgtctatttgatgattttgagcttgctatgattggtaaggctcaaaccgattactacatggacaattctttaaagatgaatatgccattttatgcctattatgaccaatttaagaaacagcaactattgaaatggatcgagaatagtagagaggatatcataggcggtgctggcagaatgtacacagctagtgggaattggatttctagtgcctatttagaaattgcattggaatccagctcgttaggtggtggtgagtacatgttgcaaatgcgtttcaaagactactcacgaagccaagagccgataccagcaggccgccagaatcgacttgagtggattgagaataatttggagaatattcgataa

SEQ ID NO: 86 - protein, 183 aa, Streptococcus sp.
MEINNDIKDLILEYVGRYFRFENDFYKLPRIKFTDSNWQKFKNGDTSIEKMGAGRVNAMLDCLFDDFELAMIGKAQTDYYMDNSLKMNMPFYAYYDQFKKQQLLKWIENSREDIIGGAGRMYTASGNWISSAYLEIALESSSLGGGEYMLQMRFKDYSRSQEPIPAGRQNRLEWIENNLENIR

SEQ ID NO: 87 - DNA, 315 bp, Bacteriophage D4252
atgaaaaaagctaaacaactactcaaagaaattaaaaccaataatgtatcatacgcaattatggacgaggataatgaaatttattgcaacaaggaaactaacaacatcatggatatttatgaatatgataatgaaaatggccatttctatggtgtttatagtgacgttgttggtggtaaagttgatagtagatacttatctgacgaatatattttgaaagctatcgataaattgctaaatttaggcgatcccgtgaaacgcactgaactacctgcggacgctgatttcaaacgcacattcttttttgaagaataa

SEQ ID NO: 88 - protein, 104 aa, Bacteriophage D4252
MKKAKQLLKEIKTNNVSYAIMDEDNEIYCNKETNNIMDIYEYDNENGHFYGVYSDVVGGKVDSRYLSDEYILKAIDKLLNLGDPVKRTELPADADFKRTFFFEE

SEQ ID NO: 89 - DNA, 315 bp, Bacteriophage D802
atgaaaaaagctcaacaactgctcaaagaaattaaaaacactaatgtatcatacgcaattatggacgaggataatgaaatttattgcaacaaggaaactaacaacatcatggatatttatggatatgataatgaaaatggccatttctatggtgtttatagtgacgttgttggtggtaaagttgatagtagatacttatctgacgaatatattttgaaagctatcgataaattgctattcctaggcgaccctataaaacgaacagatctaccttcggacgctgatttcaaacgcacattcttttttgaagaataa

SEQ ID NO: 90 - protein, 104 aa, Bacteriophage D802
MKKAQQLLKEIKNTNVSYAIMDEDNEIYCNKETNNIMDIYGYDNENGHFYGVYSDVVGGKVDSRYLSDEYILKAIDKLLFLGDPIKRTDLPSDADFKRTFFFEE

SEQ ID NO: 91 - DNA, 291 bp, Bacteriophage P9874
atgaaaaacagacttttgggttctcgatatactgacgcgatcaaaaacgattgcggaacagccaataaaatgtcgaatatttacaataaattgaacaaagatagtttgcgagaaatccatagtgcactatatggcctattaacagctggatacgacattagtaacatgcgaaacatcgaagatttagaaaaatatgtgaatttaaaaaaatcacgtggccaactattaaatgtttcgagcgatgatattaagctataccataaattatttgtcatcagatttgaaaaatag

SEQ ID NO: 92 - protein, 96 aa, Bacteriophage P9874
MKNRLLGSRYTDAIKNDCGTANKMSNIYNKLNKDSLREIHSALYGLLTAGYDISNMRNIEDLEKYVNLKKSRGQLLNVSSDDIKLYHKLFVIRFEK

SEQ ID NO: 93 - DNA, 279 bp, Bacteriophage CHPC577
atgaaaaacaaactttatactgacgcaatcaaaaacgattccagaacagccagtaaaatggcgaacatttacaataaattggaaagcgatactatgcgagaaatccatagtgcactatctggcctattaacggctggatacgacattagtaacatgcgaaacatcgaagagttagaaaaatatgtgactttaaaaaaatcacgtggccaactattaaatgtctctagcgaagacattaaattgtaccataaattatttgtcatcaggtttggcaaatag

SEQ ID NO: 94 - protein, 92 aa, Bacteriophage CHPC577
MKNKLYTDAIKNDSRTASKMANIYNKLESDTMREIHSALSGLLTAGYDISNMRNIEELEKYVTLKKSRGQLLNVSSEDIKLYHKLFVIRFGK

SEQ ID NO: 95 - DNA, 297 bp, Bacteriophage D1297
atgaaaaacagacttttgggttctcgatatactgacgcgatcaaaaacgattgcggaacagccaataaaatgtcgaatatttacaataaattgaacaaagatagtttgcgagaaattcatagtgcactatatggcctattaacagctggttacgacattagtaacatgcgaaaaatagaagagttagaaaaatatgtgaatttaaaaaaatcacgtggccaactattaaatgtttctagcaacgatattaagctataccataaattatttgtcatcagatttggaaaagagaggtaa

SEQ ID NO: 96 - protein, 98 aa, Bacteriophage D1297
MKNRLLGSRYTDAIKNDCGTANKMSNIYNKLNKDSLREIHSALYGLLTAGYDISNMRKIEELEKYVNLKKSRGQLLNVSSNDIKLYHKLFVIRFGKER

SEQ ID NO: 97 - DNA, 285 bp, Bacteriophage D2759
atgaaaaacagactatatactgacgcgatcaaaaacgattgcggaacagccaataaaatgtcgaatatttacaataaattgaacaaagatagtttgcgagaaattcatagtgcactatatggcctattaacagctggttacgacattagtaacatgcgaaaaatagaagagttagaaaaatatgtgaatttaaaaaaatcacgtggccaactattaaatgtttctagcaacgatattaagctataccataaattatttgtcatcagatttggaaaagagaggtaa

SEQ ID NO: 98 - protein, 94 aa, Bacteriophage D2759
MKNRLYTDAIKNDCGTANKMSNIYNKLNKDSLREIHSALYGLLTAGYDISNMRKIEELEKYVNLKKSRGQLLNVSSNDIKLYHKLFVIRFGKER

SEQ ID NO: 99 - DNA, 279 bp, Bacteriophage D3577
atgaaaaacaaactttatactgacgcaatcaaaaacgattccgcaacagccaataaaatggcgaatatttatagcaagctaaacaaagatagtttgcgagaaatccatagtgcactatctggcctattaacggctggatacgacattagtaacatgcaaaacatcgcagagttacaaaaatatgtgattttaaaaaaatcacgggggcaactattaaatgtctctagcaaagacattgaactgtatcataaattatttgtcatcagatttggaaaataa

SEQ ID NO: 100 - protein, 92 aa, Bacteriophage D3577
MKNKLYTDAIKNDSATANKMANIYSKLNKDSLREIHSALSGLLTAGYDISNMQNIAELQKYVILKKSRGQLLNVSSKDIELYHKLFVIRFGK

SEQ ID NO: 101 - DNA, 291 bp, Bacteriophage D4741
atgaaaaacagacttttgggttctcgatatactgacgcgatcaaaaacgattgcggaacagccaataaaatgtcgaatatttacaataaattgaacaaagatagtttgcgagaaattcatagtgcactatatggcctattaacagctggttacgacattagtaacatgcgaaaaatagaagagttagaaaaatatgtgaatttaaaaaaatcacgtggccaactattaaatgtttctagcaacgatattaagctataccataaattatttgtcatcagatttggaaaatag

SEQ ID NO: 102 - protein, 96 aa, Bacteriophage D4741
MKNRLLGSRYTDAIKNDCGTANKMSNIYNKLNKDSLREIHSALYGLLTAGYDISNMRKIEELEKYVNLKKSRGQLLNVSSNDIKLYHKLFVIRFGK

SEQ ID NO: 103 - DNA, 285 bp, Bacteriophage D4419
atgaaaaacagacttttgggttctcgatatactgacgcgatcaaaaacgattgcggaacagccaataaaatgtcgaatatttacaataaattgaacaaagatagtttgcgagaaattcatagtgcactatatggcctattaacagctggttacgacattagtaacatgcgaaaaatagaagagttagaaaaatatgtgaatttatcacgtggccaactattaaatgtttctagcaacgatattaagctatatcataaattatttgtcatcagatttggaaaatag

SEQ ID NO: 104 - protein, 94 aa, Bacteriophage D4419
MKNRLLGSRYTDAIKNDCGTANKMSNIYNKLNKDSLREIHSALYGLLTAGYDISNMRKIEELEKYVNLSRGQLLNVSSNDIKLYHKLFVIRFGK

SEQ ID NO: 105 - DNA, 303 bp, Bacteriophage D5861
atgaaaaacagacttttgggttctcgatatactgacgcaatcaaaaacgattccggaacagccaataaaatgtctaatatttacaattcagtcataaacaaggaggggttgcgaggaatccatagtgcactatatggcctattaacagctggatacgacattagtaacatgcgaaaaatagaagagttagaaaaatatgtgaatttaaaaaaatcacgtggccaactattaaatgtttctagcagcgatattaagctataccataaattatttgtcatcagatttggaaaaaagttaaaataa

SEQ ID NO: 106 - protein, 100 aa, Bacteriophage D5861
MKNRLLGSRYTDAIKNDSGTANKMSNIYNSVINKEGLRGIHSALYGLLTAGYDISNMRKIEELEKYVNLKKSRGQLLNVSSSDIKLYHKLFVIRFGKKLK

SEQ ID NO: 107 - DNA, 297 bp, Bacteriophage D6252
atgaaaaatggtaacaaaattttaggttatcgatacactgatgagattaaaaacgattctgcaacagagaataaaatgtctaatctttataacaaattggacaaagatagtttacgagagatccatagtgcattatacggtctattaacagctggatatgatatcagcaacatgcgaaatgtcgaagaacttgaaaaatacgtgaacgttaaaaaatctcatggaaaattattagatgttactaatagtgacattcagttatatcataaattatttgttgttcgatttgggaagtag

SEQ ID NO: 108 - protein, 98 aa, Bacteriophage D6252
MKNGNKILGYRYTDEIKNDSATENKMSNLYNKLDKDSLREIHSALYGLLTAGYDISNMRNVEELEKYVNVKKSHGKLLDVTNSDIQLYHKLFVVRFGK

SEQ ID NO: 109 - DNA, 291 bp, Bacteriophage D7130
atgaaaaacagacttttgggttctcgatatactgacgcgatcaaaaacgattgcggaacagccaataaaatgtcgaatatttacaataaattgaacaaagatagtttgcgagaaatccatagtgcactatatggcctattaacagctggatacgacattagtaacatgcgaaacatcgaagagttagaaaaatatgtgaatttaaaaaaatcacgtggccaactattaaatgtttctagcagcgatattaagctataccataaattatttgtcatcagatttggaaaatag

SEQ ID NO: 110 - protein, 96 aa, Bacteriophage D7130
MKNRLLGSRYTDAIKNDCGTANKMSNIYNKLNKDSLREIHSALYGLLTAGYDISNMRNIEELEKYVNLKKSRGQLLNVSSSDIKLYHKLFVIRFGK

SEQ ID NO: 111 - DNA, 294 bp, Bacteriophage N1062
atgaaaaacagacttttgggttctcgatatactgacgcaatcaaaaacgattccggaacagccaataaaatgtctaatatttacaattcagtcataaacaaggaggggttgcgaggaatccatagtgcactatatggcctattaacagctggatacgacattagtaacatgcgaaaaatagaagagttagaaaaatatgtgaatttaaaaaaatcacgtggccaactattaaatgtttctagcagcgatattaagctataccataaattatttgtcatcagatttggaaaatag

SEQ ID NO: 112 - protein, 97 aa, Bacteriophage N1062
MKNRLLGSRYTDAIKNDSGTANKMSNIYNSVINKEGLRGIHSALYGLLTAGYDISNMRKIEELEKYVNLKKSRGQLLNVSSSDIKLYHKLFVIRFGK

SEQ ID NO: 113 - DNA, 294 bp, Bacteriophage N488
atgaaaaacagacttttgggttctcgatatactgacgcaatcaaaaacgattccggaacagccaataaaatgtctaatatttacaattcagtcataaacaaggaggggttgcgagaaatccatagtgcactatatggcctattaacagctggttacgacattagtaacatgcgaaaaatagaagagttagaaaaatatgtgaatttaaaaaaatcacgtggccaactattaaatgtgtctagcaatgatattaagctataccataaattatttgtcaccagatttggaaaataa

SEQ ID NO: 114 - protein, 97 aa, Bacteriophage N488
MKNRLLGSRYTDAIKNDSGTANKMSNIYNSVINKEGLREIHSALYGLLTAGYDISNMRKIEELEKYVNLKKSRGQLLNVSSNDIKLYHKLFVTRFGK

SEQ ID NO: 115 - DNA, 291 bp, Bacteriophage P5641
atgaaaaacagacttttgggttctcgatatactgacgcaatcaaaaacgattccggaacagccaataaaatgtcgaatatttacaataaattgaacaaagatagtttgcgagaaattcatagtgcactatatggcctattaacagctggttacgacattagtaacatgcgaaacatcgaagagttagaaaaatatgtgaatttaaaaaaatcacgtggccaactattaaatgttactagcaatgatattaagctataccataaattatttgtcatcagatttggaaaatag

SEQ ID NO: 116 - protein, 96 aa, Bacteriophage P5641
MKNRLLGSRYTDAIKNDSGTANKMSNIYNKLNKDSLREIHSALYGLLTAGYDISNMRNIEELEKYVNLKKSRGQLLNVTSNDIKLYHKLFVIRFGK

SEQ ID NO: 117 - DNA, 291 bp, Bacteriophage P7602
atgaaaaacagacttttgggttctcgatatactgacgcgatcaaaaacgattgcggaacagccaataaaatgtcgaatatttacaataaattgaacaaagatagtttgcgagagatccatagtgcactatatggcctattaacagctggatacgacattagtaacatgcgaaacatcgaagagttagaaaaatatgtgaatttaaaaaaatcacgtggccaactattaaatgtttcgagcgatgatattaagctataccataaattatttgtcatcagatttggaaaatag

SEQ ID NO: 118 - protein, 96 aa, Bacteriophage P7602
MKNRLLGSRYTDAIKNDCGTANKMSNIYNKLNKDSLREIHSALYGLLTAGYDISNMRNIEELEKYVNLKKSRGQLLNVSSDDIKLYHKLFVIRFGK

SEQ ID NO: 119 - DNA, 297 bp, Bacteriophage V442
atgaaaaatggtaacaaaattttaggttatcgatacactgatgagattaaaaacgattctgcaacagagaataaaatgtctaatctttataacaaattggacaaagatagtttacgagagatccatagtgcattatacggtctattaacagctggatatgatatcagcaacatgcgaaatgtcgaagaacttgaaaaatacgtgaacgttaaaaaatctcatggaaaattattagatgttactaatagtgacattcagttatatcataaattatttgttgttcgatttgggaggtaa

SEQ ID NO: 120 - protein, 98 aa, Bacteriophage V442
MKNGNKILGYRYTDEIKNDSATENKMSNLYNKLDKDSLREIHSALYGLLTAGYDISNMRNVEELEKYVNVKKSHGKLLDVTNSDIQLYHKLFVVRFGR

SEQ ID NO: 121 - DNA, 387 bp, Bacteriophage D4090
atgacagaatggaaaacaataaactttaatgcacaaaacattgaatacgaggcggcaaaagcaatcctcattaagatgccaaacaattctgaatggcacggttacactttctggcatccgtcaaaatgtgtgcgtacattaagcaagggtaatggttatttcaaaactttcagctatacagaaaattgggagtttaccattttcaaatcaaataaaaaaggggaaagaaccattgaacaagtacttacggcaagagatatggaaaaagcatttagtgtggtgaatgaacaaattgcaagtaatgcttcaacagaaagttaccttgaaattgaagaacctaaaaaggttgataaaacagttagtattaacaatgagttaaaacgttaa

SEQ ID NO: 122 - protein, 128 aa, Bacteriophage D4090
MTEWKTINFNAQNIEYEAAKAILIKMPNNSEWHGYTFWHPSKCVRTLSKGNGYFKTFSYTENWEFTIFKSNKKGERTIEQVLTARDMEKAFSVVNEQIASNASTESYLEIEEPKKVDKTVSINNELKR

SEQ ID NO: 123 - DNA, 387 bp, Bacteriophage D4254
atgacagaatggaaaacgattaattttaataaacaaaacattgaacatgaaacagcgaaagctgttctcattaagatgccaaataattctgaatggtacggctataaattctggcatccgtcaaaatgtgtgcgtacattaagcaagggcaatggttatttcaaaactttcagctatacagaaaattgggagtttaccattttcaaatcaaataaaaagggggaaagaaccgctgaacaaatacttacagcagaggatatggaaatagcttttgatgttgttaacgaacaaattagcgcgaacgcttcaacagaaagttatcttgaaattgaagaacctaaaaaggttgataaaacagttagtattaacaatgagttaaaacgttaa

SEQ ID NO: 124 - protein, 128 aa, Bacteriophage D4254
MTEWKTINFNKQNIEHETAKAVLIKMPNNSEWYGYKFWHPSKCVRTLSKGNGYFKTFSYTENWEFTIFKSNKKGERTAEQILTAEDMEIAFDVVNEQISANASTESYLEIEEPKKVDKTVSINNELKR

SEQ ID NO: 125 - DNA, 387 bp, Bacteriophage D4368
atgacagaatggaaaacaataaactttaatgcacaaaacattgaatacgaggcggcaaaagcaatcctcattaagatgccaaacaattctgaatggcacggttacactttctggcatccgtcaaaatgtgtgcgtacattaagcaagggtaatggttatttcaaaactttcagctatacagaaaattgggagtttaccattttcaaatcaaataaaaagggggaaagaaccgctgaacaaatacttacagcagaggatatggaaatagcttttgatgttgttaacgaacaaatcagtgtagacgcttcgacagaaagttaccttgaaatcgaagagcctaaaaaggttgataaaacagttagtattaacaatgaattaaaacgttaa

SEQ ID NO: 126 - protein, 128 aa, Bacteriophage D4368
MTEWKTINFNAQNIEYEAAKAILIKMPNNSEWHGYTFWHPSKCVRTLSKGNGYFKTFSYTENWEFTIFKSNKKGERTAEQILTAEDMEIAFDVVNEQISVDASTESYLEIEEPKKVDKTVSINNELKR

SEQ ID NO: 127 - DNA, 381 bp, Bacteriophage D4598
atgtggaaatcaatcaattttaacgcacaaaacatcgaacacgagacagcgaaagctgttctcattaagatgccaaataattctgaatggagtggttataaattttggcacccatctaaatgcgtccgtactctaagcaagggcaaaggctatttcaaaattttcagctatacagaaaattgggagtttaccattttcaaatcaaataaaaagggggaaagaaccgctgaacaaatacttacagcagaggatatggaaatagcttttgatgttgttaacgaacaaattagcgcgaacgcttcaacagaaagttatcttgaaattgaagaacctaaaaaggttgataaaacagttagtattaacaatgagttaaaacgttaa

SEQ ID NO: 128 - protein, 126 aa, Bacteriophage D4598
MWKSINFNAQNIEHETAKAVLIKMPNNSEWSGYKFWHPSKCVRTLSKGKGYFKIFSYTENWEFTIFKSNKKGERTAEQILTAEDMEIAFDVVNEQISANASTESYLEIEEPKKVDKTVSINNELKR

SEQ ID NO: 129 - DNA, 381 bp, Bacteriophage D5693
atgtggaaatcaatcaattttaacgcacaaaacatcgaacacgagacagcgaaagctgttctcattaagatgccaaataattctgaatggagtggttataaattttggcacccatctaaattcgtccgtactctaagcaagggcaaaggctatttcaaaattttcagctatacagaaaattgggagtttaccattttcaaatcaaataaaaagggggaaagaaccgctgaacaaatacttacagcagaggatatggaaatagcttttgatgttgttaacgaacaaattagcgcgaacgcttcaacagaaagttatcttgaaattgaagaacctaaaaaggttgataaaacagttagtattaacaatgagttaaaacgttaa

SEQ ID NO: 130 - protein, 126 aa, Bacteriophage D5693
MWKSINFNAQNIEHETAKAVLIKMPNNSEWSGYKFWHPSKFVRTLSKGKGYFKIFSYTENWEFTIFKSNKKGERTAEQILTAEDMEIAFDVVNEQISANASTESYLEIEEPKKVDKTVSINNELKR

SEQ ID NO: 131 - DNA, 381 bp, Bacteriophage D6961
atgtggaaatcaatcaattttaacgcacaaaacatcgaacacgagacagcgaaagctgttctcattaagatgccaaataattctgaatggagtggttataaattttggcactcatctaaatgcgtccgtactctaagcaagggcaaaggctatttccaaagtttcagctatacagaaaattgggagtttaccattttcaaatcaaataaaaaaggggaaagaaccgctgaacaaatacttacagcagaggatatggaaatagcttttgatgttgttaacgaacaaattagcgcgaacgcttcaacagaaagttatcttgaaattgaagaacctaaaaaggttgataaaacagttagtattaacaatgagttaaaacgttaa

SEQ ID NO: 132 - protein, 126 aa, Bacteriophage D6961
MWKSINFNAQNIEHETAKAVLIKMPNNSEWSGYKFWHSSKCVRTLSKGKGYFQSFSYTENWEFTIFKSNKKGERTAEQILTAEDMEIAFDVVNEQISANASTESYLEIEEPKKVDKTVSINNELKR

SEQ ID NO: 133 - DNA, 387 bp, Bacteriophage D7059
atgacagaatggaaaacgattaattttaataaacaaaacattgaacatgaaacagtgaaagctgttctcattaagatgccaaataattctgaatggtacggctataaattctggcatccgtcaaaatgtgtgcgtacattaagcaagggcaatggttatttcaaaactttcagctatacagaaaattgggagtttaccattttcaaatcaaataaaaagggggaaagaaccgctgaacaaatacttacagcagaggatatggaaatagcttttgatgttgttaacgaacaaattagcgcgaacgcttcaacagaaagttatcttgaaattgaagaacctaaaaaggttgataaaacagttagtattaacaatgagttaaaacgttaa

SEQ ID NO: 134 - protein, 128 aa, Bacteriophage D7059
MTEWKTINFNKQNIEHETVKAVLIKMPNNSEWYGYKFWHPSKCVRTLSKGNGYFKTFSYTENWEFTIFKSNKKGERTAEQILTAEDMEIAFDVVNEQISANASTESYLEIEEPKKVDKTVSINNELKR

SEQ ID NO: 135 - DNA, 372 bp, Bacteriophage D4250
atgtggaaatcaatcaaatttaacgcacagaacataaaatttgagactgcgaaagcagtattgattaaaatgccgaataagtctaggtatgctggatatatgttctggcatcctttaaaacttgtccgtgttgaaggcggaaaaggctactttatgagttttagctatacagatgattttgagtttaaggtttttaaacaaggtaaaaatcgtcaaatcaccgctgaatcaatattatcacacgaagaaattgaggaagcttttgaaattgtgaatgaacaattatcttatatggatgaatgctatctagaggttacagaacctactaaaattgataaagaggtagaggtcaaagaagaattgagaaagtaa

SEQ ID NO: 136 - protein, 123 aa, Bacteriophage D4250
MWKSIKFNAQNIKFETAKAVLIKMPNKSRYAGYMFWHPLKLVRVEGGKGYFMSFSYTDDFEFKVFKQGKNRQITAESILSHEEIEEAFEIVNEQLSYMDECYLEVTEPTKIDKEVEVKEELRK

SEQ ID NO: 137 - DNA, 372 bp, Bacteriophage D4252
atgtggaaatcaatcaaatttaatgcacaaaacatcaaattcgagacagcaaaagcagtcttgattaaaatgcccaataaatctaggtatgctgggtatatgttctggcatcctgcaaaactagtccgagtggtaggtggaaaaggttactttatgagttttagctatactgatgaatttgagtttaagatatttaaacaaggaaaaaatcgtcaaattactgttgaaaaaatcttatcacccgaagaaatagaagacgcttttgaagttgtgaacgaacaattatctgatatcgatgaatgctatttagaagtgacagaaccaactaaaattaatgataaggtagaaatcagagcagaattaagaaaataa

SEQ ID NO: 138 - protein, 123 aa, Bacteriophage D4252
MWKSIKFNAQNIKFETAKAVLIKMPNKSRYAGYMFWHPAKLVRVVGGKGYFMSFSYTDEFEFKIFKQGKNRQITVEKILSPEEIEDAFEVVNEQLSDIDECYLEVTEPTKINDKVEIRAELRK

SEQ ID NO: 139 - DNA, 372 bp, Bacteriophage D4276
atgtggaaatcaatcaaatttaacgcacagaacataaaattcgagactgcgaaagcagtattaattaaaatgccaaataaatctaggtatgctggatatatgttctggcatccttcaaaacttgtccgtgttgaaggcggaaaaggctactttatgagttttagctatacagatgattttgagtttaaggtttttaaacaaggtaaaaatcgtcaaatcaccgctgaatcaatattatcacacgaagaaattgaggaagcttttgaaattgtgaatgaacaattatcttatatggatgaatgctatctagaggttacagaacctactaaaattgataaagaggtagaggtcaaagaagaattgagaaagtaa

SEQ ID NO: 140 - protein, 123 aa, Bacteriophage D4276
MWKSIKFNAQNIKFETAKAVLIKMPNKSRYAGYMFWHPSKLVRVEGGKGYFMSFSYTDDFEFKVFKQGKNRQITAESILSHEEIEEAFEIVNEQLSYMDECYLEVTEPTKIDKEVEVKEELRK

SEQ ID NO: 141 - DNA, 372 bp, Bacteriophage D6938
atgtggaaatcaataaaatttaatgcacaaaacgtaaaattcgagactgcgaattcagttttgattaaaatgccgaataaatctagctatgctggatatatgttctggcaccctgcgaaactagttcgtgtgttaggtggcaaaggttactttttgagttttagctatacagatgaatttgagtttaaggtttttaagcaaggaaaaaatcgtcaaatcaccgctgaagcaatcttatcacacgaagaaatggaagacgcgtttgaaattgtgaatgagcatttgtcctatacagatgaatgctatctagaagttgcagaacctactaaaatcgataaagaggtagagatcagagaagaattgagaaagtaa

SEQ ID NO: 142 - protein, 123 aa, Bacteriophage D6938
MWKSIKFNAQNVKFETANSVLIKMPNKSSYAGYMFWHPAKLVRVLGGKGYFLSFSYTDEFEFKVFKQGKNRQITAEAILSHEEMEDAFEIVNEHLSYTDECYLEVAEPTKIDKEVEIREELRK

SEQ ID NO: 143 - DNA, 180 bp, Bacteriophage D1422
atgaaagtttattataatctagcagatagcggactcttcaaagaaatcaagaaacaactagctctggacgatgcggaaaacggcgatttaattcatacaacagaagacaacgaggcttcagatgggacaaaaatcgtcgcaatctggaacgcaaacagacaaaactattttataaagtaa

SEQ ID NO: 144 - protein, 59 aa, Bacteriophage D1422
MKVYYNLADSGLFKEIKKQLALDDAENGDLIHTTEDNEASDGTKIVAIWNANRQNYFIK

SEQ ID NO: 145 - DNA, 438 bp, Bacteriophage D1765
atgagaaacgattttattaataaagtttatgatgaattaaatcagattattaatcattgggctaaacaaaaatatttaagtgataagatttttgaatatactaatacttttagtattaagaaggtttatggactttattgggaagttaagattttatgtaagaatgattatcgaattttgttgagattttataaaaattatgagtggtataacgattctaatattttaaatgtatctgtattagcacctgcggtggaaagagttaaaaatgaagatggaagcgttgatgtttatccaagtaaaataattaaagataaaattgaatttattgaaggtgattttgatattgatggagatgattgggtagatgaagtgttggaatatataaataaatgggtaaataaagataaagctgatgtggaggtattagataaatga

SEQ ID NO: 146 - protein, 145 aa, Bacteriophage D1765
MRNDFINKVYDELNQIINHWAKQKYLSDKIFEYTNTFSIKKVYGLYWEVKILCKNDYRILLRFYKNYEWYNDSNILNVSVLAPAVERVKNEDGSVDVYPSKIIKDKIEFIEGDFDIDGDDWVDEVLEYINKWVNKDKADVEVLDK

SEQ ID NO: 147 - DNA, 438 bp, Bacteriophage D4212
atgagaaacgattttattaataaagtttatgatgaattaaatcagattattaatcattgggctaaacaaaaatatttaagtgataagatttttgaatatactaatacttttagtattaagaaggtttatggactttattgggaagttaagattttatgtaagaatgattatcgaattttgttgagattttataaaaattatgagtggtataacgattctaatattttaaatgtatctgtattagcacctgcggtggaaagagttaaaaatgaagatggaagcgttgatgtttatccaagtaaaaaaattaaagataaaattgaatttattgaaggtgattttgatattgatggagatgattgggtagatgaagtgttggaatatataaataaatgggtaaataaagataaagctgatgtggaggtattagataaatga

SEQ ID NO: 148 - protein, 145 aa, Bacteriophage D4212
MRNDFINKVYDELNQIINHWAKQKYLSDKIFEYTNTFSIKKVYGLYWEVKILCKNDYRILLRFYKNYEWYNDSNILNVSVLAPAVERVKNEDGSVDVYPSKKIKDKIEFIEGDFDIDGDDWVDEVLEYINKWVNKDKADVEVLDK

SEQ ID NO: 149 - DNA, 438 bp, Bacteriophage D4250
atgagaaacgattttattaataaagtttatgatgaattaaatcagattattaatcattgggctaaacaaaaatatttaagtgataagatttttgaatatactaatacttttagtattaagaaggtttatggactttattgggaagttaagattttatgtaagaatgattatcgaattttgttgagattttataaaaattatgagtggtataacgattctaatattttaaatgtatctgtattagcacctgcggtggaaagagttaaaaatgaagatggaagcgttgatgtttatccaagtaaaaaaattaaagataaaattgaatttattgaaggtaattttgatattgatggagatgattgggtagatgaagtgttggaatatataaataaatgggtaaataaagataaagctgatgtggaggtattagataaatga

SEQ ID NO: 150 - protein, 145 aa, Bacteriophage D4250
MRNDFINKVYDELNQIINHWAKQKYLSDKIFEYTNTFSIKKVYGLYWEVKILCKNDYRILLRFYKNYEWYNDSNILNVSVLAPAVERVKNEDGSVDVYPSKKIKDKIEFIEGNFDIDGDDWVDEVLEYINKWVNKDKADVEVLDK

SEQ ID NO: 151 - DNA, 366 bp, Bacteriophage D4287
atgagaaacgattttattaataaagtttatgatgaattaaatcagattattaatcattgggctaaacaaaaatatttaagtgataagatttttgaatatactaatacttttagtattaagaaggtttatggactttattgggaagttaagattttatgtaagaatgattatcgaattttgttgagattttataaaaattatgagtggtataacgattctaatattttaaatgtatctgtattagcacctgcggtggaaagagttaaaaatgaagatggaagcgttgatgtttatccaagtaaaaaattaaagataaaattgaatttattgaaggtgattttgatattgatggagatgattgggtag

SEQ ID NO: 152 - protein, 121 aa, Bacteriophage D4287
MRNDFINKVYDELNQIINHWAKQKYLSDKIFEYTNTFSIKKVYGLYWEVKILCKNDYRILLRFYKNYEWYNDSNILNVSVLAPAVERVKNEDGSVDVYPSKKLKIKLNLLKVILILMEMIG

SEQ ID NO: 153 - DNA, 438 bp, Bacteriophage D6252
atgagaaacgattttattaataaagtttatgatgaattaaatcagattattaatcattgggctaaacaaaaatatttaagtgataagatttttgaatatactaatacttttagtattaagaaggtttatggactttattgggaagttaagattttatgtaagaatgattatcgaattttgttgagattttataaaaattatgagtggtataacgattctaatattttaaatgtatctgtattagcacctgcggtggaaagagttgaaaatgaagatggaagcgttgatgtttatccaagtaaaataattaaagataaaattgaatttattgaaggtgattttgatatcgatggagatgattgggtagatgaagtgttggaatatataaataaatgggtaaataaagataaagctgatgtggaggtattagataaatga

SEQ ID NO: 154 - protein, 145 aa, Bacteriophage D6252
MRNDFINKVYDELNQIINHWAKQKYLSDKIFEYTNTFSIKKVYGLYWEVKILCKNDYRILLRFYKNYEWYNDSNILNVSVLAPAVERVENEDGSVDVYPSKIIKDKIEFIEGDFDIDGDDWVDEVLEYINKWVNKDKADVEVLDK

SEQ ID NO: 155 - DNA, 438 bp, Bacteriophage D6312
atgagaaacgattttattaataaagtttatgatgaattaaatccgattattaatcattgggctaaacaaaaatatttaagtgataagatttttgaatatactaatacttttagtattaagaaggtttatggactttattgggaagttaagattttatgtaagaatgattatcgaattttgttgagattttataaaaatcatgagtggtataatgattctaatattttaaatgtatctgtattagcacctgcggtggaaagagttaaacatgaagatggaagcgttgatgtttatccaagtaaaataattaaagataaaattgaatttattgaaggtgattttgatattgatggatatgattgggtagatgaagtgttggaatatataaataaatgggtaaataaagataaagatgatgtggaggtattagataagtga

SEQ ID NO: 156 - protein, 145 aa, Bacteriophage D6312
MRNDFINKVYDELNPIINHWAKQKYLSDKIFEYTNTFSIKKVYGLYWEVKILCKNDYRILLRFYKNHEWYNDSNILNVSVLAPAVERVKHEDGSVDVYPSKIIKDKIEFIEGDFDIDGYDWVDEVLEYINKWVNKDKDDVEVLDK

SEQ ID NO: 157 - DNA, 438 bp, Bacteriophage O1205
atgagaaacgattttattaataaagtctatgatgaattaaatcagattattaatcattgggctaaacaaaaatatttaagtgataagatttttgaatatactaatacttttagtattaagaaggtttatggactctattgggaagttaagattttatgtaagaatgattatcgaattttgttgagattttataaaaattatgagtggtataatgattctaatattttaaatgtatctgtattagcacctgcggtggaaagagttaaaaatgaagatggaagcgttgatgtttatccaagtaaaataattaaagataaaattgaatttattgaaggtaattttgatattgatggagatgattgggtagatgaagtgttggaatatataaataaatgggtaaataaagataaagctgatgtggaggtattagataaatga

SEQ ID NO: 158 - protein, 145 aa, Bacteriophage O1205
MRNDFINKVYDELNQIINHWAKQKYLSDKIFEYTNTFSIKKVYGLYWEVKILCKNDYRILLRFYKNYEWYNDSNILNVSVLAPAVERVKNEDGSVDVYPSKIIKDKIEFIEGNFDIDGDDWVDEVLEYINKWVNKDKADVEVLDK

SEQ ID NO: 159 - DNA, 318 bp, Bacteriophage D4769
atgaaaaatttcaaaataagctctacttatagagctgcacgaaaacagcagaaaactgctaatcgtaaatcgttttataacgatgagggctacatgatcagcccaagtgaatgggctgatggagtcattaaggggcttataaaccctaaaaactcttggtcaaatgaccatgtgaaagggtacctccctagagtttccccacgtagccattggacaaagaatggttatagggagtaccttggtattggtaaatcaagggatatccctgaaaaagagcctgaagttatcgagatgatggatctcgagttagttccttaa

SEQ ID NO: 160 - protein, 105 aa, Bacteriophage D4769
MKNFKISSTYRAARKQQKTANRKSFYNDEGYMISPSEWADGVIKGLINPKNSWSNDHVKGYLPRVSPRSHWTKNGYREYLGIGKSRDIPEKEPEVIEMMDLELVP

SEQ ID NO: 161 - DNA, 318 bp, Bacteriophage P7633
atgaaaaatttcaaaataagctctacttatagagctgcacgaaaacagcagaaaactgctaatcgtaaatcgttttataacgatgagggctacatgatcagcccaagtgaatgggttgatggagtcattaaggggcttataaaccctaaaaactcttggtcaaatgaccatgtgaaagggtacctccctagagtttccccacgtagccattggacaaagaatggttatagggagtaccttggtattggtaaatcaagggatatccctgaaaaagagcctgaagttatcgagatgatggatctcgagttagttccttaa

SEQ ID NO: 162 - protein, 105 aa, Bacteriophage P7633
MKNFKISSTYRAARKQQKTANRKSFYNDEGYMISPSEWVDGVIKGLINPKNSWSNDHVKGYLPRVSPRSHWTKNGYREYLGIGKSRDIPEKEPEVIEMMDLELVP

SEQ ID NO: 163 - DNA, 318 bp, Bacteriophage Proph1
atgaaaaatttcaaaataagctctacttatagagctgcacgaaaacagcagaaaactgctaatcgtaaatcgttttataacgatgagggctacatgatcagcccaagtgaatgggctgatggagtcattaaggggcttataaaccctaaaaactcttggtcaaatgaccatgtgaaagggtacctccctagagtttccccacgtagccattggacaaagaatggttatagggagtaccttggtattggtaaatcaagggatatccctaaaaaagagcctgaagttatcgagatgatggatctcgagttagttccttaa

SEQ ID NO: 164 - protein, 105 aa, Bacteriophage Proph1
MKNFKISSTYRAARKQQKTANRKSFYNDEGYMISPSEWADGVIKGLINPKNSWSNDHVKGYLPRVSPRSHWTKNGYREYLGIGKSRDIPKKEPEVIEMMDLELVP

SEQ ID NO: 165 - DNA, 387 bp, Bacteriophage D5691
atgaaatatgataagtcaggaatcatgaaagaagcttggaacttatttaataatgatgacatcacttttgcagactttgaatatctcactcgtgaagaacgccaaggtaaaaaaacatttactctttgcttgaaagaagcttgggcacacgaaaaagaaattgttgacagcatcaaaaaagaccacgctgatgctgaacattcagtggaagcaaaagcttgggattgggcttgtaaaaaattaggtgtctctattgaaatggatgcttacacaaaattcgttaacgttaacgatatgaaaaaagaagcatggcctggaacaagcgtttggtcattggctatgcgtgcggttaaactacatatcaaactttttggtcaagtagcttaa

SEQ ID NO: 166 - protein, 128 aa, Bacteriophage D5691
MKYDKSGIMKEAWNLFNNDDITFADFEYLTREERQGKKTFTLCLKEAWAHEKEIVDSIKKDHADAEHSVEAKAWDWACKKLGVSIEMDAYTKFVNVNDMKKEAWPGTSVWSLAMRAVKLHIKLFGQVA

SEQ ID NO: 167 - DNA, 522 bp, Bacteriophage D6252
ttgaatggattaaaaacaatcttgaaaacattcgataaaaacatatattttttaaccaaaagtgttgacatacgtcaacataggagatataatatatatgtaaagttaagagaggaagtaaatgacatgaaaaaatcaacatacgacaaatcaggaattatgaaagaagcttggaatttatttaataacgatgacatcactactgcagattttgaatatctcactcgtggagaattgcaagaaggaaaaacatttgctatttgcttaaaagaagcttgggctcacgaaaaagacattgttgaaagtttaaacgaagattatgaaaatgctgaacattcagtacaagctaaagcttgggactgggcttgtaaaaaattaggtgtctctattgaagtagatgcttacacaaaattggttaacgtcaacgacatgcaaaaagaatcatggcctggaacaagcgcatggtctttggctatgcgtgcagttaaactacatatcaaacttttcggtcaagcggcttaa

SEQ ID NO: 168 - protein, 173 aa, Bacteriophage D6252
MNGLKTILKTFDKNIYFLTKSVDIRQHRRYNIYVKLREEVNDMKKSTYDKSGIMKEAWNLFNNDDITTADFEYLTRGELQEGKTFAICLKEAWAHEKDIVESLNEDYENAEHSVQAKAWDWACKKLGVSIEVDAYTKLVNVNDMQKESWPGTSAWSLAMRAVKLHIKLFGQAA

SEQ ID NO: 169 - DNA, 522 bp, Bacteriophage D7163
ttgaatggattaaaaacaatcttgaaaacattcgataaaaacatatattttttaaccaaaagtgttgacatacgtcaacacaggagatataatatatatgtaaagttaagagaggaagtaaatgacatgaaaaaatcaacatacgacaaatcaggaattatgaaagaagcttggaatttatttaataacgatgacatcactactgcagattttgaatatcttactcgtggagaattgcaagaaggaaaaacatttgctatttgcttaaaagaagcttgggctcacgaaaaagacattgttgaaagtttaaacgaagattatgaaaatgctgaacattcagtacaagctaaagcttgggactgggcttgtaaaaaattaggtgtctctattgaagtagatgcttacacaaaattggttaacgtcaacgacatgcaaaaagaatcatggcctggaacaagcgcatggtctttggctatgcgtgcagttaaactacatatcaaacttttcggtcaagcggcttaa

SEQ ID NO: 170 - protein, 173 aa, Bacteriophage D7163; identical to SEQ ID NO: 168

SEQ ID NO: 171 - DNA, 336 bp, Bacteriophage 5093
atgaaaaaagaagttatgacaaacgcatggaaaatcgctaaagaagcagttaagaaattcggcggcaaagctatcgaatacatcgcagaagcattgaaaatggcttgggctgccgcaaaaggcggaaacgctagcctagctaaatttcaagcagtagaatctaaaatgcgtaaagctggtaaatactcaatgattcaagttttaaatttcgctaaggaagtgaaatttaacgaagttatgcacaaagttggtgcttactacggtatcgaagtagtagctgacggagacagcattggtacttactacatcgctgaaaaagtttgggatgcagcttaa

SEQ ID NO: 172 - protein, 111 aa, Bacteriophage 5093
MKKEVMTNAWKIAKEAVKKFGGKAIEYIAEALKMAWAAAKGGNASLAKFQAVESKMRKAGKYSMIQVLNFAKEVKFNEVMHKVGAYYGIEVVADGDSIGTYYIAEKVWDAA

SEQ ID NO: 173 - DNA, 336 bp, Bacteriophage P9874
atgaaaaaagaaattatgacaaaagcatggaaaatcgctaaagaagcagttaaaacttttggtgggaaagctatcgaatacatcgctggggctatgaaaatggcttgggctgctatcaaagataacggaactagccttgctaaattccaagctgttgaagcaaaaatgcgtaaagctggtaaatactcaatgatccaagttcttgattttgctaaagaagtacgtttcaatgaagtaatgcacaaagttggcgcttattacggaatcgaagtaattgctgatggtgatagcattggtacttactacatcgctgagaatgtttggaacgcagcataa

SEQ ID NO: 174 - protein, 111 aa, Bacteriophage P9874
MKKEIMTKAWKIAKEAVKTFGGKAIEYIAGAMKMAWAAIKDNGTSLAKFQAVEAKMRKAGKYSMIQVLDFAKEVRFNEVMHKVGAYYGIEVIADGDSIGTYYIAENVWNAA

SEQ ID NO: 175 - DNA, 336 bp, Bacteriophage CHPC577
atgaaaaaagaaattatgacaaaagcatggaaaatcgctaaaaacgcaagtacaaaattcggtggcaaagctatcgaatacattgctggagctatgaaaatggcttgggctgctatcaaagaaaacggaactagccttgctaaattccaagcagttgaagctaaaatgcgcaaagctggcaaacactcaatggtccaagttttaaattttgctaaggaagtgaaatttaacgaagttatgcataaagttggtgcttactacggaattgaagtaattgctgatggtgatagcattggtacttactacatcgctgaaaaagtttggaacgcagcataa

SEQ ID NO: 176 - protein, 111 aa, Bacteriophage CHPC577
MKKEIMTKAWKIAKNASTKFGGKAIEYIAGAMKMAWAAIKENGTSLAKFQAVEAKMRKAGKHSMVQVLNFAKEVKFNEVMHKVGAYYGIEVIADGDSIGTYYIAEKVWNAA

SEQ ID NO: 177 - DNA, 336 bp, Bacteriophage D1024
atgaaaaaagaaattatgacaaaagcatggaaaatcgctaaagaagcagttgaaaaattcggtggcaaagctatcgaatacatcgctggagctatgaaaatggcttgggctgctgctaaagctggaaacactagcgtcgctaaatttcaagctgttgaagataaaatgcgcaaagctggtaaatactcaatgattcaagttttaaatttcgctaatgaagtgaaatttaacgaagttatgcacaaagctggtgcgtactacggcatcgaagtaattgctgatggtgatagcattggtacttactacatcgctgaaaaagtttgggaagtagcataa

SEQ ID NO: 178 - protein, 111 aa, Bacteriophage D1024
MKKEIMTKAWKIAKEAVEKFGGKAIEYIAGAMKMAWAAAKAGNTSVAKFQAVEDKMRKAGKYSMIQVLNFANEVKFNEVMHKAGAYYGIEVIADGDSIGTYYIAEKVWEVA

SEQ ID NO: 179 - DNA, 327 bp, Bacteriophage D1126
atgaaaaaagaagttatgacaaacgcgtgggaaattgctaaaaacgcttctaaaaaattcggtggtaaagctatcgaatacatcgctggagctatgaaaatggcttgggctgctgcaaaaggcggcttagctaaattccaagcagtagaatctaaaatgcgtaaagctggaaaacattcaatggtgcaagtgttgaatttcgctaaggaagtgaaatttaacgaagttatgcacaaagctggtgcttactacggtatcgaagtaatcgctgatggtgatagcattggtacttactacatttctgaaaaagtttgggaagtagcttaa

SEQ ID NO: 180 - protein, 108 aa, Bacteriophage D1126
MKKEVMTNAWEIAKNASKKFGGKAIEYIAGAMKMAWAAAKGGLAKFQAVESKMRKAGKHSMVQVLNFAKEVKFNEVMHKAGAYYGIEVIADGDSIGTYYISEKVWEVA

SEQ ID NO: 181 - DNA, 336 bp, Bacteriophage D1297
atgaaaaaagaaattatgacaaaagcatggaaaatcgctaaagaagcagttaaaactttcggtggtaaagctatcgaatacattgctggagctatgaaaatggcttgggctgctgctaaagctggaaacactagcttagctaaattccaagcagtagaatctaaaatgcgtaaagctggtaaatactcaatgattcaagttttaaatttcgctaaggaagtgaaatttaacgaagttatgcacaaagttggcgcttattacggtatcgaagtaattgctgatggtgatagcattggtacttactacatcgctgaaagcgtttgggaagtagcataa

SEQ ID NO: 182 - protein, 111 aa, Bacteriophage D1297
MKKEIMTKAWKIAKEAVKTFGGKAIEYIAGAMKMAWAAAKAGNTSLAKFQAVESKMRKAGKYSMIQVLNFAKEVKFNEVMHKVGAYYGIEVIADGDSIGTYYIAESVWEVA

SEQ ID NO: 183 - DNA, 336 bp, Bacteriophage D1422
atgaaaaaagaaattatgacaaaagcatggaaaatcgctaaagaagcagttgaaaaattcggtggcaaagctatcgaatacatcgctggagctatgaaaatggcttgggctgctgctaaagctggaaacactagcgtcgctaaatttcaagctgttgaagataaaatgcgcaaagctggtaaatactcaatgattcaagttttaaatttcgctaatgaagtgaaatttaacgaagttatgcacaaagctggtgcgtactacggaatcgaagtaattgctgatggtgatagcattggtacttactacatcgctgaaaaagtttgggaagtagcataa

SEQ ID NO: 184 - protein, 111 aa, Bacteriophage D1422; identical to SEQ ID NO: 178

SEQ ID NO: 185 - DNA, 318 bp, Bacteriophage D2759
atgaaaaaagaaattatgacaaaagcatggaaaatcgctaaagaagcagttaaaactttcggtggaaaagctatcgaatacattgcggaagcaatgaaaatggcttgggctgctgctaaaggcggcttagctaaattccaagcagtagaatctaaaatgcgtaaagctggaatgattcaagttttaaatttcgctaaggaagtgaaatttaacgaagttatgcacaaagttggcgcttattacggtatcgaagtaattgctgatggtgatagcattggtacttactacatcgctgaaagcgtttgggaagtagcataa

SEQ ID NO: 186 - protein, 105 aa, Bacteriophage D2759
MKKEIMTKAWKIAKEAVKTFGGKAIEYIAEAMKMAWAAAKGGLAKFQAVESKMRKAGMIQVLNFAKEVKFNEVMHKVGAYYGIEVIADGDSIGTYYIAESVWEVA

SEQ ID NO: 187 - DNA, 336 bp, Bacteriophage D3577
atgaaatcacaagtaatgagcctagcatggaaaatcgctaaaaacgcaagtacaaaattcggtggcaaagctatcgaatacattgctagagctatgaaaatggcttggtctgctatcaaagaaaacggaactagccttgctaaatttcaagcaattgaagctaaaattcgcaaagctggaaaacactcaatggtccaagttttaaaattcgctaaggaagtgaaatttaacgaagttatgcataaagttggtgcttactacggaattgaagtaattgctgatggtgatagcattggtacttactacatcgctgaaaaagtttgggatgcagcgtaa

SEQ ID NO: 188 - protein, 111 aa, Bacteriophage D3577
MKSQVMSLAWKIAKNASTKFGGKAIEYIARAMKMAWSAIKENGTSLAKFQAIEAKIRKAGKHSMVQVLKFAKEVKFNEVMHKVGAYYGIEVIADGDSIGTYYIAEKVWDAA

SEQ ID NO: 189 - DNA, 336 bp, Bacteriophage D4154
atgaaaaaagaaattatgaaaaaagcatggaaaatcgctaaagaagcagttaagaaattcggtggtaaagctatcgaatacatcgcagaagcattgaaaatggcttgggctgatgctaaaggtggtaacactagcttggctaaattccaagctgttgaggaaaagatgcgtaaagctggcaaatactcaatgattcaagtgctcaactttgctaaagaagtgaaattcaacgaagtaatgcataaagttggtgcttactacggaattgaagttattgctgacggagacaaaatcggtacttactttatcgctgaaaaagtttgggatgcagcttaa

SEQ ID NO: 190 - protein, 111 aa, Bacteriophage D4154
MKKEIMKKAWKIAKEAVKKFGGKAIEYIAEALKMAWADAKGGNTSLAKFQAVEEKMRKAGKYSMIQVLNFAKEVKFNEVMHKVGAYYGIEVIADGDKIGTYFIAEKVWDAA

SEQ ID NO: 191 - DNA, 336 bp, Bacteriophage D4160
atgaaaaaagaacttatgaaagacgcttgggaaattgctaaaaacgcttctaaaaaattcggtggtaaagctatcgaatacattgctggagctatgaaaatggcttgggctgctgctaaagctggaaacactagcgtcgctaaattccaagcggtagaagctaaaatgcgcaaagctggcaaacactcaatgattcaagttctcgatttcgctaaagaagttaagttcaacgaagtgatgcacaaagttggtgcgtactacggcatcgaagtagtcgctgacggcgatagcattggtacttactacatcgctgaaaaagtttgggatgtagcttaa

SEQ ID NO: 192 - protein, 111 aa, Bacteriophage D4160
MKKELMKDAWEIAKNASKKFGGKAIEYIAGAMKMAWAAAKAGNTSVAKFQAVEAKMRKAGKHSMIQVLDFAKEVKFNEVMHKVGAYYGIEVVADGDSIGTYYIAEKVWDVA

SEQ ID NO: 193 - DNA, 336 bp, Bacteriophage D4212
atgaaaaaagaagttatgacaaacgcatggaaaatcgctaaagaagcagttaagaaattcggtggtaaagctatcgaatacatctctgaagctatgaaaatggcttgggctgctgccaagggtgaaaacactagcttagctaaattccaagctgttgaggaaaagatgcgtaaagctggcaaatactcaatgattcaagttcttgactttgctaaagaagttaaattcaacgaagtaatgcataaagttggtgcttactacggaattgaagttattgctgacggagacaacattggtacttactacattgctgaaaaagtttgggaagtagcataa

SEQ ID NO: 194 - protein, 111 aa, Bacteriophage D4212
MKKEVMTNAWKIAKEAVKKFGGKAIEYISEAMKMAWAAAKGENTSLAKFQAVEEKMRKAGKYSMIQVLDFAKEVKFNEVMHKVGAYYGIEVIADGDNIGTYYIAEKVWEVA

SEQ ID NO: 195 - DNA, 321 bp, Bacteriophage D4276
atgacaaacgcatggaaaatcgctaaagaagcagttaagaaattcggtggtaaagctatcgaatacatctctgaagctatgaaaattgcttgggctgacgctaaagaaggaaacactagcgtagctaaattccaagctgtagaagctaaaatgcgtaaagctggaaaacattcaatggtgcaagtgttgaatttcgctaaagaagtgaaattcaacgaagtaatgcacaaagttggtgcttactacggtatcgaagtaatcgctgatggtgatagcattggtacttactacatttctgaaaaagtttgggaagtagcttaa

SEQ ID NO: 196 - protein, 106 aa, Bacteriophage D4276
MTNAWKIAKEAVKKFGGKAIEYISEAMKIAWADAKEGNTSVAKFQAVEAKMRKAGKHSMVQVLNFAKEVKFNEVMHKVGAYYGIEVIADGDSIGTYYISEKVWEVA

SEQ ID NO: 197 - DNA, 336 bp, Bacteriophage D4419
atgaaaaaagaaattatgacaaaagcatggaaaatcgctaaagaagcagttaaaactttcggtggaaaagctatcgaatacattgcggaagcaatgaaaatggcttgggctgctgctaaaggcggaaacgctagcttagctaaattccaagcagtagaatctaaaatgcgtaaagctggtaaatactcaatgattcaagttttaaatttcgctaaggaagtgaaatttaacgaagttatgcacaaagttggcgcttattacggtattgaagtaattgctgatggtgatagcattggtacttactacatcgctgaaagcgtttgggaagtagcataa

SEQ ID NO: 198 - protein, 111 aa, Bacteriophage D4419
MKKEIMTKAWKIAKEAVKTFGGKAIEYIAEAMKMAWAAAKGGNASLAKFQAVESKMRKAGKYSMIQVLNFAKEVKFNEVMHKVGAYYGIEVIADGDSIGTYYIAESVWEVA

SEQ ID NO: 199 - DNA, 327 bp, Bacteriophage D4741
atgaaaaaagaaattatgacaaaagcatggaaaatcgctaaagaagcagttaaaactttcggtggaaaagctatcgaatacattgcggaagcaatgaaaatggcttgggctgctgctaaaggcggcttagctaaattccaagcagtagaatctaaaatgcgtaaagctggtaaatactcaatgattcaagttttaaatttcgctaaggaagtgaaatttaacgaagttatgcacaaagttggcgcttattacggtatcgaagtaattgctgatggtgatagcattggtacttactacatcgctgaaagcgtttgggaagtagcataa

SEQ ID NO: 200 - protein, 108 aa, Bacteriophage D4741
MKKEIMTKAWKIAKEAVKTFGGKAIEYIAEAMKMAWAAAKGGLAKFQAVESKMRKAGKYSMIQVLNFAKEVKFNEVMHKVGAYYGIEVIADGDSIGTYYIAESVWEVA

SEQ ID NO: 201 - DNA, 336 bp, Bacteriophage D5839
atgaagaaagagattatgaaaaaagcgtgggaaatcgctaaagaagcagttaaaaaattcggtggcaaagctatcgaatacatcgcagaagcattgaaaatggcttggtctgatgcaaagggtagtaatactagcttagctaaattccaagctgttgaggaaaagatgcgtaaagctggcaaatactcaatgattcaagttcttgactttgctaaagaagttaaattcaatgaagtaatgcacaaagaaggtgcttactatggtatcgaagtggtagctgacggagacagcattggtacttattacattgctgaaaaagtttgggaagtagcataa

SEQ ID NO: 202 - protein, 111 aa, Bacteriophage D5839
MKKEIMKKAWEIAKEAVKKFGGKAIEYIAEALKMAWSDAKGSNTSLAKFQAVEEKMRKAGKYSMIQVLDFAKEVKFNEVMHKEGAYYGIEVVADGDSIGTYYIAEKVWEVA

SEQ ID NO: 203 - DNA, 336 bp, Bacteriophage D5861
atgaaaaaagaaattatgacaaaagcatgggaaattgctaaaaacgcttctaaaaaattcggtggtaaagctatcgaatacatcgctggagctatgaaaatggcttgggctgctgctaaagctggaaacactagcgtcgctaaattccaagcggtagaagctaaaatgcgcaaagctggaaaacattcaatggtccaagttttgaattttgcaaaagaagttaagttcaacgaagtaatgcacaaagttggcacttattacggcatcgaagtagtagctgacggcgatagcattggtacttactacatcgctgaaaaagtttgggatgcagcataa

SEQ ID NO: 204 - protein, 111 aa, Bacteriophage D5861
MKKEIMTKAWEIAKNASKKFGGKAIEYIAGAMKMAWAAAKAGNTSVAKFQAVEAKMRKAGKHSMVQVLNFAKEVKFNEVMHKVGTYYGIEVVADGDSIGTYYIAEKVWDAA

SEQ ID NO: 205 - DNA, 336 bp, Bacteriophage D6252
atgaaaaaagaaattatgacaaaagcttgggaaattgctaaaaacgcttctaaaaaattcggtggtaaagctatcgaatacatcgctggagctatgaaaatggcttgggctgctgctaaagctggaaaaactagcgtcgctaaattccaagcggtagaagctaaaatgcgcaaagctggaaaacattcaatggtccaagttttgaattttgctaaagaagtacgtttcaacgaagtaatgcacaaagctggcgcttattacggtatcgaagtaattgctgatggtgatagcattggtacttacttcattgctgagaatgtttggaacgcagcataa

SEQ ID NO: 206 - protein, 111 aa, Bacteriophage D6252
MKKEIMTKAWEIAKNASKKFGGKAIEYIAGAMKMAWAAAKAGKTSVAKFQAVEAKMRKAGKHSMVQVLNFAKEVRFNEVMHKAGAYYGIEVIADGDSIGTYFIAENVWNAA

SEQ ID NO: 207 - DNA, 336 bp, Bacteriophage D6312
atgaaaaaagaaattatgacaaaagcatggaaaatcgctaaagaagcagttaaaactttcggtggtaaagctatcgaatacatcgcagaagcattgaaaatggcttgggctgctgccaagggtgaaaacactagcttagctaaaattcaagctgttgaggaaaagatgcgtaaatctggtaaatactcaatgatccaagttcttgattttgctaaagaagtgaaatttaacgaagtaatgcacaaagctggtgcttactacggtatcgaagttattgctgatggcgatagcattggtacttattacattgctgaaaaagtttgggaagtagcttaa

SEQ ID NO: 208 - protein, 111 aa, Bacteriophage D6312
MKKEIMTKAWKIAKEAVKTFGGKAIEYIAEALKMAWAAAKGENTSLAKIQAVEEKMRKSGKYSMIQVLDFAKEVKFNEVMHKAGAYYGIEVIADGDSIGTYYIAEKVWEVA

SEQ ID NO: 209 - DNA, 336 bp, Bacteriophage D7130
atgaaaaaagaaattatgacaaaagcatggaaaatcgctaaagaagcagttaaaactttcggtggaaaagctatcgaatacattgcggaagcaatgaaaatggcttgggctgctgctaaaggcggaaacgctagcttagctaaattccaagcagtagaatctaaaatgcgtaaagctggtaaatactcaatgattcaagttttaaatttcgctaaggaagtgaaatttaacgaagttatgcacaaagttggcgcttattacggtatcgaagtaattgctgatggtgatagcattggtacttactacatcgctgaaaacgtttggaacgcagcataa

SEQ ID NO: 210 - protein, 111 aa, Bacteriophage D7130
MKKEIMTKAWKIAKEAVKTFGGKAIEYIAEAMKMAWAAAKGGNASLAKFQAVESKMRKAGKYSMIQVLNFAKEVKFNEVMHKVGAYYGIEVIADGDSIGTYYIAENVWNAA

SEQ ID NO: 211 - DNA, 336 bp, Bacteriophage D802
atgaaaaaagaaattatgacaaaagcatggaaaatcgctaaagaagcagttgagaagttcggtggtaaatctatcgaatacattgcggaagcaatgaaaatggcttgggctgctgcaaaaggcggaaacgctagcttagctaaatttcaagcggtagaagctaaaatgcgcaaagctggtaaatactcaatgattcaagttttaaatttcgctaaggaagtgaaatttaacgaagttatgcacaaagctggtgcttactatggaatcgaagtggtagctgacggagacagcattggtacttattacatcgctgaaaaagtttgggaagtagcataa

SEQ ID NO: 212 - protein, 111 aa, Bacteriophage D802
MKKEIMTKAWKIAKEAVEKFGGKSIEYIAEAMKMAWAAAKGGNASLAKFQAVEAKMRKAGKYSMIQVLNFAKEVKFNEVMHKAGAYYGIEVVADGDSIGTYYIAEKVWEVA

SEQ ID NO: 213 - DNA, 336 bp, Bacteriophage N1024
atgaaaaaagaaattatgacaaaagcttgggaaattgctaaaaacgcttctaaaaaattcggtggtaaagctatcgaatacatcgctggagctatgaaaatggcttgggctgctgctaaagctggaaacactagcgtcgctaaattccaagcggtagaagctaaaatgcgcaaagctggaaaacattcaatggtccaagttttgaattttgcaaaagaagttaagttcaacgaagtaatgcacaaagttggcacttattacggcatcgaagtagtagctgacggcgatagcattggtacttactacatcgctgaaaaagtttgggatgcagcataa

SEQ ID NO: 214 - protein, 111 aa, Bacteriophage N1024; identical to SEQ ID NO: 204

SEQ ID NO: 215 - DNA, 336 bp, Bacteriophage O1205
atgaaatcacaagtaatgagccaagcatggaaaatcgctaaagaagcagttaagaaattcggtggtaaagctatcgaatacatctctgaagctatgaaaatggcttgggctgctgccaagggtgaaaacactagcttaactaaatttcaagctgttgaggaaaagatgcgtaaagctggcaaatactcaatgattcaagttcttgactttgctaaagaagtgaaattcaacgaagtaatgcataaagttggtgcttactacggaattgaagttattgctgacggagacagcattggtacttactttatcgctgaaaaagtttgggatgtagcttaa

SEQ ID NO: 216 - protein, 111 aa, Bacteriophage O1205
MKSQVMSQAWKIAKEAVKKFGGKAIEYISEAMKMAWAAAKGENTSLTKFQAVEEKMRKAGKYSMIQVLDFAKEVKFNEVMHKVGAYYGIEVIADGDSIGTYFIAEKVWDVA

SEQ ID NO: 217 - DNA, 336 bp, Bacteriophage P0095
atgaaaaaagaaattatgaaaaaagcatggaaaatcgctaaagaagcagttaagaagttcggcggcaaagctatcgaatacatcgcagaagcattgaaaatggcttggtctgatgcaaagggtagtaatactagcttagctaaattccaagctgttgaggaaaagatgcgtaaagctggcaaatactcaatgatccaagttcttgattttgctaaagaagtgaaatttaacgaagtaatgcacaaagctggtgcttactacggtatcgaagttattgctgatggcgatagcattggtacttattacattgctgaaaaagtttgggaagtagcttaa

SEQ ID NO: 218 - protein, 111 aa, Bacteriophage P0095
MKKEIMKKAWKIAKEAVKKFGGKAIEYIAEALKMAWSDAKGSNTSLAKFQAVEEKMRKAGKYSMIQVLDFAKEVKFNEVMHKAGAYYGIEVIADGDSIGTYYIAEKVWEVA

SEQ ID NO: 219 - DNA, 336 bp, Bacteriophage P5641
atgaaaaaagaaattatgacaaaagcttgggaaattgctaaaaacgcttctaaaaaattcggtggtaaagctatcgaatacatcgctggagctatgaaaatggcttgggctgctgctaaagctggaaacactagcgtcgctaaattccaagcggtagaagctaaaatgcgcaaagctggaaaacattcaatggtccaagttttgaattttgcaaaagaagttaagttcaacgaagtaatgcacaaagttggcgcttattacggcatcgaagtagtagctgacggcgatagcattggtacttattacattgctgaaaaagtttgggaagtagcataa

SEQ ID NO: 220 - protein, 111 aa, Bacteriophage P5641
MKKEIMTKAWEIAKNASKKFGGKAIEYIAGAMKMAWAAAKAGNTSVAKFQAVEAKMRKAGKHSMVQVLNFAKEVKFNEVMHKVGAYYGIEVVADGDSIGTYYIAEKVWEVA

SEQ ID NO: 221 - DNA, 336 bp, Bacteriophage P7602
atgaaaaaagaaattatgacaaacgcgtgggaaattgctaaaaacgcttctaaaaaattcggtggtaaagctatcgaatacatcgcagaagcattgaaaatggcttggtctgatgcaaagggtagtaatactagcttagctaaattccaagctgttgaggaaaagatgcgtaaagctggcaaatactcaatgattcaagttttaaatttcgctaaagaagtgaaattcaatgaagtaatgcacaaagaaggtgcttactatggtatcgaagtagtagctgacggagacagcattggtacttattacattgctgaaaaagtttgggatgcagcgtaa

SEQ ID NO: 222 - protein, 111 aa, Bacteriophage P7602
MKKEIMTNAWEIAKNASKKFGGKAIEYIAEALKMAWSDAKGSNTSLAKFQAVEEKMRKAGKYSMIQVLNFAKEVKFNEVMHKEGAYYGIEVVADGDSIGTYYIAEKVWDAA

SEQ ID NO: 223 - DNA, 336 bp, Bacteriophage SFi18
atgaaaaaagaagttatgacaaacgcatggaaaatcgctaaagaagcagttaagaaattcggtggtaaagctatcgaatacatctctgaagctatgaaaatggcttgggctgctgccaagggtgaaaacactagcttagctaaattccaagctgttgaggaaaagatgcgtaaagctggcaaatactcaatgattcaagttcttgactttgctaaagaagttaaaatcaacgaagtaatgcataaagttggtgcttactacggaattgaagttattgctgacggagacaacattggtacttactacattgctgaaaaagtttgggaagtagcataa

SEQ ID NO: 224 - protein, 111 aa, Bacteriophage SFi18
MKKEVMTNAWKIAKEAVKKFGGKAIEYISEAMKMAWAAAKGENTSLAKFQAVEEKMRKAGKYSMIQVLDFAKEVKINEVMHKVGAYYGIEVIADGDNIGTYYIAEKVWEVA

SEQ ID NO: 225 - DNA, 336 bp, Bacteriophage Sfi11
atgaaaaaagaagttatgacaaacgcatggaaaatcgctaaagaagcagttaagaaattcggtggtaaagctatcgaatacatctctgaaggctatgaaatggcttgggctgctgccaagggtgaaaacactagcttagctaaattccaagctgttgaggaaaagatgcgtaaagctggcaaatactcaatgattcaagttcttgactttgctaaagaagttaaattcaacgaagtaatgcataaagttggtgcttactacggaattgaagttattgctgacggagacaacattggtacttactacattgctgaaaaagtttgggaagtagcataa

SEQ ID NO: 226 - protein, 111 aa, Bacteriophage Sfi11
MKKEVMTNAWKIAKEAVKKFGGKAIEYISEGYEMAWAAAKGENTSLAKFQAVEEKMRKAGKYSMIQVLDFAKEVKFNEVMHKVGAYYGIEVIADGDNIGTYYIAEKVWEVA

SEQ ID NO: 227 - DNA, 336 bp, Bacteriophage Sfi19
atgaagaaagagattatgaaaaaagcgtgggaaatcgctaaagaagcagttaaaaaattcggtggcaaagctatcgaatacatcgcagaagcattgaaaatggcttggtctgatgcaaagggtagtaatactagcttagctaaattccaagctgttgaggaaaagatgcgtaaagctggcaaatactcaatgattcaagttcttgactttgctaaagaagttaaattcaatgaagtaatgcacaaagaaggtgcttactatggtatcgaagtggtagctgacggagacagcattggtacttactacattgctgaaaaagtttgggaagtagcataa

SEQ ID NO: 228 - protein, 111 aa, Bacteriophage Sfi19; identical to SEQ ID NO: 202

SEQ ID NO: 229 - DNA, 333 bp, Bacteriophage Sfi21
atgaaaaaaattatgacaaacgcatggaaaatcgctaaagaagcagttaagaaattcggtggtaaagctatcgaatacatctctgaagctatgaaaattgcttgggctgatgctaaagaaggaaacactagcgtagctaaattccaagctgtagaagctaaaatgcgtaaagctggaaaacattcaatggtgcaagtgttgaatttcgctaaagaagtgaaattcaacgaagtaatgcacaaagttggtgcttactacggtatcgaagtaatcgctgatggtgatagcattggtacttactacatttctgaaaaagtttgggaagtagcttaa

SEQ ID NO: 230 - protein, 110 aa, Bacteriophage Sfi21
MKKIMTNAWKIAKEAVKKFGGKAIEYISEAMKIAWADAKEGNTSVAKFQAVEAKMRKAGKHSMVQVLNFAKEVKFNEVMHKVGAYYGIEVIADGDSIGTYYISEKVWEVA

SEQ ID NO: 231 - DNA, 336 bp, Bacteriophage Proph1
atgaaaaaagaaattatgaaaaaagcatggaaaatcgctaaagaagcagttaagaagttcggcggcaaagctatcgaatacatcgcagaagcattgaaaatggcttggtctgatgcaaagggtagtaatactagcttagctaaattccaagctgtagaagataaaatgaacaaaaccggaaaacactcaatggtccaagtcttgaattttgctaaagaagtgaatttcaaagaagtaatgcataaagttggtgcttactacggtatcgaagtagtagctgacggagacagcattggtacttactacatcgctgaaaaggtttgggatgcagcttaa

SEQ ID NO: 232 - protein, 111 aa, Bacteriophage Proph1
MKKEIMKKAWKIAKEAVKKFGGKAIEYIAEALKMAWSDAKGSNTSLAKFQAVEDKMNKTGKHSMVQVLNFAKEVNFKEVMHKVGAYYGIEVVADGDSIGTYYIAEKVWDAA

SEQ ID NO: 233 - DNA, 111 bp, Bacteriophage D1427
atgaaaaaagaagttatgacaaacgcgtgggaaattgctaaaaacgcttctaaaaaattcggtggtaaagctatcgaatacatcgctgaaaacgtttggaacgcagcataa

SEQ ID NO: 234 - protein, 36 aa, Bacteriophage D1427
MKKEVMTNAWEIAKNASKKFGGKAIEYIAENVWNAA

SEQ ID NO: 235 - DNA, 345 bp, Bacteriophage D5691
atgaaatcacaagtaatgagcctagcatggaaaatcttcaaaaacgaaaaaaacgacgtaactttttctgaagcattgaagtttgcttggaaagccgttaaacgtcaaaatatggcagatgatttctacttcttccattcttcaaatgttaaatttcaaggtgttaagaaatggtttgctgaaaaagagttccgtggacgcaacaaaaaagacttggcgttcatgtcagtaagtgcaatcagtgttaaagggttggtcgaagaaactgataaagcagttaaacttgaaatcgtgacaccttatggggtttctgctaaatggtacccaaaaagtgtaattgcttaa

SEQ ID NO: 236 - protein, 114 aa, Bacteriophage D5691
MKSQVMSLAWKIFKNEKNDVTFSEALKFAWKAVKRQNMADDFYFFHSSNVKFQGVKKWFAEKEFRGRNKKDLAFMSVSAISVKGLVEETDKAVKLEIVTPYGVSAKWYPKSVIA

SEQ ID NO: 237 - DNA, 345 bp, Bacteriophage D6193
atgaaatcacaagtaatgagcctagcatggaaaatcttcaaaaacgaaaaaaacgatgtaactttttctgaagcgttgaaatttgcttggaaagccgttaaacgtcaaaacatggcggatgatttttacttcttccgttcttcaaatgttaaattccaaggtgttaagaaatggtttgctgaaaaagaatttcgtggacgcaacaagaaagacttggcgtttatgtcagtaactgcaatcagtgttaaagggttgattgaagaaactgataaagcggttaagcttgaaatcgtaacaccttatggagtttctactaaatggtatccaaagagtgtaattgcttaa

SEQ ID NO: 238 - protein, 114 aa, Bacteriophage D6193
MKSQVMSLAWKIFKNEKNDVTFSEALKFAWKAVKRQNMADDFYFFRSSNVKFQGVKKWFAEKEFRGRNKKDLAFMSVTAISVKGLIEETDKAVKLEIVTPYGVSTKWYPKSVIA

SEQ ID NO: 239 - DNA, 345 bp, Bacteriophage D7035
atgaaatcacaagtaatgagcctagcatggaaaattttcaaaaacgaaaaaaacgacgtaactttttctgaagcattgaagtttgcttggaaagccgttaaacgtcaaaacatggcggatgatttctacttcttccgttcttcaaacgttaaattccaaggtgttaagaaatggtttgctgaaaaagaatttcgtggacgcaacaagaaagacttggcgtttatgtcagtaactgcaatcagcattaaagggttggttgaagaaactgataaagcggttaagcttgaaatcgtgacaccttatggaatttctactaaatggtatccaaagagtgtaattgcttaa

SEQ ID NO: 240 - protein, 114 aa, Bacteriophage D7035
MKSQVMSLAWKIFKNEKNDVTFSEALKFAWKAVKRQNMADDFYFFRSSNVKFQGVKKWFAEKEFRGRNKKDLAFMSVTAISIKGLVEETDKAVKLEIVTPYGISTKWYPKSVIA

SEQ ID NO: 241 - DNA, 345 bp, Bacteriophage Proph1
atgaaatcacaagtaatgagcctagcatggaaaatcttcaaaaacgaaaaaaacgatgtaactttttctgaagcgttgaaatttgcttggaaagccgttaaacgtcaaaacatggcggatgatttctacttcttccgttcttcaaacgttaaattccaaggtgttaagaaatggtttgctgaaaaagaatttcgtggacgcaacaagaaagacttggcgtttatgtcagtaactgcaatcagcgttaaagggttgatcgaagaaactgataaagcggttaagcttgaaatcgtaacaccttatggagtttctactaaatggtatccaaagagtgtaattgcttaa

SEQ ID NO: 242 - protein, 114 aa, Bacteriophage Proph1; identical to SEQ ID NO: 238

SEQ ID NO: 243 - DNA, 345 bp, Bacteriophage Proph1
atgaaatcacaagtaatgagcctagcatggaaaatcttcaaaaacgaaaaaaacgatgtaactttttctgaagcgttgaaatttgcttggaaagccgttaaacgtcaaaacatggcggatgatttctacttcttccgttcttcaaacgttaaattccaaggtgttaagaaatggtttgctgaaaaagaatttcgtggacgcaacaagaaagacttggcgtttatgtcagtaactgcaatcagcattaaagggttggttgaagaaactgataaagcggttaagcttgaaatcgtgacaccttatggaatttctactaaatggtatccaaagagtgtaattgcttaa

SEQ ID NO: 244 - protein, 114 aa, Bacteriophage Proph1; identical to SEQ ID NO: 240

SEQ ID NO: 245 - DNA, 261 bp, Bacteriophage 5093
gtgaaaacaatggatgcatataaagaacaatttcaagaattacaagaatacgcttttaacgttttaagagaatatcctctagacaagacagcagttaatgtgctttctgcactcgttaactcaaaaaagaaagatcgcatcgagttttttaaactaaacaaaggcgaagatgccatgaaagtttattataatctagcagatagcggaacgattgaaaaatatttagaaacatctgcatttttagattacatcaatgaataa

SEQ ID NO: 246 - protein, 86 aa, Bacteriophage 5093
MKTMDAYKEQFQELQEYAFNVLREYPLDKTAVNVLSALVNSKKKDRIEFFKLNKGEDAMKVYYNLADSGTIEKYLETSAFLDYINE

SEQ ID NO: 247 - DNA, 252 bp, Bacteriophage D4154
atggatacatataaagaacaatttcaaaaattacaagaatacgcttttaacgttttaagagaataccctctagataagacagcagttaatgtactttctgcactcgttaactcaaaaaagaaagatcgcatcgagttttttaaactaaacaaaggcgaagatgccatgaaagtttattataatctagcagatagcggaacgattgaaaaatatttagaaacatctgcatttttagaatacataaatgaataa

SEQ ID NO: 248 - protein, 83 aa, Bacteriophage D4154
MDTYKEQFQKLQEYAFNVLREYPLDKTAVNVLSALVNSKKKDRIEFFKLNKGEDAMKVYYNLADSGTIEKYLETSAFLEYINE

SEQ ID NO: 249 - DNA, 252 bp, Bacteriophage D4160
atggatacatataaagaacaatttcaagaattacaagaatacgcttttaacgttttaagagaatatcctctagacaagacagcagttaatgtactttctgcactcgttaactcaaaaaagaaagatcgcatcgagttttttaaactaaacaaagacgaagatgccatgaaagtttattataatctagcagatagcggaacgattgaaaaatatttagaaacatctgcatttttagaatacatcaatgaataa

SEQ ID NO: 250 - protein, 83 aa, Bacteriophage D4160
MDTYKEQFQELQEYAFNVLREYPLDKTAVNVLSALVNSKKKDRIEFFKLNKDEDAMKVYYNLADSGTIEKYLETSAFLEYINE

SEQ ID NO: 251 - DNA, 252 bp, Bacteriophage D4212
atggatacatataaagaacaatttcaagaattacaagaatacgcttttaacattttaagagaatatcctctagacaagacagcagttaatgtactttctgcactcgttaactcaaaaaagaaagatcgcatcgagttttttaaactaaacaaagacgaagatgccatgaaagtttattataatctagcagatagcggaacgattgaaaaatatttagaaacatctgcatttttagaatacatcaatgaataa

SEQ ID NO: 252 - protein, 83 aa, Bacteriophage D4212
MDTYKEQFQELQEYAFNILREYPLDKTAVNVLSALVNSKKKDRIEFFKLNKDEDAMKVYYNLADSGTIEKYLETSAFLEYINE

SEQ ID NO: 253 - DNA, 252 bp, Bacteriophage D6193
atggatacatacaaagaacaatttcaaaaattacaagaatacgcttttaacgttttaagagaataccctctagataagacagcagttaatgtactttctgcactcgttaactcaaaaaagaaagatcgcatcgagttttttaaactaaacaaaggcgaagatgccatgaaagtttattataatctagcagatagcggaacgattgaaaaatatttagaaacatctgcatttttagaatacacaaatgaataa

SEQ ID NO: 254 - protein, 83 aa, Bacteriophage D6193
MDTYKEQFQKLQEYAFNVLREYPLDKTAVNVLSALVNSKKKDRIEFFKLNKGEDAMKVYYNLADSGTIEKYLETSAFLEYTNE

SEQ ID NO: 255 - DNA, 252 bp, Bacteriophage Sfi11
atggatacatataaagaacaatttcaagaattacaagaatacgcttttaacattttaagagaatatcctctagacaagacagcagttaatgtactttctgcactcgttaactcaaaaaagaaagatcgcatcgagttttttaaacttaacaaagacgaagatgccatgaaagtttattataatctagcagatagcggaacgattgaaaaatatttagaaacatctgcatttttagaatacatcaatgaataa

SEQ ID NO: 256 - protein, 83 aa, Bacteriophage Sfi11; identical to SEQ ID NO: 252

SEQ ID NO: 257 - DNA, 252 bp, Bacteriophage Proph1
atggatacatacaaagaacaatttcaagaattacaagaatacgcttttaacgttttaagagaataccctctagataagacagcagttaatgtactttctgcactcgttaactcaaaaaagaaagatcgcatcgagttttttaaactaaacaaaggcgaagacgccatgaaagtttattataatctagcagatagcggaacgattgaaaaatatttagaaacatctgcattcttagaatacatcaatgaataa

SEQ ID NO: 258 - protein, 83 aa, Bacteriophage Proph1
MDTYKEQFQELQEYAFNVLREYPLDKTAVNVLSALVNSKKKDRIEFFKLNKGEDAMKVYYNLADSGTIEKYLETSAFLEYINE

SEQ ID NO: 259 - DNA, 252 bp, Bacteriophage Proph1
atggatacatataaagaacaatttcaagaattacaagaatacgcttttaacgttttaagagaatatcctctagacaagacagcagttaatgtactttctgcactcgttaactcaaaaaagaaagatcgcatcgagttttttaaactaaacaaaggcgaagatgccatgaaagtttattatagtctagcagatagcggaacgattgagagatacttggaagtctgtggatttttagagtacatcaacgaataa

SEQ ID NO: 260 - protein, 83 aa, Bacteriophage Proph1
MDTYKEQFQELQEYAFNVLREYPLDKTAVNVLSALVNSKKKDRIEFFKLNKGEDAMKVYYSLADSGTIERYLEVCGFLEYINE

SEQ ID NO: 261 - DNA, 282 bp, Bacteriophage D1024
atgataactaaagaacaattaaaagaatactacagcgaacacttggaagagctcgtcgaatgggcagacgatataaataaaatatgcctatttgcctacctagatgaagatgataacttgtattgtgggattaatcaactgtcctacacacaattcagagttccaattcaagctgaggtgacagtggatgatgattggaactacgatttcttcaaaaatccagctgcctatgatggatgggatgaaactttggaagaaatgttggaagaattaaatgattaa

SEQ ID NO: 262 - protein, 93 aa, Bacteriophage D1024
MITKEQLKEYYSEHLEELVEWADDINKICLFAYLDEDDNLYCGINQLSYTQFRVPIQAEVTVDDDWNYDFFKNPAAYDGWDETLEEMLEELND

SEQ ID NO: 263 - DNA, 282 bp, Bacteriophage D1811; identical to SEQ ID NO: 261

SEQ ID NO: 264 - protein, 93 aa, Bacteriophage D1811; identical to SEQ ID NO: 262

SEQ ID NO: 265 - DNA, 282 bp, Bacteriophage D7035
atgataactaaagaacaattaaaagaatactacagcgaacacttggaagagctcgtcgaatgggcagacgatataaataaaatatgcctatttgcctacctagatgaagatgataacttgtattgtgggataaatcaactgtcctacacacaattcagagttccaattcaagctgaggtgacagtggatgatgattggaactacgatttcttcaaaaatccagctgcctatgatggatgggatgaaactttggaagaaatgttggaagaattaaatgattaa

SEQ ID NO: 266 - protein, 93 aa, Bacteriophage D7035
MITKEQLKEYYSEHLEELVEWADDINKICLFAYLDEDDNLYCGINQLSYTQFRVPIQAEVTVDDDWNYDFFNNPASYDGWDETLEEMLEELND

SEQ ID NO: 267 - DNA, 141 bp, Bacteriophage D3821
gtgaaaacaatggatacatataaagaacaattttattatttggatcctatttatattagtgtggatattaataggaggacttttattttaggaaaaagagggcaatcgctctcttttttttattgtaataaaacaatttaa

SEQ ID NO: 268 - protein, 46 aa, Bacteriophage D3821
MKTMDTYKEQFYYLDPIYISVDINRRTFILGKRGQSLSFFYCNKTI

SEQ ID NO: 269 - DNA, 225 bp, Bacteriophage O1205
atgacacaaattaaagatggttggcacatggtttatgacgaaaaagtgtatgtagagagcgggaaagttgtccgtggaataactaaagacaataacaattctgaaatagcttgctacccttacgaatacaacaaagactatgattgctggattaacatttctgggaaagtaactctatcagcttatagatcaggtcgtaaaaaagggacaaaatgtatgaagtga

SEQ ID NO: 270 - protein, 74 aa, Bacteriophage O1205
MTQIKDGWHMVYDEKVYVESGKVVRGITKDNNNSEIACYPYEYNKDYDCWINISGKVTLSAYRSGRKKGTKCMK

SEQ ID NO: 271 - DNA, 225 bp, Bacteriophage Sfi21
atgacacaaattaaagatggttggcacatagtttatgacgaaaaagtgtacgtagagagcgggaaagttgtccgtggaataactaaagacaataacaattctgaaatagcttgctacccttacgaatacaacgaagactatgattgctggattaacatttctgggaaagtaactctatcagcttatagatcaggtcgtaaaaaagggacaaaatgtatgaagtga

SEQ ID NO: 272 - protein, 74 aa, Bacteriophage Sfi21
MTQIKDGWHIVYDEKVYVESGKVVRGITKDNNNSEIACYPYEYNEDYDCWINISGKVTLSAYRSGRKKGTKCMK

SEQ ID NO: 273 - DNA, 153 bp, Bacteriophage D6264
ttgtttgaatgcttggcatcgtttcggttaaattctcgaactgtaacctcgactttttgtcggggttttctttttttacaaaaaaatctaaattcctttatcaaaagtgttgacaaactatcatatatgatatataatgtatacataagataa

SEQ ID NO: 274 - protein, 50 aa, Bacteriophage D6264
MFECLASFRLNSRTVTSTFCRGFLFLQKNLNSFIKSVDKLSYMIYNVYIR

SEQ ID NO: 275 - DNA, 192 bp, Bacteriophage D2759
atgaatgaaagtgaattgcttgagcagttctgcgtttctctttgtgaatttagctctagacagtggccacgagatgggtttttagaccctattaaccgtgtggtctacatcaatagggatttaccaaccgaaagacgtttaaaggtcctactgcacgaattagggcacttagaacacgaccctaaacactaa

SEQ ID NO: 276 - protein, 63 aa, Bacteriophage D2759
MNESELLEQFCVSLCEFSSRQWPRDGFLDPINRVVYINRDLPTERRLKVLLHELGHLEHDPKH

SEQ ID NO: 277 - DNA, 150 bp, Bacteriophage D4091
ttgttgggggctaagaccaccctttttgatataatatacctatatcaatggcttcccacgcatacgcgcagatacgttctgagggaagttttttatttgctttgttttgatagaaatgctactatattaatggatacagttaaaagctga

SEQ ID NO: 278 - protein, 49 aa, Bacteriophage D4091
MLGAKTTLFDIIYLYQWLPTHTRRYVLREVFYLLCFDRNATILMDTVKS

SEQ ID NO: 279 - DNA, 150 bp, Bacteriophage D5821
ttgttgggggttaagaccaccctttttgatataatatacctatatcaatggcttcccacgcatacgcgcagatacgttctgagggaagttttttatttgctttgttttgatagaaatgctactatattaatggatacagttaaaagctga

SEQ ID NO: 280 - protein, 49 aa, Bacteriophage D5821
MLGVKTTLFDIIYLYQWLPTHTRRYVLREVFYLLCFDRNATILMDTVKS

SEQ ID NO: 281 - DNA, 138 bp, Bacteriophage 5093
atgaggaggtgtcttttttttggtttgctcaaaaaacgcaacaatggtataataatttttgcaacgacaaaccccctgcaaccacatggacagatacgctctgacgcagggctttttttatttgctttatttttataa

SEQ ID NO: 282 - protein, 45 aa, Bacteriophage 5093
MRRCLFFGLLKKRNNGIIIFATTNPLQPHGQIRSDAGLFLFALFL

SEQ ID NO: 283 - DNA, 423 bp, Bacteriophage 5093
atgaaaatcaatacgacaagagttaaaatggtcttgaagaatgaggctatacctgctgattatttagagagcgagattggcattagtcgttccgttgttgaaaaagtgagagaagatgagagcgaatttaaaaatttaactcttgattttgttgcgaaaattcaaaagtggattgatgatggaaactacactttcagctatgattacagcgacttgatagaagagttggaagaagatattgcagaaggtctaacggatgagtatatctatgttgtcagaggacaatacaacgaaattttagagaaatgcccaataattgactactactacacttctgaagagattgaagaaggagatctcgcagagaagaccctaacagcttctgccttgtctgaaatgaaacaggacaacgaaatcttttaa

SEQ ID NO: 284 - protein, 140 aa, Bacteriophage 5093
MKINTTRVKMVLKNEAIPADYLESEIGISRSVVEKVREDESEFKNLTLDFVAKIQKWIDDGNYTFSYDYSDLIEELEEDIAEGLTDEYIYVVRGQYNEILEKCPIIDYYYTSEEIEEGDLAEKTLTASALSEMKQDNEIF

SEQ ID NO: 285 - DNA, 423 bp, Bacteriophage D4154
atgaaaatcaatacgacaagagttaaaatggtcttgaagaataaggttatacctgctatttatttagagaatgagcttggtatcagtcgttctgttattgaaaaagtgagagatggcgagcgaaaaatagagaatctaacgctcgaaacaattattaaagtccagaaatggatagattcgggcaaatataccttctcttatgattattccgacttgatagaagagttggaagaagatattgcagaaggcttggtagatgagtatatctacgtagtcagaggtccgtataatgaacttttagataaatgcccaataattgactactactacacttctgaagagattgaagaaggagatctcgcagagaagaccctaacagcttctgtcttggctgaaatgaaaaaggacaacgaaatcttttaa

SEQ ID NO: 286 - protein, 140 aa, Bacteriophage D4154
MKINTTRVKMVLKNKVIPAIYLENELGISRSVIEKVRDGERKIENLTLETIIKVQKWIDSGKYTFSYDYSDLIEELEEDIAEGLVDEYIYVVRGPYNELLDKCPIIDYYYTSEEIEEGDLAEKTLTASVLAEMKKDNEIF

SEQ ID NO: 287 - DNA, 423 bp, Bacteriophage D4160
atgaaaatcaatacgacaagaattaaaatggtcttgaagaatgaggctatacctgctatttatttagaaaatgagcttggtatcagtcgttctgttattgaaaaagtgagagaagacgagagcgaatttaaaaatctaactcttgatgttgttgcgaaaattcaaaagtggattgatgatggcaattacacgtttagttatgattacagtgaatttatcgaggaattagaagaagatctcgctgagggtttaatagatgattacctattcgttgttcgtggagattatgacgaagccttaggaaaatgtcccatcattgactattactacacttccgaagaaattgaagaaggagatctcgcagagaagaccctaacagcttctgtcttggctgaaatgaaaaaggacaacggaatcttttaa

SEQ ID NO: 288 - protein, 140 aa, Bacteriophage D4160
MKINTTRIKMVLKNEAIPAIYLENELGISRSVIEKVREDESEFKNLTLDVVAKIQKWIDDGNYTFSYDYSEFIEELEEDLAEGLIDDYLFVVRGDYDEALGKCPIIDYYYTSEEIEEGDLAEKTLTASVLAEMKKDNGIF

SEQ ID NO: 289 - DNA, 423 bp, Bacteriophage D5691
atgaaaatcaatacaacaagagtcaacatggtcttgaagaacgaggctatacctgctgattatttagagaacgtgattggtatcagtcgttccgttattgaaagagtgagagaagatgagagcggatttaaaaatttaactcttgatgttattgcgaaaattcaaaagtggatagatgaaggaaactacacgtttagttatgattacagcgacttgatagaagagttggaagaagatattgcagaaggcttggtagatgagtatatctacgtagtcagaggtccttataatgagattttagagaaatgcccaatcattgactactactacacttctgaagaaattgaagaaggagatctcgcagagaagaccctgacagcctctgccttagctgaaatgaagttagacaacaaaatcttttaa

SEQ ID NO: 290 - protein, 140 aa, Bacteriophage D5691
MKINTTRVNMVLKNEAIPADYLENVIGISRSVIERVREDESGFKNLTLDVIAKIQKWIDEGNYTFSYDYSDLIEELEEDIAEGLVDEYIYVVRGPYNEILEKCPIIDYYYTSEEIEEGDLAEKTLTASALAEMKLDNKIF

SEQ ID NO: 291 - DNA, 423 bp, Bacteriophage D7035
atgaaaatcaatacgacaagagttaacatggtcttgaagaacaaagctataccagctaattatttagaaaaggaactgggaataaaccgttcgacaattacaagagtgcggaacggtgagagaaagcttgagaatctaacgctcgaaacaatcataaaagtccagaaatggatagattcgggcaaatatacattctcttatgattattccgacttgatagaagagttggaagaagatattgaagaaggcctaacagatgagtatatctatgttgtcagaggtccgtataatgaacttttagagaaatgcccaataattgactactactacacttctgaagagattgaagaaggagatctcacagagaagaccctaacagcttctgccttggctgagatgaaacaggataacgaaatcttttaa

SEQ ID NO: 292 - protein, 140 aa, Bacteriophage D7035
MKINTTRVNMVLKNKAIPANYLEKELGINRSTITRVRNGERKLENLTLETIIKVQKWIDSGKYTFSYDYSDLIEELEEDIEEGLTDEYIYVVRGPYNELLEKCPIIDYYYTSEEIEEGDLTEKTLTASALAEMKQDNEIF

SEQ ID NO: 293 - DNA, 423 bp, Bacteriophage O1205
atgataataaacactgcacgagttgaattagttttaatgaacaaagctataccagcaaattatttagaaagcgaaataggtattagtcgttcagcaattactagggtaagaaatgatgagcgaaaaatagagaatctgaagctcgaaacaatcataaaagtccagaaatggatagattcgggcaaatacacattctcttatgattattccgacttgatagaagagttggaagaagatattgcaaaaggtctggcaggtaagtatatctacgttgtcagaggaccatacaacgagattttagagaaatgtccaatcattgactattactacacttccgaagagattgaagaaggagagctcgcagagaagaccttgacagcttctgtcttggctgaaatgaagtcagacaacgaaatcttttaa

SEQ ID NO: 294 - protein, 140 aa, Bacteriophage O1205
MIINTARVELVLMNKAIPANYLESEIGISRSAITRVRNDERKIENLKLETIIKVQKWIDSGKYTFSYDYSDLIEELEEDIAKGLAGKYIYVVRGPYNEILEKCPIIDYYYTSEEIEEGELAEKTLTASVLAEMKSDNEIF

SEQ ID NO: 295 - DNA, 396 bp, Bacteriophage Proph1
atggtcttgaagaacgaggctatacctgctgattatttagagagcgagattggcattagtcgttccgttgttgaaaaagtgagagaagatgagagcgaatttaaaaatttaactcttgatgttgttgcgaaaattcaaaagtggattgatgatggaaactacactttcagctatgattacagcgacctaatcgaagaactggaggaagatattgcagaaggcttggtagatgagtatatctacgtagtcagaggtccgtataatgaacttttagagaaatgcccaatcattgactactactatacttctgaagaaattgaagaaggggatcttgcagagaagaccttgataacttctgtcttagctgaaatgaagtcagacaacaaaatcttttaa

SEQ ID NO: 296 - protein, 131 aa, Bacteriophage Proph1
MVLKNEAIPADYLESEIGISRSVVEKVREDESEFKNLTLDVVAKIQKWIDDGNYTFSYDYSDLIEELEEDIAEGLVDEYIYVVRGPYNELLEKCPIIDYYYTSEEIEEGDLAEKTLITSVLAEMKSDNKIF

SEQ ID NO: 297 - DNA, 423 bp, Bacteriophage Sfi21
atgataataaatgttgcacgagttgaaacagttttaatgaacaatgctataccagctaattatttagaaagagaaataggaattagtcgttcagcaattactagggtaagaaacggtgagcgaaaaatagagaatctgaagctcgaaacaatcataaaagtccagaaatggatagattcgggcaaatatacattctcttatgattattccgacttgatagaagagttggaagaagatattgcagaaggactaacggatgagtatatctacgttgtcagaggagcatacaacgagattttagagaaatgcccaatcattgactattactacacttccgaagagattgaagaaggagatctcgcagagaagaccctaacagcttctgccttgtctgaaatgaaacaggacaacgaaatcttttaa

SEQ ID NO: 298 - protein, 140 aa, Bacteriophage Sfi21
MIINVARVETVLMNNAIPANYLEREIGISRSAITRVRNGERKIENLKLETIIKVQKWIDSGKYTFSYDYSDLIEELEEDIAEGLTDEYIYVVRGAYNEILEKCPIIDYYYTSEEIEEGDLAEKTLTASALSEMKQDNEIF

SEQ ID NO: 299 - DNA, 423 bp, Bacteriophage TP-778L
atgataataaacactgcacgagttgaattagttttaatgaacaaagctataccagcaaattatttagaaagagagataggaattagtcgttcagcaattacaagagttcggaacggtgagagaaagcttgagaacctaacccttgaaactattatgactattcaaaagtggatagatgaaggaaactatcgctttagttacgattatagtgagcttatcgaagaccttgaggaagatattgcagaaggcctaacagatgagtatatctatgttgtcagaggtccgtataatgaacttttagagaaatgtccaatcattgactattactacacttccgaagagattgaagaaggaaatctcgcagagaagaccttgacagcttctgtcttggctgaaatgaaacaggacaacgaaatattttaa

SEQ ID NO: 300 - protein, 140 aa, Bacteriophage TP-778L
MIINTARVELVLMNKAIPANYLEREIGISRSAITRVRNGERKLENLTLETIMTIQKWIDEGNYRFSYDYSELIEDLEEDIAEGLTDEYIYVVRGPYNELLEKCPIIDYYYTSEEIEEGNLAEKTLTASVLAEMKQDNEIF

SEQ ID NO: 301 - DNA, 423 bp, Bacteriophage TP-J34
atgaaaatcaatacgacaagaattaaaatggtcttgaagaatgaggctatacctgctatttatttagaaaatgagcttggtatcagtcgttctattattgaaaaagtgagagatgatgagagcgaatttaaaaatctaactcttgaaactattataaaaatacaaagtttgataaattcgggcaaatatacattctcttatgattattccgacttgatagaagagttggaagaagatattgcagaaggactaacggatgagtatatctacgttgtcagaggaccatacaacgagattttagagaaatgtccaatcattgactattactacacttccgaagagattgaagaaggaaatctcgcagagaagaccttgacagcttctgtcttggctgaaatgaaacaggacaacgaaatattttaa

SEQ ID NO: 302 - protein, 140 aa, Bacteriophage TP-J34
MKINTTRIKMVLKNEAIPAIYLENELGISRSIIEKVRDDESEFKNLTLETIIKIQSLINSGKYTFSYDYSDLIEELEEDIAEGLTDEYIYVVRGPYNEILEKCPIIDYYYTSEEIEEGNLAEKTLTASVLAEMKQDNEIF

SEQ ID NO: 303 - DNA, 423 bp, Bacteriophage Proph1
atgaaaatcaatacgacaagagttaaaatggtcttgaagaatgaggttatacctgctatttatttagagaatgagcttggtatcagtcgttctgttattgaaaaagtgagagatggcgagcgaaaaatagagaatctaactcttgaaacgattataaaaattcaaaagtggatcgatgatggaaactacactttcagctacgactatagcgacctaatcgaagaactggaggaagatattgcagaaggcttggtagatgagtatatctacgtagtcagaggtccgtataatgaacttttagagaaatgcccaatcattgactactactatacttctgaagaaattgaagaaggggatcttgcagagaagaccttgataacttctgtcttagctgaaatgaagtcagacaacaaaatcttttaa

SEQ ID NO: 304 - protein, 140 aa, Bacteriophage Proph1
MKINTTRVKMVLKNEVIPAIYLENELGISRSVIEKVRDGERKIENLTLETIIKIQKWIDDGNYTFSYDYSDLIEELEEDIAEGLVDEYIYVVRGPYNELLEKCPIIDYYYTSEEIEEGDLAEKTLITSVLAEMKSDNKIF

SEQ ID NO: 305 - DNA, 183 bp, Bacteriophage D1126
atggaccaagttaaattagttttaatgaacaaagctataccagctaattatttagaaagacaaactggtgttagtcgttcagcaattactagggttagaaatggcgagcgaaaaatagaaaatctaacacttgaaacaattattaaaattcaaagttggatagactctgagaatacgatatag

SEQ ID NO: 306 - protein, 60 aa, Bacteriophage D1126
MDQVKLVLMNKAIPANYLERQTGVSRSAITRVRNGERKIENLTLETIIKIQSWIDSENTI

SEQ ID NO: 307 - DNA, 195 bp, Bacteriophage D1128
atgataattaatgtggaccgagttaaagcggttttaatggataaatctataccggcaaattatttagaaatgcaaactggcattagtcgttcggcaattaccagagtaaggaacggcgagcgaaagatagaaaatctaactatcggaacaattattaaaattcaaagttggttggatagaaggatgattagataa

SEQ ID NO: 308 - protein, 64 aa, Bacteriophage D1128
MIINVDRVKAVLMDKSIPANYLEMQTGISRSAITRVRNGERKIENLTIGTIIKIQSWLDRRMIR

SEQ ID NO: 309 - DNA, 183 bp, Bacteriophage D4250
atggaccgagttaaattagttttaatgaacaaagctataccagcaaattttttagaaagacaaactggagttagtcgttcagcaattactagggttagaaataacgagcgaaaaatagaaaatctaacacttgaaacaattattaaaattcaaagttggatagattctgacaatacgatatag

SEQ ID NO: 310 - protein, 60 aa, Bacteriophage D4250
MDRVKLVLMNKAIPANFLERQTGVSRSAITRVRNNERKIENLTLETIIKIQSWIDSDNTI

SEQ ID NO: 311 - DNA, 228 bp, Bacteriophage D4252
ttgggaagaaggataaggataaagataaagataatgataataaatatggaccaagttaaattagttttaatgaacaaagatataccagctaattttatagaaagacaaactggtgttagtcgttcagcaattactaaggttagaaatggtgagcgaaaaatagaaaatctaagacttgaaacaattattaaaattcaaagttggatagactctgggaatacgatatag

SEQ ID NO: 312 - protein, 75 aa, Bacteriophage D4252
MGRRIRIKIKIMIINMDQVKLVLMNKDIPANFIERQTGVSRSAITKVRNGERKIENLRLETIIKIQSWIDSGNTI

SEQ ID NO: 313 - DNA, 216 bp, Bacteriophage D4273
ttgggaagtaggataaggataatgataattaatgtggaccgagttaaagcggttttaatggataaatctataccggcaaattatttagaaatgcaaactggcattagtcgttcggcaattaccagagtaaggaacggcgagcgaaagatagaaaatctaactatcggaacaattattaaaattcaaagttggttggatagaaggatgattagataa

SEQ ID NO: 314 - protein, 71 aa, Bacteriophage D4273
MGSRIRIMIINVDRVKAVLMDKSIPANYLEMQTGISRSAITRVRNGERKIENLTIGTIIKIQSWLDRRMIR

SEQ ID NO: 315 - DNA, 195 bp, Bacteriophage D4276
atgataataaatatggaccgagttaaattagttttaatgaacaaagatataccagctaattttttagaaagacaaactggtgttagtcgttcagcaattactaaggttagaaatggtgagcgaaaaatagaaaatctaacacttgaaacaattattaaaattcaaagttggttagactctgagaatacgatatag

SEQ ID NO: 316 - protein, 64 aa, Bacteriophage D4276
MIINMDRVKLVLMNKDIPANFLERQTGVSRSAITKVRNGERKIENLTLETIIKIQSWLDSENTI

SEQ ID NO: 317 - DNA, 195 bp, Bacteriophage D6252
atgataataaacactgcacgagttgaattagttttaatgaacaaagctataccagctaattttttagaaagacaaactggtgttagtcgttcagcaattactagggttagagatggtgagcgaaagatagaaaatctaacacttgaaacaattattaaaattcaaagttggatagactctgacaataagatatag

SEQ ID NO: 318 - protein, 64 aa, Bacteriophage D6252
MIINTARVELVLMNKAIPANFLERQTGVSRSAITRVRDGERKIENLTLETIIKIQSWIDSDNKI

SEQ ID NO: 319 - DNA, 216 bp, Bacteriophage D6938
atgacaaaaaggataaagacaatgataataaatatggaccgagttaaattagttttaatgaaaaaagatataccagctaattttttagaaagacaaactggtgttagtcgttcagcaattactagggttagaaatggtgagcgaaaaatagaaaatctaacacttgaaacaattattaaaattcaaagttggatagactctgagaatacgatatag

SEQ ID NO: 320 - protein, 71 aa, Bacteriophage D6938
MTKRIKTMIINMDRVKLVLMKKDIPANFLERQTGVSRSAITRVRNGERKIENLTLETIIKIQSWIDSENTI

SEQ ID NO: 321 - DNA, 195 bp, Bacteriophage D7163
atgataataaacactgcacgagttgaattagttttaatgaacaaagctataccagcaaattatttagaaagacaaactggtgttagtcgttcagcaattactagggtgaggaatggtgagcgaaagatagaaaatctaacacttgaaacaattattaaaattcaaagttggatagactctgacaataagatatag

SEQ ID NO: 322 - protein, 64 aa, Bacteriophage D7163
MIINTARVELVLMNKAIPANYLERQTGVSRSAITRVRNGERKIENLTLETIIKIQSWIDSDNKI

SEQ ID NO: 323 - DNA, 195 bp, Bacteriophage P4761
atgataattaatgtggaccgagttaaagcggttttaatggataaatctatatcagcaaattatttagaaatagaaactggcattagtcgttcggcaattaccagagtaaggaacggcgagcgaaagatagaaaatctaactatcggaacaattattaaaattcaaagttggttggatagaaggatgattagataa

SEQ ID NO: 324 - protein, 64 aa, Bacteriophage P4761
MIINVDRVKAVLMDKSISANYLEIETGISRSAITRVRNGERKIENLTIGTIIKIQSWLDRRMIR

SEQ ID NO: 325 - DNA, 513 bp, Bacteriophage D4090
atggtagtaaaaattaaaagaattgtttgggttaaaaataatggttttgaaatcagagaacgtgagctagattgttactttaaaaatgatggaagttacaaaaagagttctggagattgggaaagtcgttgttatgaacaattcggagatgaatttcaactcattagagatagcaaagcattagaatcttatagtggtttgacaagagattatcaaaaagacttaaaaatcttgcgtaagtataaacatagagatatgactatttcagagtatgaagcaatgaaatatgtcgtggagaattggacaaaagaatggtctcagtcaccttacagttatagtttttatagttcaaaaaacattgactggggttacaaaccagaaggcagcttacgcatttctgaccattggaattttggcgaaaatggtgaacattgcccaacagctgaaccagttgatggctgggcagtatgtaagtttgaaaatggtaaatatcatttaattaaaaagttttaa

SEQ ID NO: 326 - protein, 170 aa, Bacteriophage D4090
MVVKIKRIVWVKNNGFEIRERELDCYFKNDGSYKKSSGDWESRCYEQFGDEFQLIRDSKALESYSGLTRDYQKDLKILRKYKHRDMTISEYEAMKYVVENWTKEWSQSPYSYSFYSSKNIDWGYKPEGSLRISDHWNFGENGEHCPTAEPVDGWAVCKFENGKYHLIKKF

SEQ ID NO: 327 - DNA, 513 bp, Bacteriophage D4254
atggtagtaaaaattaaaagaattgtttgggttaaaaataatggttttgaaatcagagaacgtgagctagattgttactttaaaaatgatggaagttacaaaaaaagttctggagattgggaaagtcgttgttatgaacaattcggagatgaatttcaactcattagagatagcaaagcattagaatcttatagtggtttgacaagagattatcaaaaagacttaaaaatcttgcgtaagtataaacatagagatatgactatttcagagtatgaagcaatgaaatatgtcgtggagaattggacaaaagagtggtcacaatcaccatacagcaatagtttctatagctctaaagatattgattggggctacaaaccagaaggtagcttaagagtctcagaccattggaattttggcgaaaatggtgaacattgcccaacagctgaaccagttgatggctgggcagtatgtaagtttgaaaatggtaaatatcatttaattaaaaagttttaa

SEQ ID NO: 328 - protein, 170 aa, Bacteriophage D4254
MVVKIKRIVWVKNNGFEIRERELDCYFKNDGSYKKSSGDWESRCYEQFGDEFQLIRDSKALESYSGLTRDYQKDLKILRKYKHRDMTISEYEAMKYVVENWTKEWSQSPYSNSFYSSKDIDWGYKPEGSLRVSDHWNFGENGEHCPTAEPVDGWAVCKFENGKYHLIKKF

SEQ ID NO: 329 - DNA, 474 bp, Bacteriophage D4368
atggtagtaaaaattaaaagaattgtttgggttaaaaataatggttttgaaatcagagaacgtgagctagattgttactttaaaaatgatggaagttacaaaaagagttctggagattgggaaagtcgttgttatgaacaattcggtaataaacttcaacttattaaagacagtaaaaaattagaatcgtacaacggattaacaaaagattatcaaaaagatttaaaaatcttacgtaaatgtggacgttcggaaatgaatgcaacagagtacgaagcaatgaaatatgttgaagaaaactggacaaaagagtggtcacaatcaccatacagcaatagtttctatagctctaaagatattgattggggctacaaaccagaaggtagcttaagagtctcagaccattggaattttggcgaaaatggtgaacattgcccaacagctgaaccagttgatggctgggcagtattttga

SEQ ID NO: 330 - protein, 157 aa, Bacteriophage D4368
MVVKIKRIVWVKNNGFEIRERELDCYFKNDGSYKKSSGDWESRCYEQFGNKLQLIKDSKKLESYNGLTKDYQKDLKILRKCGRSEMNATEYEAMKYVEENWTKEWSQSPYSNSFYSSKDIDWGYKPEGSLRVSDHWNFGENGEHCPTAEPVDGWAVF

SEQ ID NO: 331 - DNA, 513 bp, Bacteriophage D5700
atggtagtaaaaattaaaagaattgtttgggttaaaaataatggttttgaaatcagagaacgtgagctagattgttactttaaaaatgatggaagttacaaaaaaagttctggagattgggaaagtcgttgttatgaacaattcggagatgaatttcagctcattagagatagcaaagcattagaatcttatagtggtttgacaagagattatcaaaaagacttaaaaatcttgcgtaagtataaacatagagatatgactatttcagagtatgaagcaatgaaatatgtcgtggagaattggacaaaagagtggtcacaatcaccatacagcaatagtttctatagctctaaagatattgattggggctacaaaccagaaggtagcttaagagtctcagaccattggaattttggcgaaaatggtgaacattgcccaacagctgaaccagttgatggctgggcagtatgtaagtttgaaaatggtaaatatcatttaattaaaaagttttaa

SEQ ID NO: 332 - protein, 170 aa, Bacteriophage D5700; identical to SEQ ID NO: 328

SEQ ID NO: 333 - DNA, 513 bp, Bacteriophage D7059
atggtagtaaaaattaaaagaattgtttgggttaaaaataatggttttgaaatcagagaacgtgagctagattgttactttaaaaatgatggaagttacaaaaaaagttctggagattgggaaagtcgttgttatgaacaattcggagatgaatttcaactcattagagataacaaagcattagaatcttatagtggtttgacaagagattatcaaaaagacttaaaaatcttgcgtaagtataaacatagagatatgactatttcagagtatgaagcaatgaaatatgtcgtggagaattggacaaaagagtggtcacaatcaccatacagcaatagtttctatagctctaaagatattgattggggctacaaaccagaaggtagcttaagagtctcagaccattggaattttggcgaaaatggtgaacattgcccaacagctgaaccagttgatggctgggcagtatgtaagtttgaaaatggtaaatatcatttaattaaaaagttttaa

SEQ ID NO: 334 - protein, 170 aa, Bacteriophage D7059
MVVKIKRIVWVKNNGFEIRERELDCYFKNDGSYKKSSGDWESRCYEQFGDEFQLIRDNKALESYSGLTRDYQKDLKILRKYKHRDMTISEYEAMKYVVENWTKEWSQSPYSNSFYSSKDIDWGYKPEGSLRVSDHWNFGENGEHCPTAEPVDGWAVCKFENGKYHLIKKF

SEQ ID NO: 335 - DNA, 513 bp, Bacteriophage D7108
atggtagtaaaaattaaaagaattgtttgggttaaaaataatggttttgaaatcagagaacgtgagctagattgttactttaaaaatgatggaagttacaaaaaaagttctggagattgggaaagtcgttgttatgaacaattcggagatgaatttcaactcattagagataacaaagcattagaatcttatagtggtttgacaagagattatcaaaaagacttaaaaatcttgcgtaagtataaacatagagatatgactatttcagagtatgaagcaatgaaatatgtcgtggagaattggacaaaagagtggtcacaatcaccatacagcaatagtttttatagctctaaagatattgattggggctacaaaccagaaggtagcttaagagtctcagaccattggaattttggcgaaaatggtgaacattgcccaacagctgaaccagttgatggctgggcagtatgtaagtttgaaaatggtaaatatcatttaattaaaaagttttaa

SEQ ID NO: 336 - protein, 170 aa, Bacteriophage D7108; identical to SEQ ID NO: 334

SEQ ID NO: 337 - DNA, 225 bp, Bacteriophage D4090
atgattaaaacggaaatgattgacgatattctcactttgattgaagaaattgaagctgttagcgataagaataaagaaaagtttattgaaaaatttgacgagttagaaaccaatttacaagcattgaataaacaaaccactgatgatttggttgaaattttacaagaagattattctgataattgggtagcaaaagaggtgattgaacttgttactaacagctag

SEQ ID NO: 338 - protein, 74 aa, Bacteriophage D4090
MIKTEMIDDILTLIEEIEAVSDKNKEKFIEKFDELETNLQALNKQTTDDLVEILQEDYSDNWVAKEVIELVTNS

SEQ ID NO: 339 - DNA, 225 bp, Bacteriophage D4368
atgaataaaatagaaatgattgacgatattctcactttgattgaagagattgacgccattagtgataagagtaaagaaacgttttttgaaaaaattgatgagttggaaacaaatttacaagcattgaacagacaaatcactgatgaattggttgaaattttacaagaagattattctgataattgggtagcaaaagaggtgattgaacttgttactaacagctag

SEQ ID NO: 340 - protein, 74 aa, Bacteriophage D4368
MNKIEMIDDILTLIEEIDAISDKSKETFFEKIDELETNLQALNRQITDELVEILQEDYSDNWVAKEVIELVTNS

SEQ ID NO: 341 - DNA, 225 bp, Bacteriophage D5700
atgattaaaacggaaatgattgacgatattctcactttgattgaagaaattgaagctgttagcgataagaataaagaaaagtttattgaaaaatttgacgagttagaaaccaatttacaagcattgaataaacaaaccactgatgatttggttgaaattttacaagaagattattctgataattgggtagcaaaagaggtgattgaacttgtcgatgactactag

SEQ ID NO: 342 - protein, 74 aa, Bacteriophage D5700
MIKTEMIDDILTLIEEIEAVSDKNKEKFIEKFDELETNLQALNKQTTDDLVEILQEDYSDNWVAKEVIELVDDY

SEQ ID NO: 343 - DNA, 225 bp, Bacteriophage D6961
atgattaaaacggaaatgattgacgatattctcactttgattgaagaaattgaagctgttagcgataagaataaagaaaagtttattgaaaaatttgatgagttagaaaccaatttacaagcattgaataaacaaaccactgatgatttggttgaaattttacaagaagattattctgataattgggtagcaaaagaggtgattgaacttgtcgatgactactag

SEQ ID NO: 344 - protein, 74 aa, Bacteriophage D6961; identical to SEQ ID NO: 342

SEQ ID NO: 345 - DNA, 513 bp, Bacteriophage D4090
atgagttatacaagcccagtttataacattaaacgagtacccattgacaaaatccaagcaaacagttataatccaaatcatgtagcacctcccgaaatgaaattgctttataagtctattttagaggacggatacactatgccaatcgtttgttattatcttaaagacgaggataaatacgagattgtagacggttttcaccgttacagcactatgcttaaccacaaagatatttatgaacgtgagggtggttgtttgccagtatccgttattgataagccaattagcgaccgcatggcgtcaactatccgacacaatcgagcgagagggtcacatgatatcgacctaatgacaaacattgtcgctgaccttgtagacagtggtatgtctgacgcttggattttaaaaaatatcggaatggacgcagacgaattgttgcgtttgaaacaattaactggtttagcgagtttgtttgcagacaaagaattcagtaaatcatgggatgtagaataa

SEQ ID NO: 346 - protein, 170 aa, Bacteriophage D4090
MSYTSPVYNIKRVPIDKIQANSYNPNHVAPPEMKLLYKSILEDGYTMPIVCYYLKDEDKYEIVDGFHRYSTMLNHKDIYEREGGCLPVSVIDKPISDRMASTIRHNRARGSHDIDLMTNIVADLVDSGMSDAWILKNIGMDADELLRLKQLTGLASLFADKEFSKSWDVE

SEQ ID NO: 347 - DNA, 513 bp, Bacteriophage D4368
atgagttatacaagcccagtttataacattaaacgagtacccattgacaaaatccaagcaaacagttataatccaaatcatgtagcacctcccgaaatgaaattgctttataagtctattttagaggacggatacactatgccaatcgtttgttattatcttaaagacgaggataaatacgagattgtagacggttttcaccgttacagcactatgcttaaccacaaagatatttatgaacgtgagggtggttgtttgccagtatccgttattgataagccaattagcgaccgcatggcgtcaactatccgacacaatcgagcgagagggtcacatgatatcgacctaatgacaaacattgtcgctgaccttgtagacagtggtatgtctgacgcttggattttaaaaaatatcggaatggacgcagacgaattgttgcgtttgaaacaattaactggcttgtcgagtttgtttgcagacaaagaattcagtaaatcatgggatgtagaataa

SEQ ID NO: 348 - protein, 170 aa, Bacteriophage D4368
MSYTSPVYNIKRVPIDKIQANSYNPNHVAPPEMKLLYKSILEDGYTMPIVCYYLKDEDKYEIVDGFHRYSTMLNHKDIYEREGGCLPVSVIDKPISDRMASTIRHNRARGSHDIDLMTNIVADLVDSGMSDAWILKNIGMDADELLRLKQLTGLSSLFADKEFSKSWDVE

SEQ ID NO: 349 - DNA, 513 bp, Bacteriophage D4598
atgagttacacaagtccagtttataacattaaacgagtacccattgacaaaattcaggcaaacagttataatccaaaccatgtagcacctcctgaaatgaaactactttacaagtctattttagaggatggatacacaatgccaatcgtttgttattatcttaaagatgaagataaatatgagattgtagatggctttcaccgttatagcactatgcttaaccacaaagatatttatgaccgtgagggcggttgtttgccagtatccgttattaataagccaatcagtgaccgtatggcatcaactatccgacataatcgagcgagagggtcacatgatattgacctaatgacaaacattgtcgctgaccttgtagacagtggtatgtctgacgcttggattttaaaaaatatcggaatggacgcagacgaattgttgcgtttgaaacaattaactggcttggcaagtttgtttgcagacaaagaattcagtaaatcatgggatgtagaataa

SEQ ID NO: 350 - protein, 170 aa, Bacteriophage D4598
MSYTSPVYNIKRVPIDKIQANSYNPNHVAPPEMKLLYKSILEDGYTMPIVCYYLKDEDKYEIVDGFHRYSTMLNHKDIYDREGGCLPVSVINKPISDRMASTIRHNRARGSHDIDLMTNIVADLVDSGMSDAWILKNIGMDADELLRLKQLTGLASLFADKEFSKSWDVE

SEQ ID NO: 351 - DNA, 513 bp, Bacteriophage D5700
atgagttatacaagcccagtttataacattaaacgagtacccattgacaaaatccaagcaaatagttataatccaaatcatgtagcacctcccgaaatgaaattgctttataagtctattttagaggacggatacactatgccaatcgtttgttattatcttaaagacgaggataaatacgagattgtagacggttttcaccgttacagcactatgcttaaccacaaagatatttatgaacgtgagggtggttgtttgccagtatccgttattgataagccaattagcgaccgcatggcgtcaactatccgacacaatcgagcgagagggtcacatgatatcgacctaatgacaaacattgtcgctgaccttgtagacagtggtatgtctgacgcttggattttaaaaaatatcggaatggacgcagacgaattgttgcgtttgaaacaattaactggcttggcaagtttgtttgcagacaaagaattcagtaaatcatgggatgtagaataa

SEQ ID NO: 352 - protein, 170 aa, Bacteriophage D5700; identical to SEQ ID NO: 346

SEQ ID NO: 353 - DNA, 513 bp, Bacteriophage D6938
atgagttacacaagtccagtttataacattaaacgagtacctattgataaaattcaggcaaacagttataatccaaaccatgtagcacctcctgaaatgaaactactttacaagtctattttagaggatgggtacacaatgccaatcgtttgttattatcttaaagatgaagataaatatgagattgtagatggctttcatcgctatagcactatgcttaaccacaaagatatttatgaccgtgagggcggttgtttgccagtatccgttattaataaaccgattagtgaccgcatggcgtcaactatccgacacaaccgggcgagagggtcacatgatattgacctaatgacaaacattgttgctgaccttgtagatagtggcatgtctgacgcttggattttgaaaaatatcggaatggacgcagacgaattgttgcggttgaaacagttaactggtttagctagtctatttgcagacaaagaattcagtaaatcgtggatcgtagaataa

SEQ ID NO: 354 - protein, 170 aa, Bacteriophage D6938
MSYTSPVYNIKRVPIDKIQANSYNPNHVAPPEMKLLYKSILEDGYTMPIVCYYLKDEDKYEIVDGFHRYSTMLNHKDIYDREGGCLPVSVINKPISDRMASTIRHNRARGSHDIDLMTNIVADLVDSGMSDAWILKNIGMDADELLRLKQLTGLASLFADKEFSKSWIVE

SEQ ID NO: 355 - DNA, 513 bp, Bacteriophage D7059
atgagttacacaagtccagtttataacattaaacgagtacccattgacaaaatccaagcaaacagttataatccaaatcatgtagcacctcccgaaatgaaattgctttataagtctattttagaggacggatacactatgccaatcgtttgttattatcttaaagacgaggataaatacgagattgtagacggttttcaccgttacagcactatgcttaaccacaaagatatttatgaacgtgagggtggttgtttgccagtatccgttattgataagccaattagcgaccgcatggcgtcaactatccgacacaatcgagcgagagggtcacatgatatcgacctaatgacaaacattgtcgccgaccttgtagacagtggtatgtctgacgcttggattttaaaaaatatcggaatggacgcagacgaattgttgcgtttgaaacaattaactggcttggcaagtttgtttgcagacaaagaattcagtaaatcatgggatgtagaataa

SEQ ID NO: 356 - protein, 170 aa, Bacteriophage D7059; identical to SEQ ID NO: 346

SEQ ID NO: 357 - DNA, 180 bp, Bacteriophage D4090
atgcctaaagtttccgagagcaaacggaaagcaaatgacaaatgggacaaaaagaacaaagaacgcaagcagtatatcaacagacgttctgtcgcaaggaactttattaagaatatggaaggcgaagatattccagaatttaaaaaactaatagaagaaagagcttccaaaatcaaataa

SEQ ID NO: 358 - protein, 59 aa, Bacteriophage D4090
MPKVSESKRKANDKWDKKNKERKQYINRRSVARNFIKNMEGEDIPEFKKLIEERASKIK

SEQ ID NO: 359 - DNA, 180 bp, Bacteriophage D4254
atgcctaaagtttccgagagcaaacggaaagcaaatgacaaatgggacaaaaagaacaaagaacgcaagcagtatattaacagacgttctgtcgcaaggaactttattaagaatatggaagacgaagatattccagaatttaaaaaactaatggaagaaagagcttccaaaatcaaataa

SEQ ID NO: 360 - protein, 59 aa, Bacteriophage D4254
MPKVSESKRKANDKWDKKNKERKQYINRRSVARNFIKNMEDEDIPEFKKLMEERASKIK

SEQ ID NO: 361 - DNA, 180 bp, Bacteriophage D4368
atgcctaaagtttccgagagcaaacggaaagcaaatgacaaatgggacaaaaagaacaaagaacgcaagcagtatattaacagacgttctgtcgcaaggaactttattaagaatatggaagacgaagatattccagaatttaaaaaactaatggaagaaagaacttccaaaatcaaataa

SEQ ID NO: 362 - protein, 59 aa, Bacteriophage D4368
MPKVSESKRKANDKWDKKNKERKQYINRRSVARNFIKNMEDEDIPEFKKLMEERTSKIK

SEQ ID NO: 363 - DNA, 198 bp, Bacteriophage D6961
atgcctaaagtctcagaaagcaaacggagagcgaataataaatgggataaaaaaaataaagaacgtaaacaatatataaacaaacgttccgttgcaagaaactttattaagaacatggaagatgaagatgttccggaatttaaaaaactaatggaagaaagagcttccaaaacaaataaaacgtgttttagttcatga

SEQ ID NO: 364 - protein, 65 aa, Bacteriophage D6961
MPKVSESKRRANNKWDKKNKERKQYINKRSVARNFIKNMEDEDVPEFKKLMEERASKTNKTCFSS

SEQ ID NO: 365 - DNA, 180 bp, Bacteriophage D7059
atgcctaaagtttccgagagcaaacggaaagcaaacgacaaatgggataaaaataacaaagaacgcaagcagtatattaacagacgttctgtcgcaaggaactttattaagaatatggaagacgaagatattccagaatttaaaaaactaatggaagaaagaacttccaaaatcaaataa

SEQ ID NO: 366 - protein, 59 aa, Bacteriophage D7059
MPKVSESKRKANDKWDKNNKERKQYINRRSVARNFIKNMEDEDIPEFKKLMEERTSKIK

SEQ ID NO: 367 - DNA, 246 bp, Bacteriophage D4250
atgaagttaactaatcaacagaatcaagcctttaagaaattcaaaaatttgagagttggagctctatttatggagcaaggaacaggtaagacaagagtagcactagagttaatcagaaaaacagatgctgatttagccttgttcttttgtccgttttcaaccaaaaacaatcttttatctgagattgaaaaatggggaattgatattgaatttatggtgtatggatatgaaacgatttcatcatag

SEQ ID NO: 368 - protein, 81 aa, Bacteriophage D4250
MKLTNQQNQAFKKFKNLRVGALFMEQGTGKTRVALELIRKTDADLALFFCPFSTKNNLLSEIEKWGIDIEFMVYGYETISS

SEQ ID NO: 369 - DNA, 177 bp, Bacteriophage D4254
gtggaaacagaaccaaattttcaaataatatgttataataaaagtacctcgtttgaggtatttttttatcttacaactgcacccgaattttttcaggtgtttttttttcgcccaaaaatcacccgaaaactttgggaaaagctagaaaaaataaaaataaacgaggtaaaaacatag

SEQ ID NO: 370 - protein, 58 aa, Bacteriophage D4254
METEPNFQIICYNKSTSFEVFFYLTTAPEFFQVFFFRPKITRKLWEKLEKIKINEVKT

SEQ ID NO: 371 - DNA, 204 bp, Bacteriophage D6961
gtggaaacagaaccaaattttcaaataatatgttataataaaagtacctcgtttgaggtattttttatcttacaactgcacccgaattttttcaggtgttttttttgcccaaaaatcacccaaaaactttgggaaaagctagaaaaaataaaaaataaacgaggtaaaaacatagtatgttttactaattttcaagctgattaa

SEQ ID NO: 372 - protein, 67 aa, Bacteriophage D6961
METEPNFQIICYNKSTSFEVFFILQLHPNFFRCFFCPKITQKLWEKLEKIKNKRGKNIVCFTNFQAD

SEQ ID NO: 373 - DNA, 159 bp, Bacteriophage D4263
atgggttttacggttacatgttgcaataacctgcggtcactgagtaaccataaccactactgctgctttcttcgcctcgttttcgtcccaactaaaattgaaatcataccaataatctggtttatctttagggtgtctcacggatttcaaacggtgtga

SEQ ID NO: 374 - protein, 52 aa, Bacteriophage D4263
MGFTVTCCNNLRSLSNHNHYCCFLRLVFVPTKIEIIPIIWFIFRVSHGFQTV

SEQ ID NO: 375 - DNA, 453 bp, Bacteriophage D4445
ttggaatacttggcatcgtttcggttaaattctcgaactgtaacctcgacttttagtcgaggttttctttttttgcaaaaaaaactaaattccttaataaataaaaataaaaactataaaaacttagtacagcttcatttattctcaaattttatatattttcgttcaagaattgttctgttgttaaacctaaagcgcgagcgaaatcatcagctttattcagcgggaacacccgactacctgaaagatatcttgtttgaaatcccagctttatttgcattgacatggaactgttgtctaaatagctttttattatcgttgtttctcatatttaatagtataaacattatacaaaagttcccaaaaataaacaatatgttcccaaaaataaacttttttcatatttttttgattttagtgttgacaaatgggaacgtgttagatatactataa

SEQ ID NO: 376 - protein, 150 aa, Bacteriophage D4445
MEYLASFRLNSRTVTSTFSRGFLFLQKKLNSLINKNKNYKNLVQLHLFSNFIYFRSRIVLLLNLKRERNHQLYSAGTPDYLKDILFEIPALFALTWNCCLNSFLLSLFLIFNSINIIQKFPKINNMFPKINFFHIFLILVLTNGNVLDIL

SEQ ID NO: 377 - DNA, 282 bp, Bacteriophage D4446
atggaagttgaacaaagactagaacaactaagacaagattggttgaaacacccaaatttaacagatactttaaaagaatatctaaacgaatatttttacgatgattattcttattgtgagaaatgtgataggattgccagcgatagcgattggttttggtatgaaggcgaagactatacggattttttacacattgattgtaataaagaaaaattttacgaagcaacaaaaaaaacctctggaaggaggagaccagaggaaaacataaaaggagaaagttag

SEQ ID NO: 378 - protein, 93 aa, Bacteriophage D4446
MEVEQRLEQLRQDWLKHPNLTDTLKEYLNEYFYDDYSYCEKCDRIASDSDWFWYEGEDYTDFLHIDCNKEKFYEATKKTSGRRRPEENIKGES

SEQ ID NO: 379 - DNA, 228 bp, Bacteriophage D4446
atgaaaactaagacacttgggcgccgtttaagacgtttaagaaaaatcaatggagaaacacaaaaggaatttgccgaaaattttggaagacattatagaaccgttcaaaattgggagctagattgttcaataccagacgttttcacagcaatggcattggcagaatattataacatggacgttgaagaattggtgaatggagaagatgactatgacaaagaattttga

SEQ ID NO: 380 - protein, 75 aa, Bacteriophage D4446
MKTKTLGRRLRRLRKINGETQKEFAENFGRHYRTVQNWELDCSIPDVFTAMALAEYYNMDVEELVNGEDDYDKEF

SEQ ID NO: 381 - DNA, 378 bp, Bacteriophage D4446
atggagaagatgactatgacaaagaattttgaaaattttaaaaaaggctgggataatgttcaacaagtagtaaatgaatacagcaaaaaactcgttgaaaacagtcaagaaaatgtaaccaaccgagatagtgaagagtatcagcaaatcaaaggtaaagataacgtaattagtccaaaccactatgtaaccgataagggttttgaagtgtttgacgtgcaagaagcttttatccacgaattaaaaggaatggcagctagttactggtgcaatgttgtgaagtatattttgagatttcaaagaaagaatggagtggaagacttaaaaaaagctaagtactacttggaaaaattaattgaaaaagaggaaggtaaataa

SEQ ID NO: 382 - protein, 125 aa, Bacteriophage D4446
MEKMTMTKNFENFKKGWDNVQQVVNEYSKKLVENSQENVTNRDSEEYQQIKGKDNVISPNHYVTDKGFEVFDVQEAFIHELKGMAASYWCNVVKYILRFQRKNGVEDLKKAKYYLEKLIEKEEGK

SEQ ID NO: 383 - DNA, 546 bp, Bacteriophage D4446
atgaataaacaagaagcaattgaactagtaaaaaatacttcatacagtgtaccaattgatagcccagtgaaacatcttacagaagatacagttatcaatattatcaaacagcttgatgaaccagagaaagctacagtgccagattttgtagcaaaatacattgaagaaagcagagaatttgacagaaaattaaatgacgctttatcttactcaaacactaccgtcgcaatggacgactggtttgaagaaaacgaagtagacaacacggaaatatttgctaaggcatggcttcacggctatgaagtagaaaaagaaaaactttacacagttgaaattccagaccctaatgcaagtggttacggtaagacatttcttggcagagatgatgatggaaaagtagtgctatctacttggactggttttagttccattgaatttgctgatgattggaaacaatcagaacgtgcacagttgacagaagatgaaattaaaaaaggttttacttgggcttggaatgaagggtttgccgaagaggtgaaagaatga

SEQ ID NO: 384 - protein, 181 aa, Bacteriophage D4446
MNKQEAIELVKNTSYSVPIDSPVKHLTEDTVINIIKQLDEPEKATVPDFVAKYIEESREFDRKLNDALSYSNTTVAMDDWFEENEVDNTEIFAKAWLHGYEVEKEKLYTVEIPDPNASGYGKTFLGRDDDGKVVLSTWTGFSSIEFADDWKQSERAQLTEDEIKKGFTWAWNEGFAEEVKE

SEQ ID NO: 385 - DNA, 162 bp, Bacteriophage D4446
atgaaacgctttgtagtaacaggttacaaagatggttggtttgtcttctcatttcctttaaacgccataaactcttattatgctatccaatatgcaagcgaagatgaattggtagaaggtatggagttcgataagctggttataaaagaggtgaaagaatga

SEQ ID NO: 386 - protein, 53 aa, Bacteriophage D4446
MKRFVVTGYKDGWFVFSFPLNAINSYYAIQYASEDELVEGMEFDKLVIKEVKE

SEQ ID NO: 387 - DNA, 147 bp, Bacteriophage D4446
atgaacataaaagaggtgttctgtattgattgctatgaatggaaaaagaaagaagacttaacagggagcaaattttccaatgatattttatattgcaaagaatgtggttacgccttagttcgtacgtgtgaccgtaataacaaatga

SEQ ID NO: 388 - protein, 48 aa, Bacteriophage D4446
MNIKEVFCIDCYEWKKKEDLTGSKFSNDILYCKECGYALVRTCDRNNK

SEQ ID NO: 389 - DNA, 165 bp, Bacteriophage D547
atgacaaacattgttgctgaccttgtagatagtggcatgtctgacgcttggattttgaaaaacattgggatggatgctgacgaattgctgcgactaaagcaacttagcggactggcttccttgttcaaagataaggaattcactacagcttgggaagtaggataa

SEQ ID NO: 390 - protein, 54 aa, Bacteriophage D547
MTNIVADLVDSGMSDAWILKNIGMDADELLRLKQLSGLASLFKDKEFTTAWEVG

SEQ ID NO: 391 - DNA, 273 bp, Bacteriophage D5691
atggaaacttataaagaatacaaacaacaacagaaagaagaacgtgaaagagtaagagcgcttcgtagtgaagtattttcaggcaacgctgaaaagcttgcgacagatattgtaaggatttcgagcggagatgtttataaaattatcccacgttttgggactagatatgaaaaaagtccaatcatcaaattagacccagaagaagtagaacgccacatcaaagaagctcgtgaagtcagagaacttgcgaaaattatggcaagcaaagaatag

SEQ ID NO: 392 - protein, 90 aa, Bacteriophage D5691
METYKEYKQQQKEERERVRALRSEVFSGNAEKLATDIVRISSGDVYKIIPRFGTRYEKSPIIKLDPEEVERHIKEAREVRELAKIMASKE

SEQ ID NO: 393 - DNA, 243 bp, Bacteriophage D5700
atggcagtagtggtcgaagcctcagcattatgctggggctttttttgttataatatacctatatcaatggcctcccacgcatacgcgcagatacgttctgatgggaggttttttttgttgccgttaaaacggacaaaaaaatttaaaaagtttgattttattgttgataatacacgcataagcgtgtataatgtaattaaagataaggaaagcgaggaaaacaaaaatggtagtaaaaattaa

SEQ ID NO: 394 - protein, 80 aa, Bacteriophage D5700
MAVVVEASALCWGFFCYNIPISMASHAYAQIRSDGRFFLLPLKRTKKFKKFDFIVDNTRISVYNVIKDKESEENKNGSKN

SEQ ID NO: 395 - DNA, 471 bp, Bacteriophage D5839
ttgctggggctttttttgtgttataatagaataaaaaaacaaatagatgaggtaagaaaaacggctattgacctgtatcgtgaactggatatccaatcgttggagcaaagattggaaaagaacgaagaaaacactcaacgcttcctccaacaaacagccaaaagcttaaaccaagacaagactgaactatctctccgaactgaccagttagggcgtagtgttgaaaagattgaaaacaaactagacgacatgtacgctaagaacgaactagacttgaaattccagatgatggatcaaaagattgacgctaaatttgatacctttggtcaacgcatggaaaacatgttcttagcacaaaccaataggcaacttgaggaacaagccaagaatagaaaagaattcacatattggtttatttgcattcttgtagctatcgctgttattgctattcctgtttggttcggcaaataa

SEQ ID NO: 396 - protein, 156 aa, Bacteriophage D5839
MLGLFLCYNRIKKQIDEVRKTAIDLYRELDIQSLEQRLEKNEENTQRFLQQTAKSLNQDKTELSLRTDQLGRSVEKIENKLDDMYAKNELDLKFQMMDQKIDAKFDTFGQRMENMFLAQTNRQLEEQAKNRKEFTYWFICILVAIAVIAIPVWFGK

SEQ ID NO: 397 - DNA, 204 bp, Bacteriophage D5839
atgtcattttttacgtcaacaaaaacggcaacgtcaacttttttcatagcaagtaatagaatacttgcatcatttcgattaaattctcgaactgtacacccgtcttttttaggtgggttttttgttttgcaaaaaaatctaaatttatttatcaaaagcattgacaaactatcatgtatgatatataatatacttataagataa

SEQ ID NO: 398 - protein, 67 aa, Bacteriophage D5839
MSFFTSTKTATSTFFIASNRILASFRLNSRTVHPSFLGGFFVLQKNLNLFIKSIDKLSCMIYNILIR

SEQ ID NO: 399 - DNA, 129 bp, Bacteriophage D6252
atgttactaatagtgacattcagttatatcataaattatttgttgttcgatttgggaagtagcttaattaaaaaaggagaaagaaaatgctactataaaggatttaagacaaagaaggatgtaatctaa

SEQ ID NO: 400 - protein, 42 aa, Bacteriophage D6252
MLLIVTFSYIINYLLFDLGSSLIKKGERKCYYKGFKTKKDVI

SEQ ID NO: 401 - DNA, 159 bp, Bacteriophage D6252
ttggagtgcttatattttaggaaaaaagagggcgcttgctctcttttttttatgtattcaataaaaagtatactttataaattttagagttattttgttaaaaactcaaaaaaacttgaaaaaaaatcaagaaaactgttgacattgaattttgtttaa

SEQ ID NO: 402 - protein, 28 aa, Bacteriophage D6252
MECLYFRKKEGACSLFFMYSIKSILYKF

SEQ ID NO: 403 - DNA, 690 bp, Bacteriophage D7130
ttggatatttacgtttatactgatgaatcaggagtatttgataaagaacatgaaacaatatatgtttatggtggagtgatttttttaacttctgaggacaaagagaattcaggtagaagatatatatatgcggaaaaagcactaagaaaaagccatagtaattataggaaaggggaactgaaagcaagtaggcttaaaaatagacataaagccagtttgtttaggtcgcttaatagggaaataaaattttctatagtggtgagtattggcagggtgcatgataggattttttgtgagaaaaaaagtaagcagcgttacttagattatgtttacaaagttggtttgaaaaaggtgttacaacgtcttgtagcagattgtaaaatagagactaccgaagtagatacgatcagtatttttacagatgagcatagtactgcgactaatggaaaatatgagttaagagaggcgctgttaaacgagtttaaatatggcacgtttaacccagactggaatattttttatcctcccttattcgaaaaactatctagtttaactgttgaatactgtaattcagctaaaaagccacatatacgtatggcagatataatagcgaatagagcatattatcttgcaaagaatgatctttttggagagttgggagagaaaactatatcaatccacttcccttag

SEQ ID NO: 404 - protein, 229 aa, Bacteriophage D7130
MDIYVYTDESGVFDKEHETIYVYGGVIFLTSEDKENSGRRYIYAEKALRKSHSNYRKGELKASRLKNRHKASLFRSLNREIKFSIVVSIGRVHDRIFCEKKSKQRYLDYVYKVGLKKVLQRLVADCKIETTEVDTISIFTDEHSTATNGKYELREALLNEFKYGTFNPDWNIFYPPLFEKLSSLTVEYCNSAKKPHIRMADIIANRAYYLAKNDLFGELGEKTISIHFP

SEQ ID NO: 405 - DNA, 135 bp, Bacteriophage D7130
ttggagagttgggagagaaaactatatcaatccacttcccttagttttagaaagaggcgaggctgtaagcctctttttattataatggtcaagtatgtgggattttgcttaattctgttcatgacattagggtag

SEQ ID NO: 406 - protein, 44 aa, Bacteriophage D7130
MESWERKLYQSTSLSFRKRRGCKPLFIIMVKYVGFCLILFMTLG

SEQ ID NO: 407 - DNA, 150 bp, Bacteriophage M5728
gtgcacaaaaagggaattcatataaaaaaagtcggctattttagtcgactcttttttttatgtcatgtaaacagcagtatagcgttttctattatgttatcgatgtcgtgtcgtttctctaactttttcaaatgttggaaacttttctga

SEQ ID NO: 408 - protein, 49 aa, Bacteriophage M5728
MHKKGIHIKKVGYFSRLFFLCHVNSSIAFSIMLSMSCRFSNFFKCWKLF

SEQ ID NO: 409 - DNA, 141 bp, Bacteriophage M5782
ttgttgggggggctaagacgccccctttttgatatatcaacggcctcccacccgtcttttttaggtgggttttttgttttgcaaaaaatttttttatcaaaagtacggatacatacaaagaatacgcttttaacgttttaa

SEQ ID NO: 410 - protein, 46 aa, Bacteriophage M5782
MLGGLRRPLFDISTASHPSFLGGFFVLQKIFLSKVRIHTKNTLLTF

SEQ ID NO: 411 - DNA, 438 bp, Bacteriophage P3681
atgaacgaaatagcattatcggacaatcttgcacagattgaacttgaaatcaatcatcataagcagattgcaggtcagtctatttgggaaatcggcaggcgtttaaatcatgttaaagagcacgatttagcgcatgggcaatttatggaatgggttgaaaaacttggtataaatcaaccagaagccaatcgtatgatgagagttgctaaagaactaccaaattcttcaacgttgagtaatttaggaagcacggctctctacttaatcgccactcttccagatgatgaaaagcaagaacaaattgaaaagattgagcaaggtgaatcaccaacggtcagagaattgcaagagataaagcgtcgtctcaaactcaaagaccaagcactggaagcggtcaagggtgagttggaacgtgctatacttggtattaaagtttaa

SEQ ID NO: 412 - protein, 145 aa, Bacteriophage P3681
MNEIALSDNLAQIELEINHHKQIAGQSIWEIGRRLNHVKEHDLAHGQFMEWVEKLGINQPEANRMMRVAKELPNSSTLSNLGSTALYLIATLPDDEKQEQIEKIEQGESPTVRELQEIKRRLKLKDQALEAVKGELERAILGIKV

SEQ ID NO: 413 - DNA, 438 bp, Bacteriophage P3684
atgaacgaaatagcattatcggacaatcttgcacagattgaacttgaaatcaatcatcataagcagattgcaggtcagtctatttgggaaatcggcaggcgtttaaatcatgttaaagagcacgatttagcgcatgggcaatttatggaatgggttgaaaaacttggtataaatcaaccagaagccaatcgtatgatgagagttgctaaagaactaccaaattcttcaacgttgagtaatttaggaagcacggctctctacttaatcgccactcttccagatgatgaaaagcaagaacaaattgaaaagattgagcaaggtgaatcaccaacggtcagagaattgcaagagataaagcgtcgtctcaaactcaaagaccaagaactggaagcggtcaagggtgagttggaacgtgctatacttggtattaaagtttaa

SEQ ID NO: 414 - protein, 145 aa, Bacteriophage P3684
MNEIALSDNLAQIELEINHHKQIAGQSIWEIGRRLNHVKEHDLAHGQFMEWVEKLGINQPEANRMMRVAKELPNSSTLSNLGSTALYLIATLPDDEKQEQIEKIEQGESPTVRELQEIKRRLKLKDQELEAVKGELERAILGIKV

SEQ ID NO: 415 - DNA, 336 bp, Bacteriophage P4761
atggaagaattagaacaagcgtttgaaaatcttgatgattggtatctatcaagcatgaaagacagtgcttacaaggattttgggaaatacgaaattcgcttatcaaatcattcggcagacaataaatatcatgacctagaaaatggtcgcttaatcgttaatgttaaagctagtaaattgaacttcgttgatatcatcgagaataaaatctataaaatcattgagaaaattgaaactctcgatttagacaagtacagatttattaacgctactaaaatggaaaacgatatcaaatgttattacaagggatttaagacaaagaaggatgtgatctaa

SEQ ID NO: 416 - protein, 111 aa, Bacteriophage P4761
MEELEQAFENLDDWYLSSMKDSAYKDFGKYEIRLSNHSADNKYHDLENGRLIVNVKASKLNFVDIIENKIYKIIEKIETLDLDKYRFINATKMENDIKCYYKGFKTKKDVI

SEQ ID NO: 417 - DNA, 177 bp, Bacteriophage P5641
atgacagatgcgcacaaaaaagctgttaagaagtggaataaaaacaacagagaacatagaaattatctaaacaagcgttcatcagctcgtggtttcatcagaaataatgcgactgctgaagatttgagagagctagaggagcttattgcagaaagaagaaaaaagaattttaggtaa

SEQ ID NO: 418 - protein, 58 aa, Bacteriophage P5641
MTDAHKKAVKKWNKNNREHRNYLNKRSSARGFIRNNATAEDLRELEELIAERRKKNFR

SEQ ID NO: 419 - DNA, 294 bp, Bacteriophage P7573
ttgttaaacctaaagcgcgagcgaaatcatcagctttattcagcgggaacacccgactacctgaaagatatcttgtttgaaatcccagctttatttgcattgacatggaactgttgtctaaatagctttttattatcgttgtttctcatatttaatagtataaacattatacaaaagttcccaaaaaataaacaatatgttcccaaaaataaacttttttcatatttttttgattttagtgttgacaaatgggaacgtgttagatatactataattgttctaaggaacaagtaa

SEQ ID NO: 420 - protein, 97 aa, Bacteriophage P7573
MLNLKRERNHQLYSAGTPDYLKDILFEIPALFALTWNCCLNSFLLSLFLIFNSINIIQKFPKNKQYVPKNKLFSYFFDFSVDKWERVRYTIIVLRNK

SEQ ID NO: 421 - DNA, 105 bp, Bacteriophage P7601
ttgcaaaaaaaatatataattttttataaaaacagtttccgtctggtcgcaaaaatcgacttgaatggattgaaaacaatcttgaaaacattcgataaaaaataa

SEQ ID NO: 422 - protein, 34 aa, Bacteriophage P7601
MQKKYIIFYKNSFRLVAKIDLNGLKTILKTFDKK

SEQ ID NO: 423 - DNA, 105 bp, Bacteriophage P7602
ttgcgcacacacaagcataagggaaaattttgttggggggggctaagacgccccctttttgatataatatacctatatcaacggcctcccacccgtcttttttag

SEQ ID NO: 424 - protein, 34 aa, Bacteriophage P7602
MRTHKHKGKFCWGGLRRPLFDIIYLYQRPPTRLF

SEQ ID NO: 425 - DNA, 132 bp, Bacteriophage P9853
atgctggggcttttttttaatataaatgctactatattaatggatacagttaaaagagaagcatccagatatgatggattttatggacctgatagattggtatttagaaaatcgcaaaccataagatattga

SEQ ID NO: 426 - protein, 43 aa, Bacteriophage P9853
MLGLFFNINATILMDTVKREASRYDGFYGPDRLVFRKSQTIRY

SEQ ID NO: 427 - DNA, 222 bp, Bacteriophage TP-778L
atgtacgctaagaacgaactagatttgaaattccagatgatggatcaaaagattgacgctaaatttgatacctttggtcaacgcatggaaaacatgttcttagcacaaaccaataggcaacttgaggaacaagccaagaatagaaaagaattcacatattggtttatttgcattcttgtagctatcgctgttattgctattcctgtttggttcggcaaataa

SEQ ID NO: 428 - protein, 73 aa, Bacteriophage TP-778L
MYAKNELDLKFQMMDQKIDAKFDTFGQRMENMFLAQTNRQLEEQAKNRKEFTYWFICILVAIAVIAIPVWFGK

SEQ ID NO: 429 - DNA, 222 bp, Bacteriophage TP-J34
atgtacgctaagaacgaactagacttgaaattccagatgatggatcaaaagattgacgctaaatttgatacctttggtcaacgcatggaaaacatgttcttagcacaaaccaataggcaacttgaggaacaagccaagaatagaaaagaattcacatattggtttatttgcattcttgtagctatcgctgttattgctattcctgtttggttcggcaaataa

SEQ ID NO: 430 - protein, 73 aa, Bacteriophage TP-J34; identical to SEQ ID NO: 428

SEQ ID NO: 431 - DNA, 183 bp, Bacteriophage D3820
atggatacatataaagaacaattttattatttggatcctatttatattagtgtggatattaataggaggacttttattttaggaaaaagagggcaatcgctctctttttttattgtaataaaacaatttaaaaatataactaaaaaaacttcaaaaaaatcgaaaaaaaatattgacaaataa

SEQ ID NO: 432 - protein, 60 aa, Bacteriophage D3820
MDTYKEQFYYLDPIYISVDINRRTFILGKRGQSLSFFIVIKQFKNITKKTSKKSKKNIDK

SEQ ID NO: 433 - DNA, 177 bp, Bacteriophage P7574
atgctggggctttttttgtgttataatatgaatgagatgtcaatccccccacatccttttatggacagatacgttctgagtgggggtttttttgttttgctattttttaacctaacagcccgtaattcccccacctctaaggtggcgggatgtaagggcttcggtctagtgcagtga

SEQ ID NO: 434 - protein, 58 aa, Bacteriophage P7574
MLGLFLCYNMNEMSIPPHPFMDRYVLSGGFFVLLFFNLTARNSPTSKVAGCKGFGLVQ

SEQ ID NO: 435 - DNA, 195 bp, Bacteriophage D1422
atgttcagcgaccttgtgcgttcgaaagtgtataagggaacattttgttgtgggctaagaccccctttttttgatataatatatctatatcaatgtcctcccacgcataagcgcagatacgttctgagggaggttttttatttgttttattttgataaaaatgctactatattaacggatacagttaaaagctga

SEQ ID NO: 436 - protein, 64 aa, Bacteriophage D1422
MFSDLVRSKVYKGTFCCGLRPPFFDIIYLYQCPPTHKRRYVLREVFYLFYFDKNATILTDTVKS

SEQ ID NO: 437 - DNA, 195 bp, Bacteriophage D5861
atgttcagcgaccttgtgcgttcgcaagtgtataagggaacattttgttgtgggctaagaccccctttttttgatataatatatctatatcaatgtcctcccacgcataagcgcagatacgttctgagggaggttttttatttgttttattttgatataaatgctactataataatggatacagttaaaagctga

SEQ ID NO: 438 - protein, 64 aa, Bacteriophage D5861
MFSDLVRSQVYKGTFCCGLRPPFFDIIYLYQCPPTHKRRYVLREVFYLFYFDINATIIMDTVKS

SEQ ID NO: 439 - DNA, 264 bp, Bacteriophage P3681
atgaatagcatgaaaaagccccacactgcggaaaacggcgatttaattcatacaacagaagacaacgaggcttcagatatatcaatcattacaatttcgtttgttcgcaaaacgaacaagcaaatattgaaaaattcgaaagtttgcctaaaacgttacaagctcaagtatctaaaccatctgccaatccagaggttaatcaagcagtattcgacggagatatcaaagcaaaaagaaattatagctcttgaaaaaaatgagtga

SEQ ID NO: 440 - protein, 87 aa, Bacteriophage P3681
MNSMKKPHTAENGDLIHTTEDNEASDISIITISFVRKTNKQILKNSKVCLKRYKLKYLNHLPIQRLIKQYSTEISKQKEIIALEKNE

SEQ ID NO: 441 - DNA, 243 bp, Bacteriophage P3684
atgaatagcatgaaaaagccccacactgcggaaaacggcgatttaattcatacaacagaagacaacgaggcttcagatatatcaatcattacaatttcgtttgttcgcaaaacgaacaagcaaatattgaaaaattcgaaagtttgcctaaaacgttacaagctcaagtatctaaaccatctgccaatccagaggttaatcaagcagtattcgacggagatatcaaagcaaaaagaatattga

SEQ ID NO: 442 - protein, 80 aa, Bacteriophage P3684
MNSMKKPHTAENGDLIHTTEDNEASDISIITISFVRKTNKQILKNSKVCLKRYKLKYLNHLPIQRLIKQYSTEISKQKEY

SEQ ID NO: 443 - DNA, 81 bp, Bacteriophage D2767
atgttcagcgaccttgtgcgttcgaaagtgtataagggaacattttgttgtgggctaagaccccccttttttttgatataa

SEQ ID NO: 444 - protein, 26 aa, Bacteriophage D2767
MFSDLVRSKVYKGTFCCGLRPPFFLI

SEQ ID NO: 445 - DNA, 153 bp, Bacteriophage D6660
atggcagtagtggtcgaagcctcagcatttttgctggggctttttttgtgttataatatgaaacatcattttatggacagatatttgctttgttttgataaaaatgctactatattaatggtcttcgataaactctctctcgccctgacttga

SEQ ID NO: 446 - protein, 50 aa, Bacteriophage D6660
MAVVVEASAFLLGLFLCYNMKHHFMDRYLLCFDKNATILMVFDKLSLALT

SEQ ID NO: 447 - DNA, 276 bp, Bacteriophage D802
atgataactaaagaacaattaaaaggatactacagcgaacacttggaagagctcgtcgaatgggcagacgatataaataaaatcgcttatgagatagatgggaaaagtcatcaaactaagataggttgggtgaatgatagattaaaagaccattttatgaaagaaaaaggggttttagttattcattacaccaatgagcaagtcgaaacagcctacaatgagtgggtaaaaattacagaggaggcgtttaatggattctttaataacacaatctaa

SEQ ID NO: 448 - protein, 91 aa, Bacteriophage D802
MITKEQLKGYYSEHLEELVEWADDINKIAYEIDGKSHQTKIGWVNDRLKDHFMKEKGVLVIHYTNEQVETAYNEWVKITEEAFNGFFNNTI

SEQ ID NO: 449 - DNA, 138 bp, Bacteriophage P9871
atggcagcagtggtcgaagcctcagcatttttgctggggctttttttgtgttataatatgaatgagatgtcaatccccccacatccttttatggacagatacgttctgatgggaagttttttatttgctttgttttga

SEQ ID NO: 450 - protein, 45 aa, Bacteriophage P9871
MAAVVEASAFLLGLFLCYNMNEMSIPPHPFMDRYVLMGSFLFALF

SEQ ID NO: 451 - DNA, 147 bp, Bacteriophage D4254
atggcagtagtggtcgaagcctcagcattatgctggggctttttttgtgttataatatacctatatcaatggcctcccacgcatacgcgcagatacgttctgatgggaggtttttttgttgccgttaaaacggacaaaaaaatttaa

SEQ ID NO: 452 - protein, 48 aa, Bacteriophage D4254
MAVVVEASALCWGFFCVIIYLYQWPPTHTRRYVLMGGFFVAVKTDKKI

SEQ ID NO: 453 - DNA, 120 bp, Bacteriophage D4753
gtggtcgaagcctcagcattatgctggggctttttttgtgttataatacatatatcaatggcttcccacgcatacgcgcagatacgttctgagggaagttttttatttgcttttttttga

SEQ ID NO: 454 - protein, 39 aa, Bacteriophage D4753
MVEASALCWGFFCVIIHISMASHAYAQIRSEGSFLFAFF

SEQ ID NO: 455 - DNA, 126 bp, Bacteriophage D5944
atggcagtagtggtcgaagcctcagcattttgctggggctttttttgtgttataatatacatggaacgacaaaccccctgcatccacatggacagatacgctctgacgcagggcttttttatttga

SEQ ID NO: 456 - protein, 41 aa, Bacteriophage D5944
MAVVVEASAFCWGFFCVIIYMERQTPCIHMDRYALTQGFFI

SEQ ID NO: 457 - DNA, 132 bp, Bacteriophage P0095
atggcagcagtggtcgaagcctcagcatttttgctggggctttttttgtgttataatatacctatatcaatggcttcccacgcatacgcgcagatacgttctgagggaggttttttgtttgctttattttga

SEQ ID NO: 458 - protein, 43 aa, Bacteriophage P0095
MAAVVEASAFLLGLFLCYNIPISMASHAYAQIRSEGGFLFALF

SEQ ID NO: 459 - DNA, 519 bp, Bacteriophage D6961
atggaaaattactctagtccagtgtataatattaaaaaaatcccgattgaaaaaattcaagcgaatagctataaccccaaccatgtagcgacaccagaaatgaagttgttatatgaatccatcaaagcagacggatacacaatgcctatcgtttgttattatcttaaagatgaagacaaatacgagattgtagatggctttcaccgttatacaactatgcttaatcataaagatatttacgaacgagagaatggctgtttacctgtatctgttattgataaaccattagaggagcgcatggcttctacagtacgacacaatcgagcaagaggtagtcatgatattggcttaatggctaatattgtaactgaattggttgatagcggaatgtctgatgccaaagttatgaaaagtcttggaatggacgcagacgagttattaagattaaaacaggttagcggtttagcaagtttgtttgcaaacaaggagttcagtaaatcgtgggatataaaaaaatag

SEQ ID NO: 460 - protein, 172 aa, Bacteriophage D6961
MENYSSPVYNIKKIPIEKIQANSYNPNHVATPEMKLLYESIKADGYTMPIVCYYLKDEDKYEIVDGFHRYTTMLNHKDIYERENGCLPVSVIDKPLEERMASTVRHNRARGSHDIGLMANIVTELVDSGMSDAKVMKSLGMDADELLRLKQVSGLASLFANKEFSKSWDIKK

SEQ ID NO: 461 - DNA, 516 bp, Bacteriophage D4250
atgcaaacatactctagccctgtatataatattaagcgcgtgcctattgagaaaattcaagcaaacagctacaatcctaaccatgtagcaagcccagaaatgaagttgctttaccaatccatcaaagaagatggttacacaatgccaatcgtatgttattaccttgaggatgaagataagtatgaaattgtggacggtttccatcggtatacaacgatgaaagaacacaaggatatctatgaaagagaggaggggtgtctaccagtttctgttatagataaaccaatcagtgaccgaatggcatcaactatcagacacaatagagcaagagggtcgcacgacatcggtctgatgactaatatcatttctgacctagttgattctgggatgtcagatgcgtggattatgaaaaatattggtatggatgctgatgaattactacgactaaaacaagttagcggactggcttccttgttcaaagataaggaattcacgacagcttgggaagaaggataa

SEQ ID NO: 462 - protein, 171 aa, Bacteriophage D4250
MQTYSSPVYNIKRVPIEKIQANSYNPNHVASPEMKLLYQSIKEDGYTMPIVCYYLEDEDKYEIVDGFHRYTTMKEHKDIYEREEGCLPVSVIDKPISDRMASTIRHNRARGSHDIGLMTNIISDLVDSGMSDAWIMKNIGMDADELLRLKQVSGLASLFKDKEFTTAWEEG

SEQ ID NO: 463 - DNA, 516 bp, Bacteriophage D4252
atgcaaacatactctagccctgtatataatattaagcgcgtgcctattgataaaattcaagcaaacagctacaatcctaaccatgtagcaagcccagaaatgaagttgctttatcaatccatcaaagaagatggttacacaatgccaatcgtatgttattaccttgaggatgaagataagtatgaaattgtggacggttttcatcggtatacaacgatgaaagaacacaaggatatctatgaaagagaggaggggtgtctaccagtgtctgtcatagataaaccaatcagtgaccgaatggcatcaactatcagacacaatagagcaagaggttcgcacgacatcggtctgatgactaatatcatttctgacctagttgattctgggatgtcagatgcgtggattatgaaaaatattggtatggatgctgatgaattactacgactaaaacaagttagcggactggcttccttgttcaaagataaggaattcacgacagcttgggaagaaggataa

SEQ ID NO: 464 - protein, 171 aa, Bacteriophage D4252
MQTYSSPVYNIKRVPIDKIQANSYNPNHVASPEMKLLYQSIKEDGYTMPIVCYYLEDEDKYEIVDGFHRYTTMKEHKDIYEREEGCLPVSVIDKPISDRMASTIRHNRARGSHDIGLMTNIISDLVDSGMSDAWIMKNIGMDADELLRLKQVSGLASLFKDKEFTTAWEEG

SEQ ID NO: 465 - DNA, 513 bp, Bacteriophage D4276
atgcaaacatactatagccctgtatataatattaagcgcgtgcctattgagaaaattcaagcaaacagctacaatcctaaccatgtagcaagcccagaaatgaagttgctttatcaatccatcaaagaagatggttacacaatgccaatcgtatgttattaccttgaggatgaagataagtatgaaattgtggacggtttccatcggtatacaacgatgaaagaacacaaggatatctatgaaagagaggaggggtgtctaccagtttctgtcatagataaaccaatcagtgaccgaatggcatcgactatcagacacaatagagcaagagggtcgcacgacatcggtctgatgactaatatcatttctgacctagttgattctgggatgtcagatgcgtggattatgaaaaatattggtatggatgctgatgaattactacgactaaaacaagttagcggactggcttccttgttcaaagataaggaattcacgacagcttgggaagaatga

SEQ ID NO: 466 - protein, 170 aa, Bacteriophage D4276
MQTYYSPVYNIKRVPIEKIQANSYNPNHVASPEMKLLYQSIKEDGYTMPIVCYYLEDEDKYEIVDGFHRYTTMKEHKDIYEREEGCLPVSVIDKPISDRMASTIRHNRARGSHDIGLMTNIISDLVDSGMSDAWIMKNIGMDADELLRLKQVSGLASLFKDKEFTTAWEE

SEQ ID NO: 467 - DNA, 225 bp, Bacteriophage D5691
atggcacaaattaaagatggttggcataaagtttataacgaaaatgtttatgttgaaaacgaaaaagtagtacgaggaacaaaaaaagattataacggttctgaggtcacttgttatccttacgaatacgataaaaaccaagattgttggattaatatttctgggaaagcaactctttcttcttatagagcaggactcaaaaaaggcactaagtgtatgaagtaa

SEQ ID NO: 468 - protein, 74 aa, Bacteriophage D5691
MAQIKDGWHKVYNENVYVENEKVVRGTKKDYNGSEVTCYPYEYDKNQDCWINISGKATLSSYRAGLKKGTKCMK

SEQ ID NO: 469 - DNA, 138 bp, Bacteriophage D1024
atgttcagcgaccttgtgcgttcgaaagtgtataagggaacattttgttgtgggctaagaccccctttttttgatataatatatctatatcaatgtcctcccacgcataagcgcagatacgtgctgagtcttcgataa

SEQ ID NO: 470 - protein, 45 aa, Bacteriophage D1024
MFSDLVRSKVYKGTFCCGLRPPFFDIIYLYQCPPTHKRRYVLSLR

SEQ ID NO: 471 - DNA, 123 bp, Bacteriophage D1018
atgctggggctttttttgtgttataatatgaatgagatgtcaatccccccacatccttttatggacagatacgttctgagtgggggtttttttgttttgctattttttaaaaatgtggtataa

SEQ ID NO: 472 - protein, 40 aa, Bacteriophage D1018
MLGLFLCYNMNEMSIPPHPFMDRYVLSGGFFVLLFFKNVV

SEQ ID NO: 473 - DNA, 141 bp, Bacteriophage D5738
atgctggggctttttttgtgttataatatgaatgagatgtcaatccccccacatccttttatggacagatacgttctgagtgggggttttttgttttgctattttttaaaaatgtggtataatataaatatccattcataa

SEQ ID NO: 474 - protein, 46 aa, Bacteriophage D5738
MLGLFLCYNMNEMSIPPHPFMDRYVLSGGFLFCYFLKMWYNINIHS

SEQ ID NO: 475 - DNA, 258 bp, Bacteriophage D4276
atgaagaaattttggcatagcggtatgattgacaagaaggttattgaaaaacgtaaacaagatgattatatgaataaattacacaggactattcttgagttgagtataaaaccacctgaacccgaaccttggtacagacatccagaaatgagagcattgttggataggattgattctatggacatgatagattggtattcaaaatatctaaaacatcgcaaaccatacgataattatagtggagaattagagaaatga

SEQ ID NO: 476 - protein, 85 aa, Bacteriophage D4276
MKKFWHSGMIDKKVIEKRKQDDYMNKLHRTILELSIKPPEPEPWYRHPEMRALLDRIDSMDMIDWYSKYLKHRKPYDNYSGELEK

SEQ ID NO: 477 - DNA, 180 bp, Bacteriophage 5093
atgaagaaattttggcgtagtggaatgattgacaagaaggttatcgaaaaacgacaacaagaagagtatattaataagttacataggactattcttgagttgagtataaaaccacctgaaccagaaccttggtacagacatccagaaatgagagcattgttggatagaattgatgattag

SEQ ID NO: 478 - protein, 59 aa, Bacteriophage 5093
MKKFWRSGMIDKKVIEKRQQEEYINKLHRTILELSIKPPEPEPWYRHPEMRALLDRIDD

SEQ ID NO: 479 - DNA, 198 bp, Bacteriophage D4154
atgaagaagttttggcgtagtggaatgattgacaagaaagttattgaaaaacgacaacaagatgattatatgaataagttacataggactattcttgagttgagtataaaaccacctgaacccgaaccttggtacagacatccagaaatgagagcatttttggataggatttatgattcgagaagcaatttaaagtaa

SEQ ID NO: 480 - protein, 65 aa, Bacteriophage D4154
MKKFWRSGMIDKKVIEKRQQDDYMNKLHRTILELSIKPPEPEPWYRHPEMRAFLDRIYDSRSNLK

SEQ ID NO: 481 - DNA, 180 bp, Bacteriophage D4160
atgaagaaattttggcgtagtggaatgattgacaagaaaattattgcgaaacgtgaacaggatgagtatttgaataaattacacaggactattcttgagttgagtagaaaaccacctgaacaagaaccttggtacagacatccagaaatgagagcattgttggatagaattgatgattag

SEQ ID NO: 482 - protein, 59 aa, Bacteriophage D4160
MKKFWRSGMIDKKIIAKREQDEYLNKLHRTILELSRKPPEQEPWYRHPEMRALLDRIDD

SEQ ID NO: 483 - DNA, 180 bp, Bacteriophage D5925
atgaaaaaattttggcatagcggtatgattgacaagaaagttattgaaaaacgtaaacaagatgattatatgaataagttacataggactattcttgagttgagtataaaaccacctgaaccagaaccttggtacagacatccagaaatgagagcattgttggataggattgatgattag

SEQ ID NO: 484 - protein, 59 aa, Bacteriophage D5925
MKKFWHSGMIDKKVIEKRKQDDYMNKLHRTILELSIKPPEPEPWYRHPEMRALLDRIDD

SEQ ID NO: 485 - DNA, 198 bp, Bacteriophage D6193
atgaagaagttttggcgtagtggaatgattgacaagaaagttattgaaaaacgacaacaagatgattatatgaataagttacataggactattcttgagttgagtataaaaccacctgaacccgaaccttggtacagacatccagaaatgagagcattgttggataggatttatgattcgagaagcaatttaaagtaa

SEQ ID NO: 486 - protein, 65 aa, Bacteriophage D6193
MKKFWRSGMIDKKVIEKRQQDDYMNKLHRTILELSIKPPEPEPWYRHPEMRALLDRIYDSRSNLK

SEQ ID NO: 487 - DNA, 180 bp, Bacteriophage TP-J34
atgaagaaattttggcgtagtggaatgattgacaagaaggttattgaaaaacgtaaacaagatgattatatgaataaattacacaggactattcttgagttgagtataaaaccacctgaaccagaaccttggtacagacatccagaaatgagagcattgttggatagaattgatgattag

SEQ ID NO: 488 - protein, 59 aa, Bacteriophage TP-J34
MKKFWRSGMIDKKVIEKRKQDDYMNKLHRTILELSIKPPEPEPWYRHPEMRALLDRIDD

SEQ ID NO: 489 - DNA, 180 bp, Bacteriophage Proph1
atgaagaaattttggcgtagtggcatgattgacaagaaggttattgaaaaacgtaaacaagatgattatatgaataaattacacaggactattcttgagttgagtataaaaccacctgaacccgaaccttggtacagacatccagaaatgagagcattgttggataggattgatgattag

SEQ ID NO: 490 - protein, 59 aa, Bacteriophage Proph1; identical to SEQ ID NO: 488

SEQ ID NO: 491 - DNA, 177 bp, Bacteriophage D1126
atgaagaaattttggcgtagtggcatgattgacaagaaggttattaaaaaacgtaaacaggaagagtatatgaataagatgcataggactattcttgaattaaaaaatgagaagcatccagatatgatggattttatggacctgatagattggtatttagaaaatcgcaaaccataa

SEQ ID NO: 492 - protein, 58 aa, Bacteriophage D1126
MKKFWRSGMIDKKVIKKRKQEEYMNKMHRTILELKNEKHPDMMDFMDLIDWYLENRKP

SEQ ID NO: 493 - DNA, 189 bp, Bacteriophage D3607
atgaagaaattttggcatagcggtatgatcgacaagaaagttattgaaaaacgtaaacaggatgagtatttgaataaattacacaggactattcttgagttaaaaaatgagaagcatccagatatgatggattttatggacctgatagattggtatttagagaatcgcaaaccacgagatattgattag

SEQ ID NO: 494 - protein, 62 aa, Bacteriophage D3607
MKKFWHSGMIDKKVIEKRKQDEYLNKLHRTILELKNEKHPDMMDFMDLIDWYLENRKPRDID

SEQ ID NO: 495 - DNA, 189 bp, Bacteriophage D4252
atgaagaaattttggcatagcggtatgattgacaagaaggttattgaaaaacgtaaacaggaagaatgtattaatgaactgcataggactattcttgagttgaaaaatgagaagcatccagatatgatggattttatggacctgatagattggtatttagaaaatcgcaaaccacgagatatttattag

SEQ ID NO: 496 - protein, 62 aa, Bacteriophage D4252
MKKFWHSGMIDKKVIEKRKQEECINELHRTILELKNEKHPDMMDFMDLIDWYLENRKPRDIY

SEQ ID NO: 497 - DNA, 183 bp, Bacteriophage D4487
atgatcgacaagaaagttattgaaaaacgtaaacaggatgagtatttgaataaattacacaggactattcttgagttaaaaaatgagaagcatccagatatgatagattttatggacctgatagattttatggacctgatagattggtatttagagaatcgcaaaccacgagatattgattag

SEQ ID NO: 498 - protein, 60 aa, Bacteriophage D4487
MIDKKVIEKRKQDEYLNKLHRTILELKNEKHPDMIDFMDLIDFMDLIDWYLENRKPRDID

SEQ ID NO: 499 - DNA, 189 bp, Bacteriophage D6938
atgaataaattttggcatagcggtatgatcgacaagaaagttattgaaaaccgtaaacaggaagaatatattaataaactgcatagcactattcttgaattgaaaaatgagaagcatccagatatgatggattttatggacctgatagattggtatttagaaaatcgcaaaccacaagatattgattag

SEQ ID NO: 500 - protein, 62 aa, Bacteriophage D6938
MNKFWHSGMIDKKVIENRKQEEYINKLHSTILELKNEKHPDMMDFMDLIDWYLENRKPQDID

SEQ ID NO: 501 - DNA, 189 bp, Bacteriophage P5641
atgaagaaattttggcgtagtggcatgattgacaataaggttattgaaaaacgtaaacaagatgattatatgaataaattacacaggactattcttgagttgacccgtgaaattgaattgagacgtggcccagatatgatggatttcatggatctgatagattggtatttaaacagccgcaaaccgtag

SEQ ID NO: 502 - protein, 62 aa, Bacteriophage P5641
MKKFWRSGMIDNKVIEKRKQDDYMNKLHRTILELTREIELRRGPDMMDFMDLIDWYLNSRKP

SEQ ID NO: 503 - DNA, 216 bp, Bacteriophage D1765
atgaagaagttttggcatagcggtatgattgacaagaaagttattgaaaaacgccaacatgatgagtatataaataaaatacataagactattattgagttgaggaaagaaccacctgaacctaaaccttgctcttgtcacaaagatatagatattaatgctttgattaatgatattgagtgggatgattattatacatggtttaaagataaataa

SEQ ID NO: 504 - protein, 71 aa, Bacteriophage D1765
MKKFWHSGMIDKKVIEKRQHDEYINKIHKTIIELRKEPPEPKPCSCHKDIDINALINDIEWDDYYTWFKDK

SEQ ID NO: 505 - DNA, 216 bp, Bacteriophage D4212
atgaagaaattttggcgtagtggaatgattgacaagaaggttattgaaaaacgtaaacaagatgattatatgaataaattacacaggactattcttgagttgagtataaaaccacctgaacctaaaccttgctcttgtcacaaagatatagatattaatgctttgattaatgatattgagtgggatgattattatacatggtttaaagataaataa

SEQ ID NO: 506 - protein, 71 aa, Bacteriophage D4212
MKKFWRSGMIDKKVIEKRKQDDYMNKLHRTILELSIKPPEPKPCSCHKDIDINALINDIEWDDYYTWFKDK

SEQ ID NO: 507 - DNA, 216 bp, Bacteriophage D4250
atgaagaaattttggcgtagtggcatgattgacaagaaggttattgaaaaacgtaaacaggaagagtatatgaataagatgcataggactattcttgagttgagtataaaaccacctgaacctaaaccttgctcttgtcacaaagatatagatattaatgctttgattaatgatattgagtgggatgattattatacatggtttaaagataaataa

SEQ ID NO: 508 - protein, 71 aa, Bacteriophage D4250
MKKFWRSGMIDKKVIEKRKQEEYMNKMHRTILELSIKPPEPKPCSCHKDIDINALINDIEWDDYYTWFKDK

SEQ ID NO: 509 - DNA, 192 bp, Bacteriophage D4282
atgattgacaagaaggttattgaaaaacgtaaacaagatgattatatgaataaattacacaggactattcttgagttgagtataaaaccacctgaacctaaaccttgctcttgtcacaaagatatagatattaatgctttgattaatgatattgagtgggatgattattatacatggtttaaagataaataa

SEQ ID NO: 510 - protein, 63 aa, Bacteriophage D4282
MIDKKVIEKRKQDDYMNKLHRTILELSIKPPEPKPCSCHKDIDINALINDIEWDDYYTWFKDK

SEQ ID NO: 511 - DNA, 216 bp, Bacteriophage D7163
atgaagaaattttggcatagcggtatgattgacaagaaagttattaaaaaacgtaaacaggaagaatatatgaataaacttcaaagaattatccttgagttgagtataaaaccacctgaacctaaaccttgctcttgtcacaaagatatagatattaatgctttgattaatgatattgagtgggatgattattatacatggtttaaagataaataa

SEQ ID NO: 512 - protein, 71 aa, Bacteriophage D7163
MKKFWHSGMIDKKVIKKRKQEEYMNKLQRIILELSIKPPEPKPCSCHKDIDINALINDIEWDDYYTWFKDK

SEQ ID NO: 513 - DNA, 213 bp, Bacteriophage O1205
atgaagaagttttggcatagcggtatgattgacaagaaaattattgaaaaacgtgaacatgatgagtatttgaataaattacatatgactattattgagttgagaaaagaaccacctgaaactaaaccttgctcttgtcacaaaaatgtagatattaatgaattaattaactatattgagtggaatgattattatacatggtttaaagattaa

SEQ ID NO: 514 - protein, 70 aa, Bacteriophage O1205
MKKFWHSGMIDKKIIEKREHDEYLNKLHMTIIELRKEPPETKPCSCHKNVDINELINYIEWNDYYTWFKD

SEQ ID NO: 515 - DNA, 183 bp, Bacteriophage D4263
atgaagaaattttggcatagcggtatgatcgacaagaaagttattgaaaaacgtaaacaggatgagtatttgaataaattacacaggactattcttgagatagactttccaattcaacgtgtttgtcaccggtcactatcaccgacacccataacggtgcccacggaaacccttgatatataa

SEQ ID NO: 516 - protein, 60 aa, Bacteriophage D4263
MKKFWHSGMIDKKVIEKRKQDEYLNKLHRTILEIDFPIQRVCHRSLSPTPITVPTETLDI

SEQ ID NO: 517 - DNA, 135 bp, Bacteriophage D6252
atgaagaaattttggcatagcggtatgattgacaagaaagttattaaaaaacgtaaacaggaagagtatatgaataagatgcataggactattcttgagttgagtataaaaccaatagaagaaatggttttttaa

SEQ ID NO: 518 - protein, 44 aa, Bacteriophage D6252
MKKFWHSGMIDKKVIKKRKQEEYMNKMHRTILELSIKPIEEMVF

SEQ ID NO: 519 - DNA, 267 bp, Bacteriophage Sfi19
atgaagaaattttggcgtagtggaatgattgacaagaaggttattgaaaaacgtaaacaagatgattatatgaataaattacacaggactattcttgagttgagtataaaaccacctgaacctaaaccttgctcttgtcacaaagatatagatattaatgctttgattaatgatattgagtgggatgattgggtagatgaagtgttggaatatataaataaatgggtaaataaagataaagctgatgtggaggtattagataaatga

SEQ ID NO: 520 - protein, 88 aa, Bacteriophage Sfi19
MKKFWRSGMIDKKVIEKRKQDDYMNKLHRTILELSIKPPEPKPCSCHKDIDINALINDIEWDDWVDEVLEYINKWVNKDKADVEVLDK

SEQ ID NO: 521 - DNA, 633 bp, Bacteriophage D4234
atgaccaccccacaaaagtttcttagtatcagggaattgcttaaaccactccctagcaacggtgttaagtttcctaagttctctgcactctatcacgaaagccaagtgggagcgtggcagaagaaaatgagtaagcgaagacaccaagcaaaggtacaagtagctatggataagaaccgtggtgaactagttcctcgtgagttagaggacttctctaactggcaacgtgctagacaaatgaaagcacgctatcaagagaaggtggctaacaagcgtaaggactacctacacaaactaaccacttatcttgttaagacttatgatgttatcgtgattgaggacttgaaagctaagaacttgatgaagaaccattacttagctaaatcaatcgctaacgcttcatggcatgagtttaagagactgctagaatacaagtgttcgtggtatggcaaggaacttattgttgttccggctcaccatactagtcaagagtgttctaactgtcaccacaattcaggtaagaaaccgctccatatccgtgagtggatgtgtgataattgtggtactcaccatgatagagacattaacgcaagtatcaatatcttgcaccgtggacttgccacgttaaattaa

SEQ ID NO: 522 - protein, 210 aa, Bacteriophage D4234
MTTPQKFLSIRELLKPLPSNGVKFPKFSALYHESQVGAWQKKMSKRRHQAKVQVAMDKNRGELVPRELEDFSNWQRARQMKARYQEKVANKRKDYLHKLTTYLVKTYDVIVIEDLKAKNLMKNHYLAKSIANASWHEFKRLLEYKCSWYGKELIVVPAHHTSQECSNCHHNSGKKPLHIREWMCDNCGTHHDRDINASINILHRGLATLN

SEQ ID NO: 523 - DNA, 303 bp, Bacteriophage D4620
atgtcaacagttttcttgattttttttcaagtttttttgattttattattaaacatcttgaaaattagtaaaacatactatatattgttctttgtatgtatccattgtttttacctcgtttttttattttttatcgaatgttttccaagttgctctcaatccattctagtctattttggcgaccagacggaaactgtttttataaaaaaatatatatttttttgcaaaacaaaaaccctgactaattcaagtcagggcaagagagagtttatcgaagactcagcttttaactgtatccattaa

SEQ ID NO: 524 - protein, 100 aa, Bacteriophage D4620
MSTVFLIFFQVFLILLLNILKISKTYYILFFVCIHCFYLVFLFFIECFPSCSQSILVYFGDQTETVFIKKYIFFCKTKTLTNSSQGKREFIEDSAFNCIH

SEQ ID NO: 525 - DNA, 303 bp, Bacteriophage D5930
atgtcaacagttttcttgattttttttcaagttttcttgatttttttattaaacatcttgaaaattagtaaaacatactatatattgttctttgtatgtatccattgtttttacctcgtttttttattttttatcgaatgttttccaagttgctctcaatccattctagtctattttggtgaccagacggaaactgtttttataaaaaaatatatatttttttgcaaaacaaaaaccctgactaattcaagtcagggtgagagagagtttatcgaagactcagcttttaactgtattcattaa

SEQ ID NO: 526 - protein, 100 aa, Bacteriophage D5930
MSTVFLIFFQVFLIFLLNILKISKTYYILFFVCIHCFYLVFLFFIECFPSCSQSILVYFGDQTETVFIKKYIFFCKTKTLTNSSQGEREFIEDSAFNCIH

SEQ ID NO: 527 - DNA, 303 bp, Bacteriophage P0091
atgtcaacagttttcttgattttttttcaagttttcttgatttttttattaaacatcttgaaaattagtaaaacatactatatattgttctttgtatgtatccattgtttttacctcgtttttttattttttatcgaatgttttccaagttgctctcaatccattctagtctattttggtgaccagacggaaactgtttttataaaaaaatatatatttttttgcaaaacaaaaaccctgactaattcaagtcagggtgagagagagtttatcgaagataacagcttttactgtaaccattaa

SEQ ID NO: 528 - protein, 100 aa, Bacteriophage P0091
MSTVFLIFFQVFLIFLLNILKISKTYYILFFVCIHCFYLVFLFFIECFPSCSQSILVYFGDQTETVFIKKYIFFCKTKTLTNSSQGEREFIEDNSFYCNH

SEQ ID NO: 529 - DNA, 231 bp, Bacteriophage P0093
ttgattttttttaaagtttttttgattttattattaaacaacttgaaaattagtaaaacatactatatattgttctttgtatgtatccattgtttttacctcgtttttttattttttatcgaatattttccagattgttttcaatccattcaagtcgatttttgcgaccagacggaaactgtttttataaaaaattatatattttttttgcaaaacaaaaaccctgactaa

SEQ ID NO: 530 - protein, 76 aa, Bacteriophage P0093
MIFFKVFLILLLNNLKISKTYYILFFVCIHCFYLVFLFFIEYFPDCFQSIQVDFCDQTETVFIKNYIFFLQNKNPD

SEQ ID NO: 531 - DNA, 246 bp, Bacteriophage P0094
atgtcaatagttttcttgattttttttaaagtttttttgattttattattaaacaacttgaaaattagtaaaacatactatatattgttctttgtatgtatccattgtttttacctcgtttttttattttttatcgaatattttccagattgttttcaatccattcaagtcgatttttgcgaccagacggaaactgtttttataaaaaaatatatattttttttgcaaaacaaaaaccctgactaa

SEQ ID NO: 532 - protein, 81 aa, Bacteriophage P0094
MSIVFLIFFKVFLILLLNNLKISKTYYILFFVCIHCFYLVFLFFIEYFPDCFQSIQVDFCDQTETVFIKKYIFFLQNKNPD

SEQ ID NO: 533 - DNA, 234 bp, Bacteriophage P7632
atgtcaacagttttcttgattttttttcaagtttttttgatttttttatatatttactttaaaattagtaaaacatactatatattgttctttgtatgtatccattgtttttttattttttatcgaatgttttccaagttgctctcaatccattctagtctattttggcgaccagacggaaactgtttttataaaaaaatatatatttttttgcaaaacaaaaaccctgactaa

SEQ ID NO: 534 - protein, 77 aa, Bacteriophage P7632
MSTVFLIFFQVFLIFLYIYFKISKTYYILFFVCIHCFFIFYRMFSKLLSIHSSLFWRPDGNCFYKKIYIFLQNKNPD

SEQ ID NO: 535 - DNA, 219 bp, Bacteriophage P7952
ttgattttttttcaagttttcttgatttttttattaaacatcttgaaaattagtaaaacatactatatattgttctttgtatgtatccattgttttttattttttatcgaatgttttccaagttgctctcaatccattctagtctattttggcgaccagacggaaactgtttttataaaaaaaatatatatttttttgcaaaacaaaaaccctgactaa

SEQ ID NO: 536 - protein, 72 aa, Bacteriophage P7952
MIFFQVFLIFLLNILKISKTYYILFFVCIHCFLFFIECFPSCSQSILVYFGDQTETVFIKKIYIFLQNKNPD

SEQ ID NO: 537 - DNA, 198 bp, Bacteriophage D5738
ttgtttatttttgggaactgttgtataatgtttatactatatatatcatgtatgatagtttgtcaacagttttacctaaattattttagttttttttgcaaaaaaagaaaacctcgactaaaagtcgaggttacagttcgagaatttaaccgaaacgataccaagtattccaacaattatattaccacttttctatga

SEQ ID NO: 538 - protein, 65 aa, Bacteriophage D5738
MFIFGNCCIMFILYISCMIVCQQFYLNYFSFFCKKRKPRLKVEVTVREFNRNDTKYSNNYITTFL

SEQ ID NO: 539 - DNA, 189 bp, Bacteriophage D5839
gtgagttctgaacatagtattcaaaatcaaattcgagtggaattatccaaggctggcaacatggtatttagaattaacgttggtaaagtcagaatggctgatggacgttggtttgatactggagcaccaaaaggattttgtgacctgtttggatttagaccagctactgtaatagcacttatctattag

SEQ ID NO: 540 - protein, 62 aa, Bacteriophage D5839
MSSEHSIQNQIRVELSKAGNMVFRINVGKVRMADGRWFDTGAPKGFCDLFGFRPATVIALIY

SEQ ID NO: 541 - DNA, 141 bp, Bacteriophage P0093
ttgccaatcctctttattgtcggtaacgcacagggagcaagtcactgcactagaccgaagcccttacatcccgccaccttagaggtgggggaattacgggctgttaggttaaaaaaagcaaacaaaaaagccccagcataa

SEQ ID NO: 542 - protein, 46 aa, Bacteriophage P0093
MPILFIVGNAQGASHCTRPKPLHPATLEVGELRAVRLKKANKKAPA

SEQ ID NO: 543 - DNA, 171 bp, Bacteriophage P7152
atgtcaacagttttcttgattttttttcaagttttcttgatttttttattaaacatcttgaaaattagtaaaacatactatatattgttctttgtatgtatccattgtttttttattttttatcgaatgttttccaagttgctctcaatccattctagtctattttggtga

SEQ ID NO: 544 - protein, 56 aa, Bacteriophage P7152
MSTVFLIFFQVFLIFLLNILKISKTYYILFFVCIHCFFIFYRMFSKLLSIHSSLFW

SEQ ID NO: 545 - DNA, 144 bp, Bacteriophage P7954
ttgattttttttcaagttttcttgatttttttattaaacatcttgaaaattagtaaaacatactatatattgttctttgtatgtatccattgttttttttattttttatcgaatgttttccaagttgctctcaatccattctag

SEQ ID NO: 546 - protein, 47 aa, Bacteriophage P7954
MIFFQVFLIFLLNILKISKTYYILFFVCIHCFFYFLSNVFQVALNPF

SEQ ID NO: 547 - DNA, 171 bp, Bacteriophage P7953
ttggtcttagcccccaacaaaacgttcccttatgcttgtgtgtgcgcaagcaatagggcgctgaacctaatcagtcttttaccttttgcactagataaattgtatctaggttatccaattacattttatcaaattatcatttataagtcaaataaaaaagccccagcataa

SEQ ID NO: 548 - protein, 56 aa, Bacteriophage P7953
MVLAPNKTFPYACVCASNRALNLISLLPFALDKLYLGYPITFYQIIIYKSNKKAPA

SEQ ID NO: 549 - DNA, 198 bp, Bacteriophage P7955
ttgagaataaatgaagctgtactaagtttttatagtttttatttttatttattaaggaatttagtttttttttgcaaaaaaagaaaacctcgactaaaagtcgaggttacagttcgagaatttaaccgaaacgatgccaagtattccaacaattatatgaaaatagcaaacaaaaagagctacgagattatctcatag

SEQ ID NO: 550 - protein, 65 aa, Bacteriophage P7955
MRINEAVLSFYSFYFYLLRNLVFFCKKRKPRLKVEVTVREFNRNDAKYSNNYMKIANKKSYEIIS

SEQ ID NO: 551 - DNA, 195 bp, Bacteriophage Sequence3
ttgttctacctattgactaaagcgagtttttacctctctctttatcttatgtatacattacatatcatatatgatagtctgccaactgtttttataaaaaaatatatatttttttgcaaaacaaaaaccctgactaattcaagtcagggtgagagagagtttatcgaagactcagcttttaactgtattcattaa

SEQ ID NO: 552 - protein, 64 aa, Bacteriophage Sequence3
MFYLLTKASFYLSLYLMYTLHIIYDSLPTVFIKKYIFFCKTKTLTNSSQGEREFIEDSAFNCIH